European Patent Application EP 4 299 750 A2, published January 3, 2024. Title: COMPOSITIONS AND METHODS FOR TREATING ORNITHINE TRANSCARBAMYLASE DEFICIENCY. Applicant: ARCTURUS THERAPEUTICS, INC. Application EP, filed December 5, 2019. The sequence listing filed with the application follows.

SEQUENCE LISTING (253 sequences)

SEQ ID NO: 1 - RNA, 1065 nt, Homo sapiens
  source 1..1065: mol_type = mRNA
atgctgtttaatctgaggatcctgttaaacaatgcagcttttagaaatggtcacaacttcatggttcgaaattttcggtgtggacaaccactacaaaataaagtgcagctgaagggccgtgaccttctcactctaaaaaactttaccggagaagaaattaaatatatgctatggctatcagcagatctgaaatttaggataaaacagaaaggagagtatttgcctttattgcaagggaagtccttaggcatgatttttgagaaaagaagtactcgaacaagattgtctacagaaacaggctttgcacttctgggaggacatccttgttttcttaccacacaagatattcatttgggtgtgaatgaaagtctcacggacacggcccgtgtattgtctagcatggcagatgcagtattggctcgagtgtataaacaatcagatttggacaccctggctaaagaagcatccatcccaattatcaatgggctgtcagatttgtaccatcctatccagatcctggctgattacctcacgctccaggaacactatagctctctgaaaggtcttaccctcagctggatcggggatgggaacaatatcctgcactccatcatgatgagcgcagcgaaattcggaatgcaccttcaggcagctactccaaagggttatgagccggatgctagtgtaaccaagttggcagagcagtatgccaaagagaatggtaccaagctgttgctgacaaatgatccattggaagcagcgcatggaggcaatgtattaattacagacacttggataagcatgggacaagaagaggagaagaaaaagcggctccaggctttccaaggttaccaggttacaatgaagactgctaaagttgctgcctctgactggacatttttacactgcttgcccagaaagccagaagaagtggatgatgaagtcttttattctcctcgatcactagtgttcccagaggcagaaaacagaaagtggacaatcatggctgtcatggtgtccctgctgacagattactcacctcagctccagaagcctaaattttga

SEQ ID NO: 2 - DNA, 1065 bp, Homo sapiens
  source 1..1065: mol_type = other DNA
atgctgtttaatctgaggatcctgttaaacaatgcagcttttagaaatggtcacaacttcatggttcgaaattttcggtgtggacaaccactacaaaataaagtgcagctgaagggccgtgaccttctcactctaaaaaactttaccggagaagaaattaaatatatgctatggctatcagcagatctgaaatttaggataaaacagaaaggagagtatttgcctttattgcaagggaagtccttaggcatgatttttgagaaaagaagtactcgaacaagattgtctacagaaacaggctttgcacttctgggaggacatccttgttttcttaccacacaagatattcatttgggtgtgaatgaaagtctcacggacacggcccgtgtattgtctagcatggcagatgcagtattggctcgagtgtataaacaatcagatttggacaccctggctaaagaagcatccatcccaattatcaatgggctgtcagatttgtaccatcctatccagatcctggctgattacctcacgctccaggaacactatagctctctgaaaggtcttaccctcagctggatcggggatgggaacaatatcctgcactccatcatgatgagcgcagcgaaattcggaatgcaccttcaggcagctactccaaagggttatgagccggatgctagtgtaaccaagttggcagagcagtatgccaaagagaatggtaccaagctgttgctgacaaatgatccattggaagcagcgcatggaggcaatgtattaattacagacacttggataagcatgggacaagaagaggagaagaaaaagcggctccaggctttccaaggttaccaggttacaatgaagactgctaaagttgctgcctctgactggacatttttacactgcttgcccagaaagccagaagaagtggatgatgaagtcttttattctcctcgatcactagtgttcccagaggcagaaaacagaaagtggacaatcatggctgtcatggtgtccctgctgacagattactcacctcagctccagaagcctaaattttga

SEQ ID NO: 3 - protein, 353 aa, Homo sapiens
MLFNLRILLNNAAFRNGHNFMVRNFRCGQPLQNKVQLKGRDLLTLKNFTGEEIKYMLWLSADLKFRIKQKGEYLPLLQGKSLGMIFEKRSTRTRLSTETGFALLGGHPCFLTTQDIHLGVNESLTDTARVLSSMADAVLARVYKQSDLDTLAKEASIPIFGLSDLYHPIQILADYLTLQEHYSSLKGLTLSWIGDGNNILHSIMMSAAKFGMHLQAATPKGYEPDASVTKLAEQYAKENGTKLLLTNDPLEAAHGGNVLITDTWISMGQEEEKKKRLQAFQGYQVTMKTAKVAASDWTFLHCLPRKPEEVDDEVFYSPRSLVFPEAENRKWTIMAVMVSLLTDYSPQLQKPKF

SEQ ID NO: 4 - protein, 355 aa, synthetic construct
MLVFNLRILLNNAAFRNGHNFMVRNFRCGQPLQNRVQLKGRDLLTLKNFTGEEIRYMLWLSADLKFRIKQKGEYLPLLQGKSLGMIFEKRSTRTRLSTETGFALLGGHPCFLTTQDIHLGVNESLTDTARVLSSMADAVLARVYKQSDLDTLAKEASIPIINGLSDLYHPIQILADYLTLQEHYSSLKGLTLSWIGDGNNILHSIMMSAAKFGMHLQAATPKGYEPDASVTKLAEQYAKENGTKLLLTNDPLEAAHGGNVLITDTWISMGQEEEKKKRLQAFQGYQVTMKTAKVAASDWTFLHCLPRKPEEVDDEVFYSPRSLVFPEAENRKWTIMAVMVSLLTDYSPQLQKPKF

SEQ ID NO: 5 - RNA, 129 nt, synthetic construct
  source 1..129: mol_type = other RNA
tcaacacaacatatacaaaacaaacgaatctcaagcaatcaagcattctacttctattgcagcaatttaaatcatttcttttaaagcaaaagcaattttctgaaaattttcaccatttacgaacgatag

SEQ ID NO: 6 - RNA, 28 nt, synthetic construct
  source 1..28: mol_type = other RNA
attattacatcaaaacaaaaagccgcca

SEQ ID NO: 7 - RNA, 245 nt, synthetic construct
  source 1..245: mol_type = other RNA
cttaagggggcgctgcctacggaggtggcagccatctccttctcggcatcaagcttaccatggtgccccaggccctgctcttggtcccgctgctggtgttccccctctgcttcggcaagttccccatctacaccatccccgacaagctggggccgtggagccccatcgacatccaccacctgtcctgccccaacaacctcgtggtcgaggacgagggctgcaccaacctgagcgggttctcctac

SEQ ID NO: 8 - RNA, 177 nt, synthetic construct
  source 1..177: mol_type = other RNA
tgagtgtcgtacagcctccaggcccccccctcccgggagagccatagtggtctgcggaaccggtgagtacaccggaattgccgggaagactgggtcctttcttggataaacccactctatgcccggccatttgggcgtgcccccgcaagactgctagccgagtagtgttgggttgcg

SEQ ID NO: 9 - RNA, 89 nt, synthetic construct
  source 1..89: mol_type = other RNA
aattattggttaaagaagtatattagtgctaatttccctccgtttgtcctagcttttctcttctgtcaaccccacacgcctttggcaca

SEQ ID NO: 10 - RNA, 569 nt, synthetic construct
  source 1..569: mol_type = other RNA
ctccctcccccccccctaacgttactggccgaagccgcttggaataaggccggtgtgcgtttgtctatatgttattttccaccatattgccgtcttttggcaatgtgagggcccggaaacctggccctgtcttcttgacgagcattcctaggggtctttcccctctcgccaaaggaatgcaaggtctgttgaatgtcgtgaaggaagcagttcctctggaagcttcttgaagacaaacaacgtctgtagcgaccctttgcaggcagcggaaccccccacctggcgacaggtgcctctgcggccaaaagccacgtgtataagatacacctgcaaaggcggcacaaccccagtgccacgttgtgagttggatagttgtggaaagagtcaaatggctctcctcaagcgtattcaacaaggggctgaaggatgcccagaaggtaccccattgtatgggatctgatctggggcctcggtgcacatgctttacgtgtgtttagtcgaggttaaaaaacgtctaggccccccgaaccacggggacgtggttttcctttgaaaaacacgatgataat

SEQ ID NO: 11 - RNA, 44 nt, synthetic construct
  source 1..44: mol_type = other RNA
gtcagctttcaaactctttgtttcttgtttgttgattgagaata

SEQ ID NO: 12 - RNA, 54 nt, synthetic construct
  source 1..54: mol_type = other RNA
ctctcgcctgagaaaaaaaatccacgaaccaatttctcagcaaccagcagcacg

SEQ ID NO: 13 - RNA, 52 nt, synthetic construct
  source 1..52: mol_type = other RNA
acctgtgagggttcgaaggaagtagcagtgttttttgttcctagaggaagag

SEQ ID NO: 14 - RNA, 71 nt, synthetic construct
  source 1..71: mol_type = other RNA
acacagaaacattcgcaaaaacaaaatcccagtatcaaaattcttctctttttttcatatttcgcaaagac

SEQ ID NO: 15 - RNA, 52 nt, synthetic construct
  source 1..52: mol_type = other RNA
cagaaaaatttgctacattgtttcacaaacttcaaatattattcatttattt

SEQ ID NO: 16 - RNA, 158 nt, synthetic construct
  source 1..158: mol_type = other RNA
ctagtgactgactaggatctggttaccactaaaccagcctcaagaacacccgaatggagtctctaagctacataataccaacttacacttacaaaatgttgtcccccaaaatgtagccattcgtatctgctcctaataaaaagaaagtttcttcacat

SEQ ID NO: 17 - RNA, 166 nt, synthetic construct
  source 1..166: mol_type = other RNA
tgcaaggctggccggaagcccttgcctgaaagcaagatttcagcctggaagagggcaaagtggacgggagtggacaggagtggatgcgataagatgtggtttgaagctgatgggtgccagccctgcattgctgagtcaatcaataaagagctttcttttgacccat

SEQ ID NO: 18 - RNA, 143 nt, synthetic construct
  source 1..143: mol_type = other RNA
acgccgaagcctgcagccatgcgaccccacgccaccccgtgcctcctgcctccgcgcagcctgcagcgggagaccctgtccccgccccagccgtcctcctggggtggaccctagtttaataaagattcaccaagtttcacgca

SEQ ID NO: 19 - RNA, 220 nt, synthetic construct
  source 1..220: mol_type = other RNA
tagagcggcaaaccctagctacactccatagctagtttcttttttttttgtttttttttttttttttttttttttttttttttttttttcctttcttttccttctttttttcctcttttcttggtggctccatcttagccctagtcacggctagctgtgaaaggtccgtgagccgcatgactgcagagagtgccgtaactggtctctctgcagatcatgt

SEQ ID NO: 20 - RNA, 170 nt, synthetic construct
  source 1..170: mol_type = other RNA
acacatcacaaccacaaccttctcaggctaccctgagaaaaaaagacatgaagactcaggactcatcttttctgttggtgtaaaatcaacaccctaaggaacacaaatttctttaaacatttgacttcttgtctctgtgctgcaattaataaaaaatggaaagaatctac

SEQ ID NO: 21 - RNA, 110 nt, synthetic construct
  source 1..110: mol_type = other RNA
gctggagcctcggtagccgttcctcctgcccgctgggcctcccaacgggccctcctcccctccttgcaccggcccttcctggtctttgaataaagtctgagtgggcagca

SEQ ID NO: 22 - RNA, 123 nt, synthetic construct
  source 1..123: mol_type = other RNA
tagtgcagtcactggcacaacgcgttgcccggtaagccaatcgggtatacacggtcgtcatactgcagacagggttcttctactttgcaagatagtctagagtagtaaaataaatagtataag

SEQ ID NO: 23-25 - skipped (3 entries)

SEQ ID NO: 26 - RNA, 1368 nt, synthetic construct
  source 1..1368: mol_type = other RNA
tcaacacaacatatacaaaacaaacgaatctcaagcaatcaagcattctacttctattgcagcaatttaaatcatttcttttaaagcaaaagcaattttctgaaaattttcaccatttacgaacgatagccaccatgctgtttaatctgaggatcctgttaaacaatgcagcttttagaaatggtcacaacttcatggttcgaaattttcggtgtggacaaccactacaaaataaagtgcagctgaagggccgtgaccttctcactctaaaaaactttaccggagaagaaattaaatatatgctatggctatcagcagatctgaaatttaggataaaacagaaaggagagtatttgcctttattgcaagggaagtccttaggcatgatttttgagaaaagaagtactcgaacaagattgtctacagaaacaggctttgcacttctgggaggacatccttgttttcttaccacacaagatattcatttgggtgtgaatgaaagtctcacggacacggcccgtgtattgtctagcatggcagatgcagtattggctcgagtgtataaacaatcagatttggacaccctggctaaagaagcatccatcccaattatcaatgggctgtcagatttgtaccatcctatccagatcctggctgattacctcacgctccaggaacactatagctctctgaaaggtcttaccctcagctggatcggggatgggaacaatatcctgcactccatcatgatgagcgcagcgaaattcggaatgcaccttcaggcagctactccaaagggttatgagccggatgctagtgtaaccaagttggcagagcagtatgccaaagagaatggtaccaagctgttgctgacaaatgatccattggaagcagcgcatggaggcaatgtattaattacagacacttggataagcatgggacaagaagaggagaagaaaaagcggctccaggctttccaaggttaccaggttacaatgaagactgctaaagttgctgcctctgactggacatttttacactgcttgcccagaaagccagaagaagtggatgatgaagtcttttattctcctcgatcactagtgttcccagaggcagaaaacagaaagtggacaatcatggctgtcatggtgtccctgctgacagattactcacctcagctccagaagcctaaattttgactcgagctagtgactgactaggatctggttaccactaaaccagcctcaagaacacccgaatggagtctctaagctacataataccaacttacacttacaaaatgttgtcccccaaaatgtagccattcgtatctgctcctaataaaaagaaagtttcttcacattctag

SEQ ID NO: 27 - RNA, 1368 nt, synthetic construct
  source 1..1368: mol_type = other RNA
tcaacacaacatatacaaaacaaacgaatctcaagcaatcaagcattctacttctattgcagcaatttaaatcatttcttttaaagcaaaagcaattttctgaaaattttcaccatttacgaacgatagccaccatgctctttaatctgcgcatcttactgaacaacgccgcattccggaacggtcacaacttcatggtccgcaatttccgctgtggccagccgcttcaaaacaaggtccagctgaagggacgggatctgctgacactgaagaacttcaccggagaagagatcaagtacatgctgtggctcagcgcagacttgaagttccggatcaagcagaagggagaatacttgcccctgctgcaaggaaagtcgctgggaatgatttttgagaagcggtcaactcgcaccagactctccaccgaaactggtttcgcactgcttggcgggcacccttgcttcctgacgactcaggacatccacctcggcgtgaacgaatcgctaaccgataccgccagagtgctttcttccatggccgacgcggtgctggccagggtgtacaagcagtccgacctcgataccttggcaaaggaggcttccattcccatcatcaacggcctgagcgacctgtaccacccaatccaaatcctggctgactacctgaccctgcaagagcactacagcagcctgaagggtctgaccctgtcatggattggcgatggaaacaatattctgcactccatcatgatgtccgccgcgaagttcggaatgcatctgcaagccgccactccaaaaggatacgaaccggatgcgtccgtgaccaagttggcggaacagtacgcgaaggagaacggaaccaagcttctgctgactaacgaccccctcgaggctgcgcatgggggcaacgtgctgattaccgacacctggatctccatggggcaggaggaagagaagaagaagagactgcaggcattccaggggtaccaggtcaccatgaaaaccgcaaaagtggcagcttcggactggactttcctgcattgcctgccgaggaagccggaggaagtcgacgacgaagtgttctactcgcctcggtccctggtgttccccgaggccgaaaaccggaagtggaccatcatggccgtgatggtgtccttgctgactgactatagcccgcagctgcagaagcctaagttctagctcgagctagtgactgactaggatctggttaccactaaaccagcctcaagaacacccgaatggagtctctaagctacataataccaacttacacttacaaaatgttgtcccccaaaatgtagccattcgtatctgctcctaataaaaagaaagtttcttcacattctag

SEQ ID NO: 28 - RNA, 1368 nt, synthetic construct
  source 1..1368: mol_type = other RNA
tcaacacaacatatacaaaacaaacgaatctcaagcaatcaagcattctacttctattgcagcaatttaaatcatttcttttaaagcaaaagcaattttctgaaaattttcaccatttacgaacgatagccaccatgctgtttaacctacgtattttgctcaacaatgcagcctttagaaacggacataactttatggttcgaaactttcgctgcgggcagccactgcagaacaaggtccagctgaaagggagagatttgctcacgctgaagaactttactggcgaagaaatcaagtatatgctgtggttgtccgcggacctcaagtttcggattaagcagaaaggggagtatctgccactgctgcaaggaaagagcctcggcatgatcttcgagaagcggagcactcggaccaggctgagtaccgaaactggcttcgcattgttgggtggacatccatgttttctgacaacgcaggacattcatctgggcgtgaacgagagtctgacggacacagctcgcgttctgtcctctatggctgatgcggtgttggcccgggtctataagcagtccgatttggacaccttggctaaggaagctagcataccgattatcaatgggctgtccgacctgtatcaccctattcaaatcctggccgactacctcacactgcaagaacactatagctcattgaagggactgaccctgagctggataggggacggaaacaacatcctacatagcattatgatgtccgctgccaagtttggcatgcatcttcaagccgccacgccaaagggttatgagcccgacgcgtcagtgacaaagctggccgagcagtacgctaaggagaatggtaccaaattactgctgactaatgatccactggaggctgcacatggcggcaatgtactgatcaccgacacatggatctcgatgggccaggaggaagaaaagaagaagaggcttcaggccttccaaggctaccaggtcaccatgaaaacagctaaggttgcagcatctgattggacctttctgcactgtctgccaaggaagcccgaagaggtggacgatgaagtattctatagcccacggagtttggtgttccctgaggctgaaaataggaagtggacaattatggccgtaatggtgtccctgttaaccgactactctccgcaactgcagaaacctaagttttagctcgagctagtgactgactaggatctggttaccactaaaccagcctcaagaacacccgaatggagtctctaagctacataataccaacttacacttacaaaatgttgtcccccaaaatgtagccattcgtatctgctcctaataaaaagaaagtttcttcacattctag

SEQ ID NO: 29 - RNA, 1368 nt, synthetic construct
  source 1..1368: mol_type = other RNA
tcaacacaacatatacaaaacaaacgaatctcaagcaatcaagcattctacttctattgcagcaatttaaatcatttcttttaaagcaaaagcaattttctgaaaattttcaccatttacgaacgatagccaccatgctgtttaacttaaggatcctgctgaacaacgccgcttttcgtaacggtcataactttatggtccggaactttagatgtggccagccgctgcagaacaaggttcagctgaaggggagggatctgctgaccttgaagaactttaccggcgaagagatcaagtacatgttgtggctgagcgccgatctgaagtttaggattaagcagaagggggagtatttgccactgctgcaaggaaaatccttggggatgatcttcgagaagcgctccactagaacccggctaagcacagaaaccggcttcgcacttctgggtggacatccctgttttctgacgacgcaggatatacacctgggcgtgaatgagagtctgacggacacagctagggtgttgagcagcatggccgatgcagtactggcccgcgtttataagcagagcgacttggacacactggccaaggaagcgtcaattccgattatcaatgggctgtcagacctgtatcatcccattcaaatcttggctgactatctgaccctgcaagaacattacagctccctgaagggcctcacgttgtcctggattggcgacggaaacaacattctgcattcgatcatgatgagcgctgctaagtttggcatgcacctccaagccgctacacctaagggatatgagcctgatgccagcgtaaccaagctggccgaacagtacgcgaaggagaatggcacgaaactgctgttgacaaatgacccactggaggcagctcacggtggcaacgtgctgatcaccgacacgtggatatctatgggacaggaagaagagaagaagaagcggctgcaggcattccaagggtatcaggtcaccatgaaaacggccaaggttgctgcatccgactggacatttctgcattgcttgccccgcaaaccagaagaagtagacgacgaagtcttttattccccacggtcgctggtgttccccgaggcggagaatcgaaagtggacgattatggccgtgatggtgtccctgctgactgattactctccccaactgcaaaagcctaagttttagctcgagctagtgactgactaggatctggttaccactaaaccagcctcaagaacacccgaatggagtctctaagctacataataccaacttacacttacaaaatgttgtcccccaaaatgtagccattcgtatctgctcctaataaaaagaaagtttcttcacattctag

SEQ ID NO: 30 - RNA, 1368 nt, synthetic construct
  source 1..1368: mol_type = other RNA
tcaacacaacatatacaaaacaaacgaatctcaagcaatcaagcattctacttctattgcagcaatttaaatcatttcttttaaagcaaaagcaattttctgaaaattttcaccatttacgaacgatagccaccatgcttttcaacctgaggatcctcctgaacaacgccgcctttcgcaatggtcacaactttatggtccggaacttcagatgcggccagccgctgcagaacaaggtccagctgaagggacgggatctgctgactctgaagaacttcaccggagaagagatcaagtacatgctgtggctgtcggccgacctgaagttcaggatcaagcagaagggagaatacctcccgctgctgcaaggaaagtccctgggcatgattttcgagaagcgctcgaccagaactcggttgtccaccgaaaccgggtttgcgctgctgggcggacatccttgcttcctgacgactcaggatattcacctgggagtgaacgagtcgctgaccgacaccgccagagtgctgagctcgatggccgacgccgtgttggcacgcgtgtacaagcagtccgatctggataccctggccaaagaagcttccatcccgatcattaacgggctgagcgacctctaccaccccattcaaatcctggccgactacctgactctgcaagaacactacagctcgctgaaggggttgactctgtcctggatcggcgacggaaacaacatcctgcactccatcatgatgtcggccgcaaagttcggcatgcatttgcaagccgccaccccaaagggctacgaaccagacgcgagcgtcaccaagctggccgaacagtacgcgaaggaaaatggtactaagctgctgctgaccaacgacccattggaagctgcccatggtggaaacgtgctgatcaccgacacctggatctcgatgggccaggaagaggagaagaagaagcggctgcaggcgttccaggggtatcaggtcaccatgaaaacagccaaagtggcagcgtcagactggaccttcctccactgtctgcctcgcaagccagaggaggtggacgacgaggtgttctactcccctcggtccctcgtgttccctgaggctgagaaccggaagtggaccattatggccgtgatggtgtcactcctgactgattactccccgcaactgcagaagcccaagttctagctcgagctagtgactgactaggatctggttaccactaaaccagcctcaagaacacccgaatggagtctctaagctacataataccaacttacacttacaaaatgttgtcccccaaaatgtagccattcgtatctgctcctaataaaaagaaagtttcttcacattctag

SEQ ID NO: 31 - RNA, 1368 nt, synthetic construct
  source 1..1368: mol_type = other RNA
tcaacacaacatatacaaaacaaacgaatctcaagcaatcaagcattctacttctattgcagcaatttaaatcatttcttttaaagcaaaagcaattttctgaaaattttcaccatttacgaacgatagccaccatgctgtttaacctgaggatcctattgaacaatgctgcttttcgtaatggccataactttatggttcggaactttagatgcgggcagccactgcagaacaaggtccagttgaaaggccgcgatctgttgacattgaagaactttaccggcgaagagattaagtatatgctgtggctgtctgctgacctcaagtttcgaatcaagcagaagggcgaatatctccccctgctgcaaggaaagtctctcggcatgatctttgagaagcggagtacccgaacacggctgagcaccgaaacgggcttcgcactgctggggggccatccctgttttctgacaacgcaggacatccacttgggggttaacgaatcattgactgataccgcccgcgtactgtcatccatggccgacgctgtgctggctagggtgtacaagcagtcagatctggatacactggccaaggaagctagcataccaatcatcaatggactgagtgacctttatcacccgattcaaatactagccgattatctgaccctgcaagagcattactcctcgctgaaaggcctcacgctgtcctggatcggcgacggcaacaacattctgcatagtattatgatgtctgctgccaaattcggcatgcatctgcaagctgctacgccgaagggttatgaacccgacgcgtcagttacgaagctcgctgagcagtatgcaaaggagaatggcacaaagctgttgcttaccaacgatcccctggaagctgctcatggcggcaatgtgctgattactgacacctggatttcaatgggccaggaggaggagaagaagaagaggttacaggcttttcaaggttaccaagtcacgatgaaaaccgctaaggtcgcagccagcgactggacattcctgcactgtctgccaagaaagccggaagaagtggacgacgaggtgttctattccccgcggtctttggtgtttccggaggccgaaaacaggaaatggaccattatggccgtgatggtatcgttgctgacggactacagccctcagttgcaaaagcccaagttctagctcgagctagtgactgactaggatctggttaccactaaaccagcctcaagaacacccgaatggagtctctaagctacataataccaacttacacttacaaaatgttgtcccccaaaatgtagccattcgtatctgctcctaataaaaagaaagtttcttcacattctag

SEQ ID NO: 32 - RNA, 1368 nt, synthetic construct
  source 1..1368: mol_type = other RNA
tcaacacaacatatacaaaacaaacgaatctcaagcaatcaagcattctacttctattgcagcaatttaaatcatttcttttaaagcaaaagcaattttctgaaaattttcaccatttacgaacgatagccaccatgctctttaacctccgcatcctcctcaacaacgccgccttccggaatgggcataacttcatggtccggaacttcagatgcggccagcccctgcaaaacaaggtccagttgaagggacgggacctccttacgctgaagaactttaccggagaagagattaagtacatgctgtggttgtccgctgacctcaagttccgcattaagcagaagggagaatatctgccgctgctgcaaggaaagagcctgggcatgatcttcgaaaagcgctccactagaacccggctgtcgactgagactggattcgccttgctcggtggacacccgtgcttcctgacgacccaggacatccacctgggagtgaacgagtcacttacggataccgcgagggtgctgtcctcaatggccgacgcagtgctcgcgcgcgtgtacaagcagtcagatctggataccctggccaaggaagccagcattcccatcatcaacggactgagcgacctttaccacccaatccagatcctcgccgactacttaaccctgcaagagcactacagctccctgaagggactgactctgtcctggatcggggatggaaacaacatcctgcactccatcatgatgtctgccgctaagtttgggatgcatctgcaagccgcaacccctaagggatacgagcccgacgcctcggtgaccaaacttgcggaacagtacgccaaggaaaacggtaccaagctgctgctgaccaacgaccctctggaagcggcccacggaggaaatgtgctgattaccgacacctggatttcgatgggccaggaggaggagaagaagaagagactgcaggcgttccagggatatcaggtcaccatgaaaaccgccaaggtcgccgccagcgactggaccttcctgcactgtctccctcggaaaccggaagaagtggatgacgaggtgttctactccccgcgctcgctggtgttcccggaggctgaaaacaggaagtggacaatcatggccgtgatggtgtccctgttgaccgactactccccacaactgcagaagcccaagttctagctcgagctagtgactgactaggatctggttaccactaaaccagcctcaagaacacccgaatggagtctctaagctacataataccaacttacacttacaaaatgttgtcccccaaaatgtagccattcgtatctgctcctaataaaaagaaagtttcttcacattctag

SEQ ID NO: 33 - RNA, 1368 nt, synthetic construct
  source 1..1368: mol_type = other RNA
tcaacacaacatatacaaaacaaacgaatctcaagcaatcaagcattctacttctattgcagcaatttaaatcatttcttttaaagcaaaagcaattttctgaaaattttcaccatttacgaacgatagccaccatgcttttcaatctgcgcatcctcctgaacaacgccgccttccgcaatggacacaactttatggtccgcaacttccgctgtgggcagccgctgcagaacaaggtccagctcaaggggagagatctcctgaccctgaagaacttcactggagaggagatcaagtacatgctgtggctgtccgccgacctgaaatttcggattaagcagaagggcgaatacctcccactgctgcaaggaaagtctttgggcatgatcttcgaaaagagaagcacccggacccggttgagcaccgaaactgggttcgcgctcctcggtggacacccgtgcttcctgaccacccaagatattcatctgggtgtcaacgaaagcctgaccgacaccgccagggtgctgtcatccatggctgacgcagtgctcgcccgggtgtacaagcagtcagacctggacaccctcgccaaggaagcttcgatccctatcatcaacggactttccgacctgtaccaccccatccaaattctggccgactacctgactctgcaagaacactatagctcgctgaaaggacttactctgtcctggatcggggacggcaacaacattctccattccatcatgatgtccgctgccaagttcggaatgcaccttcaagcagcgactcccaagggatacgaacctgatgcctccgtgactaagctggcagagcagtacgccaaggagaacggtacaaagctgctgctcacgaacgaccccctggaggcggcccacggcggaaacgtgctgattaccgatacctggatctcaatgggccaggaagaggagaagaagaagcggctccaggcgtttcaaggctaccaggtcaccatgaaaaccgcgaaggtcgccgcctccgactggactttcttgcactgcctgccgcggaagcccgaggaagtggatgacgaagtgttctactcgccgagatcgttggtgttccctgaggccgaaaacaggaagtggaccatcatggccgtgatggtgtccctgctgactgattacagcccacagctgcagaagcctaagttctagctcgagctagtgactgactaggatctggttaccactaaaccagcctcaagaacacccgaatggagtctctaagctacataataccaacttacacttacaaaatgttgtcccccaaaatgtagccattcgtatctgctcctaataaaaagaaagtttcttcacattctag

SEQ ID NO: 34 - RNA, 1368 nt, synthetic construct
  source 1..1368: mol_type = other RNA
tcaacacaacatatacaaaacaaacgaatctcaagcaatcaagcattctacttctattgcagcaatttaaatcatttcttttaaagcaaaagcaattttctgaaaattttcaccatttacgaacgatagccaccatgcttttcaatctccgcatcctccttaacaacgccgcgtttagaaacggccacaacttcatggtccggaacttcagatgtggccagccgcttcaaaacaaggtccagctgaagggccgggatcttctgaccctgaagaactttactggcgaagagatcaagtacatgctctggctctccgcggacttgaagttccgcattaagcagaagggggaataccttccgctgcttcaaggaaagagcctcggcatgatctttgagaagcgctcaaccaggacccgcctttctactgaaactgggttcgcgctgctcggtggccacccctgcttcctgacgacccaggacatccacctcggagtgaacgaatccctcaccgataccgcccgggtgttatcgagcatggcagatgccgtgctggccagggtgtacaaacagtccgatctggacactctggccaaggaggcgtcaattcctattatcaacggccttagtgacctctaccatccgattcagatcctggccgattacctcaccctgcaagaacactacagctccctgaagggtctgacattgtcctggatcggcgacggcaacaacattctccattccatcatgatgtccgccgcaaaattcggcatgcatcttcaagccgccacgccgaagggttacgagcccgacgcttccgtgactaagctcgccgagcagtacgctaaggagaacggaaccaagcttctgctgactaacgacccactagaagcagcccacgggggcaacgtgcttattactgacacctggatctccatgggccaggaagaagagaaaaagaagcggctgcaggcgttccagggatatcaggtcaccatgaaaaccgccaaggtcgctgcctccgactggaccttcctgcactgcctgcctcgcaagcctgaagaagtggacgacgaggtgttctactcgccacggagcctcgtgttccccgaggccgagaatagaaagtggaccatcatggccgtgatggtgtcactgctcaccgactacagcccgcagcttcagaagcccaagttctagctcgagctagtgactgactaggatctggttaccactaaaccagcctcaagaacacccgaatggagtctctaagctacataataccaacttacacttacaaaatgttgtcccccaaaatgtagccattcgtatctgctcctaataaaaagaaagtttcttcacattctag

SEQ ID NO: 35 - RNA, 1368 nt, synthetic construct
  source 1..1368: mol_type = other RNA
tcaacacaacatatacaaaacaaacgaatctcaagcaatcaagcattctacttctattgcagcaatttaaatcatttcttttaaagcaaaagcaattttctgaaaattttcaccatttacgaacgatagccaccatgcttttcaacctgagaatcctcctgaacaacgccgccttccgcaatggtcataacttcatggtccgcaactttcgctgcggacagcctctccaaaacaaggtccagctcaaggggcgcgacctcctcacactgaagaacttcactggagaagaaatcaagtacatgctgtggctgagcgccgatctgaagttccggatcaagcagaagggagagtaccttcctctgctgcaagggaagtccttgggaatgattttcgagaagcggtccacccggaccaggctgagcactgaaactggcttcgccctgctgggaggccacccttgtttcctgaccactcaggacatccacctgggcgtgaacgagtccctgaccgatactgccagagtgctgtcctccatggccgacgccgtgctcgcccgggtgtacaagcagtcagacctcgatacgctggccaaggaagcctccattcccattatcaatggtctgtcggacctctaccatccaatccaaatcctcgccgactacctgactctgcaagaacactacagctcactcaagggcctcaccctctcctggatcggcgacggaaacaacatccttcactcgattatgatgtcggccgcgaagttcgggatgcacctccaagctgccactccaaaaggctacgagccggatgcctcagtgactaagttggcggaacagtatgcgaaggagaacggtaccaagctcctgctgactaacgacccgctggaggccgcccacgggggaaacgtgctcatcaccgatacttggatttccatgggacaggaggaagagaagaagaagcggttgcaggcatttcagggctaccaggtcaccatgaaaactgccaaagtcgccgccagcgactggaccttcctgcactgcctgccccgcaagcctgaagaagtggacgacgaggtgttctactctccccggtccctcgtgttccctgaggccgaaaacaggaagtggaccatcatggctgtgatggtgtccctcctgaccgactacagccctcagctccaaaaacccaagttttagctcgagctagtgactgactaggatctggttaccactaaaccagcctcaagaacacccgaatggagtctctaagctacataataccaacttacacttacaaaatgttgtcccccaaaatgtagccattcgtatctgctcctaataaaaagaaagtttcttcacattctag

SEQ ID NO: 36 - RNA, 1368 nt, synthetic construct
  source 1..1368: mol_type = other RNA
tcaacacaacatatacaaaacaaacgaatctcaagcaatcaagcattctacttctattgcagcaatttaaatcatttcttttaaagcaaaagcaattttctgaaaattttcaccatttacgaacgatagccaccatgcttttcaacctgagaatcctcttgaacaatgctgcttttcggaatggccacaactttatggttcggaacttccgttgcggccagcctttacaaaacaaggtccagctgaagggccgggatttgctcacactgaagaactttactggggaggagattaagtatatgctgtggctgtccgctgacctgaagtttaggatcaagcagaagggcgaatatctgccgctgctgcaagggaaaagtctgggcatgatttttgaaaagcgctctacccggaccagactgtctacggaaacaggctttgccctgctgggcggccacccctgttttctgacaacgcaggacatccatctgggcgtgaacgaatcactgaccgatactgctcgggtactcagttctatggctgacgcagtgctggctagggtgtacaagcagagcgacttggacacactggctaaggaggccagcatccccattatcaatggcctgtctgatttgtaccatcccattcaaatcctggctgattatctgacactacaagagcattactcaagtctgaagggtttgactctctcctggatcggcgacggcaacaacattttacattccattatgatgagtgctgctaagtttggcatgcatttgcaagctgctaccccaaagggctatgaacctgacgctagcgtaaccaagttggccgaacagtatgctaaagagaatggcaccaagctgctcctgacgaatgaccccctggaagctgctcatggcggaaacgtacttataactgatacatggattagcatgggccaggaagaggagaagaagaagagactgcaggccttccaaggctatcaggtcaccatgaaaactgccaaggttgcagctagcgactggaccttcctgcactgtttgccgaggaaacccgaggaggtggacgatgaagtcttttattctccccgctccttggtgtttcccgaggctgaaaatcgaaagtggacgataatggcagtgatggtgtccctactgaccgactattctccacaactgcagaagcctaaattctagctcgagctagtgactgactaggatctggttaccactaaaccagcctcaagaacacccgaatggagtctctaagctacataataccaacttacacttacaaaatgttgtcccccaaaatgtagccattcgtatctgctcctaataaaaagaaagtttcttcacattctag

SEQ ID NO: 37 - RNA, 1368 nt, synthetic construct
  source 1..1368: mol_type = other RNA
tcaacacaacatatacaaaacaaacgaatctcaagcaatcaagcattctacttctattgcagcaatttaaatcatttcttttaaagcaaaagcaattttctgaaaattttcaccatttacgaacgatagccaccatgcttttcaatctgaggatcctgctgaacaacgctgcttttcgcaacggtcataactttatggttcgcaattttcgttgtggccagccgctgcagaacaaggttcagctgaagggcagagatctgctgactctgaagaacttcactggggaagaaatcaagtatatgttatggctgtccgcggatctgaaatttcgaatcaagcagaagggcgaatatcttcccctgctgcaagggaaatccttgggcatgatttttgagaagaggagcactaggactagattgtcaacagaaacaggctttgctttgttgggcggacatccctgctttctgacgacacaggatatccacctcggcgtaaacgagtccctcaccgacactgctagggtactgagcagcatggccgacgctgtgctagcccgggtttacaagcagtcagacctggacacccttgccaaggaagcttctattccaattatcaacggcctgagtgacctgtatcaccctattcaaatactcgccgactatttgacgcttcaagaacattacagcagcctcaagggcttaaccttgagttggataggcgacggcaacaatatcctgcattccattatgatgtctgccgctaagtttggcatgcatctacaagccgcaacacccaagggctatgaacccgacgctagcgtgaccaagctggccgagcagtatgctaaggaaaatggcacaaagctccttcttaccaacgatcccctggaggctgctcacggcggcaacgtgctgattaccgatacatggattagcatgggccaggaggaggagaaaaagaagcggctccaggcttttcaaggctatcaggtcaccatgaaaactgcaaaggtcgctgcctccgactggactttcctgcattgtctaccccgcaagcctgaggaagtggacgatgaggtgttctactccccacggagtctggtgttcccggaagcagagaatcggaagtggaccatcatggctgtcatggtgtcgctcttgactgactattctccccaactgcaaaaacccaagttttagctcgagctagtgactgactaggatctggttaccactaaaccagcctcaagaacacccgaatggagtctctaagctacataataccaacttacacttacaaaatgttgtcccccaaaatgtagccattcgtatctgctcctaataaaaagaaagtttcttcacattctag

SEQ ID NO: 38 - RNA, 1368 nt, synthetic construct
  source 1..1368: mol_type = other RNA
tcaacacaacatatacaaaacaaacgaatctcaagcaatcaagcattctacttctattgcagcaatttaaatcatttcttttaaagcaaaagcaattttctgaaaattttcaccatttacgaacgatagccaccatgttattcaaccttcgtatcctgctaaacaatgctgcttttcgcaatggccataactttatggttcgcaactttagatgcggccagccgctgcagaacaaggttcagctgaagggccgggacttgctgacgctgaaaaactttaccggggaagagattaagtatatgctgtggctaagcgctgatctgaagtttaggatcaagcagaagggcgaatatctgccactgctgcaagggaagagtcttggcatgatttttgaaaagcggtctaccagaacccggctgtcgaccgagacaggttttgctctgctggggggccatccctgttttctgacaactcaggacattcacctgggcgtgaatgagtccctgaccgatactgctagggtgttgagtagcatggccgacgctgtactcgctcgagtgtataagcagtctgatctggacactctggctaaggaagcttccattcctattatcaacggcttgagcgacctgtaccaccccattcaaatcctcgctgattacttgactttgcaagaacattacagcagcttgaagggcttaacactgagctggataggcgacggaaacaacatcttgcattccataatgatgtccgccgctaagttcgggatgcacctccaagcagccacacccaagggctatgaaccggatgcttccgtgacaaaactggctgagcagtatgctaaggagaatggcacgaaactgctgctcaccaacgacccattggaagctgcacatggtggcaacgtactgatcactgacacttggatctcaatgggccaggaggaagagaagaagaaaaggctgcaggcatttcagggataccaagtcactatgaaaactgccaaggtcgctgcctccgactggacattcctgcattgtctgccacggaagcctgaggaagtcgatgacgaagtgttctatagcccacgaagcttggtgtttcccgaggctgagaataggaagtggaccattatggctgttatggtgtccctgctcaccgactattcccctcaactgcaaaaacccaagttttagctcgagctagtgactgactaggatctggttaccactaaaccagcctcaagaacacccgaatggagtctctaagctacataataccaacttacacttacaaaatgttgtcccccaaaatgtagccattcgtatctgctcctaataaaaagaaagtttcttcacattctag

SEQ ID NO: 39 - RNA, 1365 nt, synthetic construct
  source 1..1365: mol_type = other RNA
tcaacacaacatatacaaaacaaacgaatctcaagcaatcaagcattctacttctattgcagcaatttaaatcatttcttttaaagcaaaagcaattttctgaaaattttcaccatttacgaacgatagccatgctttttaatctccgcatcctccttaacaacgccgcgtttagaaacggccacaacttcatggtccggaacttcagatgtggccagccgcttcaaaacaaggtccagctgaagggccgggatcttctgaccctgaagaactttactggcgaagagatcaagtacatgctctggctctccgcggacttgaagttccgcattaagcagaagggggaataccttccgctgcttcaaggaaagagcctcggcatgatctttgagaagcgctcaaccaggacccgcctttctactgaaactgggttcgcgctgctcggtggccacccctgcttcctgacgacccaggacatccacctcggagtgaacgaatccctcaccgataccgcccgggtgttatcgagcatggcagatgccgtgctggccagggtgtacaaacagtccgatctggacactctggccaaggaggcgtcaattcccatcatcaacggcctgagcgacctgtaccacccaatccaaatcctggctgactacctgaccctgcaagagcactacagcagcctgaagggtctgaccctgtcatggattggcgatggaaacaatattctgcactccatcatgatgtccgccgcgaagttcggaatgcatctgcaagccgccacgccaaaaggatacgaaccggatgcgtccgtgacgaagttggcggaacagtacgcgaaggagaacggaaccaagcttctgctgactaacgaccccctcgaggctgcgcatgggggcaacgtgctgattaccgacacctggatctccatggggcaggaggaagagaagaagaagagactgcaggcattccaggggtaccaggtcaccatgaaaaccgcaaaagtggcagcttcggactggactttcctgcattgcctgccgaggaagccggaggaagtcgacgacgaagtgttctactcgcctcggtccctggtgttccccgaggccgaaaaccggaagtggaccatcatggccgtgatggtgtccttgctgactgactatagcccgcagctgcagaagcctaagttctagctcgagctagtgactgactaggatctggttaccactaaaccagcctcaagaacacccgaatggagtctctaagctacataataccaacttacacttacaaaatgttgtcccccaaaatgtagccattcgtatctgctcctaataaaaagaaagtttcttcacattctag

SEQ ID NO: 40 - RNA, 1365 nt, synthetic construct
  source 1..1365: mol_type = other RNA
tcaacacaacatatacaaaacaaacgaatctcaagcaatcaagcattctacttctattgcagcaatttaaatcatttcttttaaagcaaaagcaattttctgaaaattttcaccatttacgaacgatagccatgcttttcaacctgagaatcctcttgaacaatgctgcttttcggaatggccacaactttatggttcggaacttccgttgcggccagcctttacaaaacaaggtccagctgaagggccgggatttgctcacactgaagaactttactggagaagagatcaagtacatgctgtggctgtcggccgacctgaagttcaggatcaagcagaagggagaataccttccgctgcttcaaggaaagagcctcggcatgatctttgagaagcgctcaaccaggacccgcctttctactgaaactgggttcgcgctgctcggtggccacccctgcttcctgacgacccaggacatccacctcggagtgaacgaatccctcaccgataccgcccgggtgttatcgagcatggcagatgccgtgctggccagggtgtacaaacagtccgatctcgataccttggcaaaggaggcttccattcccatcatcaacggcctgagcgacctgtaccacccaatccaaatcctggctgactacctgaccctgcaagagcactacagcagcctgaagggtctgaccctgtcatggattggcgatggaaacaatattctgcactccatcatgatgtccgccgcgaagttcggaatgcatctgcaagccgccactccaaaaggatacgaaccggatgcgtccgtgaccaagttggcggaacagtacgcgaaggagaacggaaccaagcttctgctgactaacgaccccctcgaggctgcgcatgggggcaacgtgctgattaccgacacctggatctccatggggcaggaggaagagaagaagaagagactgcaggcattccaggggtaccaggtcaccatgaaaaccgcaaaagtggcagcttcggactggactttcctgcattgcctgccgaggaagccggaggaagtcgacgacgaagtgttctactcgcctcggtccctggtgttccccgaggccgaaaaccggaagtggaccatcatggccgtgatggtgtccttgctgactgactatagcccgcagctgcagaagcctaagttctagctcgagctagtgactgactaggatctggttaccactaaaccagcctcaagaacacccgaatggagtctctaagctacataataccaacttacacttacaaaatgttgtcccccaaaatgtagccattcgtatctgctcctaataaaaagaaagtttcttcacattctag

SEQ ID NO: 41 - RNA, 1365 nt, synthetic construct
  source 1..1365: mol_type = other RNA
tcaacacaacatatacaaaacaaacgaatctcaagcaatcaagcattctacttctattgcagcaatttaaatcatttcttttaaagcaaaagcaattttctgaaaattttcaccatttacgaacgatagccatgcttttcaacctgagaatcctcttgaacaatgctgcttttcggaatggccacaactttatggttcggaacttccgttgcggccagcctttacaaaacaaggtccagctgaagggccgggatttgctcacactaaagaactttactggagaagagatcaagtacatgctatggctgtcggccgacctgaagttccgtatcaagcagaagggagaataccttccgctgcttcaaggaaagagcctcggcatgatctttgagaagcgctcaaccaggacccgcctttctactgaaactgggttcgcgctgctcggtggccacccctgcttcctgacgacccaggacatccacctcggagtgaacgaatccctcaccgataccgcccgggtgttatcgagcatggcagatgccgtgctggccagggtgtacaaacagtccgatctcgataccttggcaaaggaggcttccattcccatcatcaacggcctgagcgacctgtaccacccaatccaaatcctggctgactacctgaccctgcaagagcactacagcagcctgaagggtctgaccctgtcatggattggcgatggaaacaatattctgcactccatcatgatgtccgccgcgaagttcggaatgcatctgcaagccgccactccaaaaggatacgaaccggatgcatccgtgaccaagttggcggaacagtacgcgaaggagaacggaaccaagctcctgctgactaacgacccgctcgaggctgcgcatgggggtaacgtgctgattacggacacctggatctccatggggcaggaggaagagaagaagaagagactgcaggcattccaggggtaccaggtcaccatgaaaaccgcaaaagtggcagcttcggactggactttcctgcattgcctgccgaggaagccggaggaagtcgacgacgaagtgttctactcgcctcggtccctggtgttccccgaggccgaaaaccggaagtggaccatcatggccgtgatggtgtccttgctgactgactatagcccgcagctgcagaagcctaagttctagctcgagctagtgactgactaggatctggttaccactaaaccagcctcaagaacacccgaatggagtctctaagctacataataccaacttacacttacaaaatgttgtcccccaaaatgtagccattcgtatctgctcctaataaaaagaaagtttcttcacattctag

SEQ ID NO: 42 - RNA, 1365 nt, synthetic construct
  source 1..1365: mol_type = other RNA
tcaacacaacatatacaaaacaaacgaatctcaagcaatcaagcattctacttctattgcagcaatttaaatcatttcttttaaagcaaaagcaattttctgaaaattttcaccatttacgaacgatagccatgcttttcaacctgagaatcctcttgaacaatgctgcttttcggaatggccacaactttatggttcggaacttccgttgcggccagcctttacaaaacaaggtccagctgaagggccgggatttgctcacactaaagaactttactggagaagagatcaagtacatgctatggctgtcggccgacctgaagttccgtatcaagcagaagggagaataccttccgctgcttcaaggaaagagcctcggcatgatctttgagaagcgctcaaccaggacccgcctttctactgaaactgggttcgcgctgctcggtggccacccctgcttcctgacgacccaggacatccacctcggagtgaacgaatccctcaccgataccgcccgggtgttatcgagcatggcagatgccgtgctggccagggtgtacaaacagtccgatctcgataccttggcaaaggaggcttccattcccatcatcaacggcctgagcgacctgtaccacccaatccaaatcctggctgactacctgaccctgcaagagcactacagcagcctgaagggtctgaccctgtcatggattggcgatggaaacaatattctgcactccatcatgatgtccgccgcgaagttcggaatgcatctgcaagccgccactccaaaaggatacgaaccggatgcgtccgtgaccaagttggcggaacagtacgcgaaggagaacggaaccaagcttctgctgactaacgaccccctcgaggctgcgcatgggggcaacgtgctgattaccgacacctggatctccatggggcaggaggaagagaagaagaagagactgcaggcattccaggggtaccaggtcaccatgaaaaccgcaaaagtggcagcttcggactggactttcctgcattgcctgccgaggaagccggaggaagtcgacgacgaagtgttctactcgcctcggtccctggtgttccccgaggccgaaaaccggaagtggaccatcatggccgtgatggtgtccttgctgactgactatagcccgcagctgcagaagcctaagttctagctcgagctagtgactgactaggatctggttaccactaaaccagcctcaagaacacccgaatggagtctctaagctacataataccaacttacacttacaaaatgttgtcccccaaaatgtagccattcgtatctgctcctaataaaaagaaagtttcttcacattctag

SEQ ID NO: 43 - RNA, 1371 nt, synthetic construct
  source 1..1371: mol_type = other RNA
tcaacacaacatatacaaaacaaacgaatctcaagcaatcaagcattctacttctattgcagcaatttaaatcatttcttttaaagcaaaagcaattttctgaaaattttcaccatttacgaacgatagccaccatgctgttcaacctgcgaatcctgctgaacaacgccgcttttcggaacgggcacaactttatggtgaggaactttcgctgcggacagcccctccagaataaggtccagctgaagggcagggacctgctgaccctgaaaaatttcacaggggaggaaatcaagtatatgctgtggctgtcagctgatctgaagttccggatcaagcagaagggcgaatatctgcctctgctccagggcaaaagcctggggatgatcttcgaaaagcgcagtactcggaccagactgtcaaccgagactggattcgctctgctgggaggacacccttgttttctgaccactcaggacattcacctgggagtgaacgagtccctgaccgacactgctcgcgtcctgagctctatggccgacgctgtgctggctcgagtctacaaacagtccgacctggataccctggccaaggaagcttctatcccaattattaacggcctgtcagacctgtatcaccccatccagattctggccgattacctgaccctccaggagcactattctagtctgaaagggctgacactgagttggattggggacggaaacaatatcctgcactctattatgatgtcagccgccaagtttggaatgcacctccaggctgcaaccccaaaaggctacgaacccgatgcctcagtgacaaagctggctgaacagtacgccaaagagaacggcactaagctgctgctgaccaacgaccctctggaggccgctcacggaggcaacgtgctgatcaccgatacctggattagtatgggacaggaggaagagaagaagaagcggctccaggccttccagggctaccaggtgacaatgaaaaccgctaaggtcgcagccagcgattggacctttctgcactgcctgcccagaaagcccgaagaggtggacgacgaggtcttctactctcccagaagcctggtgtttcccgaagctgagaataggaagtggacaattatggcagtgatggtcagcctgctgactgattattcacctcagctccagaaaccaaagttctgataactcgagctagtgactgactaggatctggttaccactaaaccagcctcaagaacacccgaatggagtctctaagctacataataccaacttacacttacaaaatgttgtcccccaaaatgtagccattcgtatctgctcctaataaaaagaaagtttcttcacattctag

SEQ ID NO: 44 - RNA, 1371 nt, synthetic construct
  source 1..1371: mol_type = other RNA
tcaacacaacatatacaaaacaaacgaatctcaagcaatcaagcattctacttctattgcagcaatttaaatcatttcttttaaagcaaaagcaattttctgaaaattttcaccatttacgaacgatagccaccatgctgttcaacctgcgcatcctgctgaacaacgccgccttccgcaacggccacaacttcatggtgcgcaacttccgctgcggccagcccctgcagaacaaggtgcagctgaagggccgcgacctgctgaccctgaagaacttcaccggcgaggagatcaagtacatgctgtggctgagcgccgacctgaagttccgcatcaagcagaagggcgagtacctgcccctgctgcagggcaagagcctgggcatgatcttcgagaagcgcagcacccgcacccgcctgagcaccgagacaggcctggccctgctgggcggccacccctgcttcctgaccacccaggacatccacctgggcgtgaacgagagcctgaccgacaccgcccgcgtgctgagcagcatggccgacgccgtgctggcccgcgtgtacaagcagagcgacctggacaccctggccaaggaggccagcatccccatcatcaacggcctgagcgacctgtaccaccccatccagatcctggccgactacctgaccctgcaggagcactacagcagcctgaagggcctgaccctgagctggatcggcgacggcaacaacatcctgcacagcatcatgatgagcgccgccaagttcggcatgcacctgcaggccgccacccccaagggctacgagcccgacgccagcgtgaccaagctggccgagcagtacgccaaggagaacggcaccaagctgctgctgaccaacgaccccctggaggccgcccacggcggcaacgtgctgatcaccgacacctggatcagcatgggccaggaggaggagaagaagaagcgcctgcaggccttccagggctaccaggtgaccatgaagaccgccaaggtggccgccagcgactggaccttcctgcactgcctgccccgcaagcccgaggaggtggacgacgaggtgttctacagcccccgcagcctggtgttccccgaggccgagaaccgcaagtggaccatcatggccgtgatggtgagcctgctgaccgactacagcccccagctgcagaagcccaagttctgataactcgagctagtgactgactaggatctggttaccactaaaccagcctcaagaacacccgaatggagtctctaagctacataataccaacttacacttacaaaatgttgtcccccaaaatgtagccattcgtatctgctcctaataaaaagaaagtttcttcacattctag

SEQ ID NO: 45 - RNA, 1371 nt, synthetic construct
  source 1..1371: mol_type = other RNA
tcaacacaacatatacaaaacaaacgaatctcaagcaatcaagcattctacttctattgcagcaatttaaatcatttcttttaaagcaaaagcaattttctgaaaattttcaccatttacgaacgatagccaccatgctgttcaacctgcgaatcctgctgaacaacgccgcttttcggaacgggcacaactttatggtgaggaactttcgctgcggacagcccctccagaataaggtccagctgaagggcagggacctgctgaccctgaaaaatttcacaggggaggaaatcaagtatatgctgtggctgtcagctgatctgaagttccggatcaagcagaagggcgaatatctgcctctgctccagggcaaaagcctggggatgatcttcgaaaagcgcagtactcggaccagactgtcaaccgagactggattcgctctgctgggaggacacccttgttttctgaccactcaggacattcacctgggagtgaacgagtccctgaccgacactgctcgcgtcctgagctctatggccgacgctgtgctagctcgagtctacaaacagtccgacctggataccctggccaaggaagcttctatcccaattattaacggcctgtcagacctgtatcaccccatccagattctggccgattacctgaccctccaggagcactattctagtctgaaagggctgacactgagttggattggggacggaaacaatatcctgcactctattatgatgtcagccgccaagtttggaatgcacctccaggctgcaaccccaaaaggctacgaacccgatgcctcagtgacaaagctggctgaacagtacgccaaagagaacggcactaagctgctgctgaccaacgaccctctggaggccgctcacggaggcaacgtgctgatcaccgatacctggattagtatgggacaggaggaagagaagaagaagcggctccaggccttccagggctaccaggtgacaatgaaaaccgctaaggtcgcagccagcgattggacctttctgcactgcctgcccagaaagcccgaagaggtggacgacgaggtcttctactctcccagaagcctggtgtttcccgaagctgagaataggaagtggacaattatggcagtgatggtcagcctgctgactgattattcacctcagctccagaaaccaaagttctgataactcgagctagtgactgactaggatctggttaccactaaaccagcctcaagaacacccgaatggagtctctaagctacataataccaacttacacttacaaaatgttgtcccccaaaatgtagccattcgtatctgctcctaataaaaagaaagtttcttcacattctag

SEQ ID NO: 46 - RNA, 1371 nt, synthetic construct
  source 1..1371: mol_type = other RNA
tcaacacaacatatacaaaacaaacgaatctcaagcaatcaagcattctacttctattgcagcaatttaaatcatttcttttaaagcaaaagcaattttctgaaaattttcaccatttacgaacgatagccaccatgctgttcaacctgcgaatcctgctgaacaatgccgcttttcggaacgggcacaatttcatggtgaggaactttcgctgcggacagcccctccagaacaaggtccagctgaagggcagggacctgctgaccctgaaaaatttcacaggggaggaaatcaagtacatgctgtggctgtcagccgatctgaagttccggatcaagcagaagggcgaatatctgcctctgctccagggcaaaagcctggggatgatcttcgaaaagcgcagtactcggaccagactgtcaacagagactggattcgcactgctgggaggacacccatgttttctgaccacacaggacattcatctgggagtgaacgagtccctgaccgacacagcacgcgtcctgagctccatggctgatgcagtgctggctcgagtctacaaacagtctgacctggataccctggccaaggaagcttctatcccaatcattaatggcctgagtgacctgtatcaccccatccagattctggccgattacctgaccctccaggagcattattctagtctgaaagggctgacactgagctggattggggacggaaacaatatcctgcactccattatgatgagcgccgccaagtttggaatgcacctccaggctgcaaccccaaaaggctacgaacccgatgcctccgtgacaaagctggcagaacagtatgccaaagagaacggcactaagctgctgctgaccaatgaccctctggaggccgctcacggaggcaacgtgctgatcactgatacctggattagtatgggacaggaggaagagaagaagaagcggctccaggccttccagggctaccaggtgacaatgaaaactgctaaggtcgcagccagcgactggacctttctgcattgcctgcccagaaagcctgaagaggtggacgatgaggtcttctactcacccagaagcctggtgtttcctgaagctgagaataggaagtggacaatcatggcagtgatggtcagcctgctgactgattattcccctcagctccagaaaccaaagttctgataactcgagctagtgactgactaggatctggttaccactaaaccagcctcaagaacacccgaatggagtctctaagctacataataccaacttacacttacaaaatgttgtcccccaaaatgtagccattcgtatctgctcctaataaaaagaaagtttcttcacattctag

SEQ ID NO: 47 - RNA, 1368 nt, synthetic construct
  source 1..1368: mol_type = other RNA
tcaacacaacatatacaaaacaaacgaatctcaagcaatcaagcattctacttctattgcagcaatttaaatcatttcttttaaagcaaaagcaattttctgaaaattttcaccatttacgaacgatagccaccatgcttttcaaccttcgcattctcctcaacaacgccgcgtttagaaacggacacaacttcatggtccgcaacttccgctgcggacagccgctgcagaacaaggtccagctcaagggtcgggatctcctgacgctgaagaactttaccggcgaagagattaagtacatgctgtggctgtccgccgaccttaagttccggatcaagcagaagggcgaataccttcccctgctgcaaggaaagtccctgggcatgatcttcgagaagcgcagtaccagaaccagactctccactgaaaccgggttcgcgctgcttggcggccacccgtgtttcctcactacgcaagacatccatcttggcgtgaacgagtcccttaccgacaccgccagggtgctgtcaagcatggccgacgccgtccttgcgcgcgtgtacaagcagtcagaccttgatactctggccaaggaagcctccatccctattatcaacggcctatccgacctttaccacccgatccagatcctcgctgactacctgaccctgcaagaacactacagcagcctcaagggactgactctgtcctggatcggcgacgggaacaacatcctgcactcaatcatgatgagcgcagccaagttcggcatgcatctccaagccgctacacccaagggttatgaaccggacgcctctgtgaccaagttggcagaacagtacgccaaggagaacggtactaagctccttttaaccaacgaccccctcgaagcagcccatggcgggaatgtgctcattaccgatacctggatttcgatgggccaggaggaggagaagaagaagcggctgcaggcgttccagggctaccaggtcaccatgaaaactgccaaagtggccgcctcggattggacctttctccactgcctgcctcggaagcctgaggaggtggacgacgaagtgttctactccccacggtccctcgtgttccccgaggccgaaaataggaagtggaccatcatggccgtgatggtgtccctcttgaccgattacagcccgcagcttcagaagcctaaattctagctcgagctagtgactgactaggatctggttaccactaaaccagcctcaagaacacccgaatggagtctctaagctacataataccaacttacacttacaaaatgttgtcccccaaaatgtagccattcgtatctgctcctaataaaaagaaagtttcttcacattctag

SEQ ID NO: 48 - RNA, 1368 nt, synthetic construct
  source 1..1368: mol_type = other RNA
tcaacacaacatatacaaaacaaacgaatctcaagcaatcaagcattctacttctattgcagcaatttaaatcatttcttttaaagcaaaagcaattttctgaaaattttcaccatttacgaacgatagccaccatgcttttcaatcttcgcatcctgttgaacaacgccgccttccgcaatggtcacaacttcatggtccggaacttcagatgtggacagcctctccaaaacaaggtccagctgaagggaagggacctcttaaccctcaaaaactttactggagaggagatcaagtacatgctgtggcttagcgccgaccttaagttccggatcaagcagaagggagagtacctcccgctgctgcaaggaaagagtcttggaatgatcttcgagaagcggtccaccagaactcgcctctccactgaaaccggattcgcactcctgggtggacacccgtgctttctgaccacccaagacatccacctcggagtgaacgagagcctcacggacaccgcgagagtgctgtcatccatggccgacgccgtgcttgcacgggtctacaagcagtccgatctggacactcttgccaaggaagcctccattcctatcattaacggtctgtcggatctgtaccacccgattcagatccttgcggactacctcacacttcaagaacactattcaagcctaaagggtctgaccctgtcctggatcggagatggaaacaacattctccattccatcatgatgagcgctgccaagttcggaatgcatctccaagcagcgactcctaagggttacgagccggacgcctcagtgactaagctggccgagcagtacgccaaggagaacggtaccaaactgttgcttactaacgacccgcttgaagcggcccatggaggaaacgtgctgattaccgacacctggatttcgatgggacaggaagaggagaagaagaagcggctccaggcgttccagggataccaggtcaccatgaaaacggccaaagtggccgctagcgattggacctttctgcactgcctcccgcgcaagcctgaagaagtggacgacgaagtgttctactcccctcgctctcttgtgttcccggaagccgaaaacaggaagtggaccatcatggccgtgatggtgtccctcctgaccgattacagcccgcagctgcagaagcctaagttctagctcgagctagtgactgactaggatctggttaccactaaaccagcctcaagaacacccgaatggagtctctaagctacataataccaacttacacttacaaaatgttgtcccccaaaatgtagccattcgtatctgctcctaataaaaagaaagtttcttcacattctag

SEQ ID NO: 49 - RNA, 1368 nt, synthetic construct
  source 1..1368: mol_type = other RNA
tcaacacaacatatacaaaacaaacgaatctcaagcaatcaagcattctacttctattgcagcaatttaaatcatttcttttaaagcaaaagcaattttctgaaaattttcaccatttacgaacgatagccaccatgcttttcaatctccgcatcctcctcaacaacgccgcgtttagaaacggccacaacttcatggtccggaacttcagatgtggccagccgcttcagaacaaggtccagctcaagggccgggatcttctgaccctgaagaactttactggcgaagaaatcaagtacatgctctggctctccgccgacttgaagttccgcattaagcagaagggggaataccttccgctgctgcaaggaaagtcgctcggcatgatctttgagaagcgctcaacccgcaccaggctgtccactgaaaccgggttcgcgctgcttggtggccacccctgcttcctgaccacccaagacattcacctcggagtgaacgaatcgctcactgatactgcccgggtgctgtcgtcgatggccgatgcagtgctggccagggtgtacaaacagtccgatctggacactctggccaaggaggcgtccatccctattatcaacggcctttccgacctctaccacccgattcagatccttgccgattacctcaccctgcaagaacactactcgtcactgaagggtctgaccttgtcctggatcggcgacggcaacaacatcctccattccattatgatgtccgccgccaaattcggcatgcatcttcaagccgcaacccctaagggttacgagccggacgcttccgtgaccaagctcgccgagcagtacgctaaggagaacggaaccaagcttctgctgactaacgaccccctagaggcagcccacgggggcaacgtgcttattactgacacctggatctccatgggacaggaagaagagaagaagaagcggttacaggcgttccagggctatcaggtcaccatgaaaaccgccaaggtcgctgcctcggactggaccttcctgcattgcctgcctcgcaagcccgaagaagtggacgacgaggtgttctactcgccacggtcccttgtgttccctgaggccgagaatagaaagtggaccattatggccgtgatggtgtcccttctcaccgactactcgccgcaactgcagaaacccaagttctagctcgagctagtgactgactaggatctggttaccactaaaccagcctcaagaacacccgaatggagtctctaagctacataataccaacttacacttacaaaatgttgtcccccaaaatgtagccattcgtatctgctcctaataaaaagaaagtttcttcacattctag

SEQ ID NO: 50 - RNA, 1368 nt, synthetic construct
  source 1..1368: mol_type = other RNA
tcaacacaacatatacaaaacaaacgaatctcaagcaatcaagcattctacttctattgcagcaatttaaatcatttcttttaaagcaaaagcaattttctgaaaattttcaccatttacgaacgatagccaccatgcttttcaatcttcgcatcctcctcaacaacgccgccttccggaacggtcacaacttcatggtccggaacttccgctgcggccagccgctccaaaacaaagtgcagcttaagggccgcgatctcctgaccctgaagaacttcaccggagaggaaatcaagtacatgctgtggctctcggcggacctgaagtttaggattaagcagaagggggagtatctgccgctgctccaagggaagtcccttggcatgatcttcgaaaagaggtccacccggactcggctcagcaccgaaacaggttttgcacttctggggggccacccgtgcttcctgacgacccaggacatccatctgggtgtcaacgagagtttgaccgacactgccagagtgctgtcatccatggcggacgcggtgctcgcgagagtgtacaagcagtccgatcttgacaccctggcaaaagaggcttcaatcccgatcattaacggactctcggatctgtaccaccctatccaaatcttggccgactacctgaccctgcaagaacactacagctccctgaagggcctgactctttcctggattggcgatggaaacaacattctccattctattatgatgtccgccgccaagttcggcatgcaccttcaagccgccaccccgaagggctacgaacctgacgcctccgtgactaagctagccgaacagtacgctaaggagaacggcactaagcttctccttaccaacgatccgctggaggcggcccatggcggaaatgtgcttatcaccgacacctggattagcatggggcaggaagaagagaagaagaaacggctccaggcattccagggctaccaggtcaccatgaaaactgccaaggtcgccgctagcgactggaccttcctccactgtctgcctcgcaagcctgaagaagtggacgacgaggtgttctactccccgcgctccctcgtgtttcctgaggccgagaacagaaagtggaccatcatggccgtgatggtgtcattacttacggactacagcccgcagctgcagaagccgaagttctagctcgagctagtgactgactaggatctggttaccactaaaccagcctcaagaacacccgaatggagtctctaagctacataataccaacttacacttacaaaatgttgtcccccaaaatgtagccattcgtatctgctcctaataaaaagaaagtttcttcacattctag

SEQ ID NO: 51 - RNA, 1368 nt, synthetic construct
  source 1..1368: mol_type = other RNA
tcaacacaacatatacaaaacaaacgaatctcaagcaatcaagcattctacttctattgcagcaatttaaatcatttcttttaaagcaaaagcaattttctgaaaattttcaccatttacgaacgatagccaccatgctttttaacttgagaatccttctgaacaacgccgctttccgcaacggtcataacttcatggtccggaacttcagatgtggccagcccctccaaaacaaagtgcagctgaagggccgggaccttcttacgctgaagaatttcaccggcgaagaaatcaagtacatgctctggctgtccgccgatcttaagttccgcattaagcagaagggggaatacctcccgctgctgcaagggaagtcgctgggcatgatttttgagaagcggtcaactcgcacccgcctgtccactgaaactggattcgcactgctcggtggccatccctgcttcctgaccacccaagacatccacctcggcgtgaacgagtccctgactgacaccgcccgggtcttatcctcgatggccgatgctgtgcttgcgagggtgtacaagcagtccgacctcgacacactcgcgaaggaggcctccatccccatcatcaacggcctgtccgacctttaccacccaattcagatcctcgccgattacctgaccctgcaagagcactactcgtcgctcaaggggcttaccctctcgtggattggcgacggcaacaacatccttcactccatcatgatgtcggcagcgaagttcggcatgcatctgcaagccgccacgcctaagggttatgaaccggatgcctcagtgaccaagctcgccgaacagtacgcgaaagagaatggaaccaagctacttctgaccaacgaccccctggaggccgctcacggcggcaacgtcctcattaccgatacttggatttcgatgggacaggaagaggaaaagaagaagagactgcaggcgttccagggataccaggtcaccatgaaaactgccaaagtggcagcctccgactggaccttccttcactgcctgccgaggaagcctgaagaggtggacgacgaggtgttctactccccgcgctccttggtgtttcctgaggccgaaaaccggaagtggactatcatggccgtgatggtgtccctcctcaccgactactcgccgcaactgcagaagcctaagttctagctcgagctagtgactgactaggatctggttaccactaaaccagcctcaagaacacccgaatggagtctctaagctacataataccaacttacacttacaaaatgttgtcccccaaaatgtagccattcgtatctgctcctaataaaaagaaagtttcttcacattctag

SEQ ID NO: 52 - RNA, 1368 nt, synthetic construct
  source 1..1368: mol_type = other RNA
tcaacacaacatatacaaaacaaacgaatctcaagcaatcaagcattctacttctattgcagcaatttaaatcatttcttttaaagcaaaagcaattttctgaaaattttcaccatttacgaacgatagccaccatgttattcaaccttagaattctccttaacaacgccgccttccggaatgggcataactttatggtccgcaatttccgctgtggacagcctctgcaaaacaaggtccagctcaagggccgggatctgctgactctcaagaacttcactggggaagaaatcaagtacatgctctggctgagcgccgacctcaagttccgcatcaagcagaagggagagtacctcccgctgctccaagggaagtccctgggcatgatcttcgagaagagatccacccgcaccagactttccactgagactggcttcgccttgctgggaggccacccatgcttcctgacgacccaggacattcaccttggcgtgaacgagtccctgactgacaccgcaagggtgttgtcctcgatggccgacgccgtgcttgcccgggtgtacaagcagagcgatcttgacaccctggctaaggaagcttccattcccatcatcaacggtctgagcgacctgtaccacccgattcagatcctggcggactacctaaccctgcaagagcactatagctccctgaagggcctcacactttcatggatcggcgacggcaacaacatcctgcactctattatgatgagcgctgccaaattcggcatgcacctccaagccgccacgcctaaaggctacgagcccgacgcctcggtgaccaagcttgcggagcagtacgcgaaggaaaacggcaccaagctgcttctcaccaacgatcctctggaagcggcccatggtggcaacgtgctcattaccgacacttggatctccatgggacaggaggaggaaaagaagaagcggctccaggcgtttcagggttaccaggtcaccatgaaaaccgccaaggtcgcagcctccgactggaccttccttcattgccttccgcgcaagcccgaagaagtggacgatgaagtgttttactcacctcggtcactcgtgttcccggaagcagagaacaggaaatggaccattatggccgtgatggtgtccctgctcaccgattacagtccgcaactgcagaagcccaagttctagctcgagctagtgactgactaggatctggttaccactaaaccagcctcaagaacacccgaatggagtctctaagctacataataccaacttacacttacaaaatgttgtcccccaaaatgtagccattcgtatctgctcctaataaaaagaaagtttcttcacattctag

SEQ ID NO: 53 - RNA, 1368 nt, synthetic construct
  source 1..1368: mol_type = other RNA
tcaacacaacatatacaaaacaaacgaatctcaagcaatcaagcattctacttctattgcagcaatttaaatcatttcttttaaagcaaaagcaattttctgaaaattttcaccatttacgaacgatagccaccatgcttttcaatctccgcatcctccttaacaacgccgcgtttagaaacggccacaacttcatggtccggaacttcagatgtggccagccgcttcaaaacaaggtccagctgaagggccgggatcttctgaccctgaagaactttactggcgaagagatcaagtacatgctctggctctccgcggacttgaagttccgcattaagcagaagggggaataccttccgctgcttcaaggaaagagcctcggcatgatctttgagaagcgctcaaccaggacccgcctttctactgaaactgggttcgcgctgctcggtggccacccctgcttcctgacgacccaggacatccacctcggagtgaacgaatccctcaccgataccgcccgggtgttatcgagcatggcagatgccgtgctggccagggtgtacaaacagtccgatctggacactctggccaaggaggcgtcaattcctattatcaacggccttagtgacctctaccatccgattcaaatcctggccgattacctcaccctgcaagaacactacagctccctgaagggtctgacattgtcctggatcggcgacggcaacaacattctccattccatcatgatgtccgccgcaaaattcggcatgcatcttcaagccgccacgcctaagggttacgaacccgacgcttccgtgactaagctcgccgagcagtacgctaaggagaacggaaccaagctgctgctgactaacgacccgctagaagcagcccacgggggcaacgtgcttattactgacacctggatctccatgggccaggaggaagagaaaaagaagcggctgcaggcgttccagggatatcaggtcaccatgaaaaccgccaaggtcgctgcctccgactggaccttcctgcactgcctgcctcgcaagcctgaagaagtggacgacgaggtgttctactcgccacggagcctcgtgttccccgaggccgagaatagaaagtggaccatcatggccgtgatggtgtcacttctcaccgactacagcccgcagcttcagaagcccaagttctagctcgagctagtgactgactaggatctggttaccactaaaccagcctcaagaacacccgaatggagtctctaagctacataataccaacttacacttacaaaatgttgtcccccaaaatgtagccattcgtatctgctcctaataaaaagaaagtttcttcacattctag

SEQ ID NO: 54 - RNA, 1368 nt, synthetic construct
  source 1..1368: mol_type = other RNA
tcaacacaacatatacaaaacaaacgaatctcaagcaatcaagcattctacttctattgcagcaatttaaatcatttcttttaaagcaaaagcaattttctgaaaattttcaccatttacgaacgatagccaccatgcttttcaatctccgcatcctccttaacaacgccgcgtttagaaacggccacaacttcatggtccggaacttcagatgtggccagccgcttcaaaacaaggtccagcttaagggccgggatctcctcacccttaaaaacttcaccggcgaagagatcaagtacatgctctggctctccgcggaccttaagttccgcattaagcagaagggggaataccttccgctgcttcaaggaaagagcctcggcatgatctttgagaagcgctcaaccaggaccaggctttctactgaaactgggttcgcgcttctcggcggtcatccctgcttcctcacgacccaagacatccacctcggagtgaacgaatccctcacggatactgcccgcgtgctttcgagcatggcagacgccgtgctcgcccgggtgtacaaacagtccgatctcgacactctcgccaaggaggcgtcaattcctattatcaacggtcttagtgacctttaccacccgatccagatcctcgccgattacctcacactccaagaacactacagctcccttaagggtcttaccctctcctggatcggcgacggcaacaacattctccactccatcatgatgtccgccgcaaagttcggcatgcatcttcaagccgccaccccgaagggctacgagcctgatgcttccgtgactaagctcgccgagcagtacgctaaggagaacggaaccaagcttcttctcactaacgacccactcgaagcagcccatgggggcaacgtgcttatcactgacacctggatctccatgggccaggaagaagagaagaagaagcggctccaggcgttccagggatatcaggtcaccatgaaaaccgccaaggtcgctgcctccgactggacctttctccactgcctccctcgcaaacctgaagaagtggacgacgaggtgttctactcgccccggagcctcgtgttccccgaggccgagaatagaaagtggaccattatggccgtgatggtgtcactcctcaccgactacagcccgcagcttcagaagcccaagttctagctcgagctagtgactgactaggatctggttaccactaaaccagcctcaagaacacccgaatggagtctctaagctacataataccaacttacacttacaaaatgttgtcccccaaaatgtagccattcgtatctgctcctaataaaaagaaagtttcttcacattctag

SEQ ID NO: 55 - RNA, 1368 nt, synthetic construct
  source 1..1368: mol_type = other RNA
tcaacacaacatatacaaaacaaacgaatctcaagcaatcaagcattctacttctattgcagcaatttaaatcatttcttttaaagcaaaagcaattttctgaaaattttcaccatttacgaacgatagccaccatgcttttcaatctccgcatcctccttaacaacgccgcgtttagaaacggacataacttcatggtccggaacttcagatgtggacagccgcttcaaaacaaggtccagctgaagggtcgggatcttctgaccctgaagaactttaccggagaagagatcaagtacatgctctggctctccgcggacttgaagttccgcattaagcagaagggagaatacctcccgctgcttcaaggaaagagcctcggaatgatttttgagaagcgctcaaccaggacccgcctttctactgaaactggattcgcgctgctgggtggacacccctgcttcctgacgacccaggacatccacctcggagtgaacgaatccctcactgataccgcccgggtgttatcgagcatggcagatgccgtgctggccagggtgtacaaacagtccgatctggacactctggccaaggaggcgtcaattcctatcatcaacggacttagtgacctctaccatccgattcaaatcctggccgactacctcaccctgcaagaacactacagctccctgaagggtctgacattgtcctggatcggagatggaaacaacattctccactccatcatgatgtccgccgcaaaattcggaatgcatcttcaagccgccacgcctaagggttacgaacccgacgcttccgtgactaagctcgccgagcagtacgctaaggagaacggtaccaagcttctcctgaccaacgacccactagaagcagcccacggtggaaacgtgcttattactgacacttggatctccatgggacaggaggaagagaaaaagaagcggctgcaggcgttccagggatatcaggtcaccatgaaaaccgccaaggtcgctgcctccgactggaccttcctgcactgcctgcctcgcaagcctgaagaagtggacgacgaggtgttctactcgccgcggagcctcgtgttccccgaggccgagaatagaaagtggaccatcatggccgtgatggtgtcactgctcaccgactacagcccgcagcttcagaagcccaagttctagctcgagctagtgactgactaggatctggttaccactaaaccagcctcaagaacacccgaatggagtctctaagctacataataccaacttacacttacaaaatgttgtcccccaaaatgtagccattcgtatctgctcctaataaaaagaaagtttcttcacattctag

SEQ ID NO: 56 - RNA, 1368 nt, synthetic construct
  source 1..1368: mol_type = other RNA
tcaacacaacatatacaaaacaaacgaatctcaagcaatcaagcattctacttctattgcagcaatttaaatcatttcttttaaagcaaaagcaattttctgaaaattttcaccatttacgaacgatagccaccatgcttttcaacctccgcattctcctcaacaacgctgccttccggaatggacataacttcatggtccggaacttcagatgcggacagccgcttcagaacaaggtccagcttaaggggagagatctccttaccctcaaaaacttcactggcgaagaaatcaagtacatgctctggcttagtgcggatctcaagttccgcatcaagcagaagggagaatacctcccgctccttcaaggaaagagcctcggcatgatttttgagaagaggtccaccagaactcgcctttcaaccgagactgggttcgccctgcttggcggtcacccctgcttcctcactacccaagacatccacctcggcgtgaacgagagccttaccgacaccgcccgcgtgctctcctcaatggccgacgctgtgctcgcccgggtgtacaagcagtccgaccttgatactctcgccaaggaggcctccatcccaattatcaacgggctctctgatctctaccaccctatccaaatcctcgcggactacctcaccctccaagagcactatagctcgctcaagggcctcaccctttcctggattggcgacggcaacaacattcttcactcgatcatgatgtccgccgccaagttcggcatgcatctccaagccgcgacccccaagggctacgagcctgacgcatccgtgaccaagctcgccgagcagtacgcgaaggaaaatggcaccaagcttcttctcaccaacgacccccttgaggccgctcatggcggcaacgtgctcatcactgacacttggatcagcatgggccaggaggaggaaaagaagaagcgccttcaggcattccagggttaccaggtcaccatgaaaaccgccaaagtggccgcctccgactggacctttcttcactgtctcccgcggaagcctgaagaagtggatgacgaagtgttttactcccctcggtcactcgtgttcccggaagcagaaaacaggaagtggaccattatggcggtcatggtgtccctcctcaccgactacagcccgcagcttcagaaacccaagttctagctcgagctagtgactgactaggatctggttaccactaaaccagcctcaagaacacccgaatggagtctctaagctacataataccaacttacacttacaaaatgttgtcccccaaaatgtagccattcgtatctgctcctaataaaaagaaagtttcttcacattctag

SEQ ID NO: 57 - RNA, 1368 nt, synthetic construct
  source 1..1368: mol_type = other RNA
tcaacacaacatatacaaaacaaacgaatctcaagcaatcaagcattctacttctattgcagcaatttaaatcatttcttttaaagcaaaagcaattttctgaaaattttcaccatttacgaacgatagccaccatgcttttcaatctccgcatcctccttaacaacgcagcgtttagaaacggtcacaacttcatggtccggaacttccgctgtggacagccgcttcaaaacaaggtccagctgaagggtcgggaccttctgaccctgaagaactttactggagaagagatcaagtacatgctttggctgtccgcggacttgaagttccgcattaagcagaagggagaataccttccgctgctccaaggaaagagcctgggaatgatctttgagaagcgctcaaccaggacccgcctttctactgaaactggattcgcgctgctgggtggtcacccttgcttcctgacgacccaggacattcacctcggagtgaacgagtccctcactgataccgccagagtgttatcgagcatggcagatgccgtgctggctagggtgtacaaacagtccgatctggacaccctggccaaggaggcatcaattcctattatcaacggacttagtgacctctaccatccgattcaaatcctggccgattacctcaccctgcaagaacactacagctccctgaagggtctgacattgtcctggatcggagatggaaacaacattctccattccatcatgatgtccgcggccaagttcggaatgcatctccaagccgccacgccgaaaggatacgagccggacgcttccgtgactaagctcgccgagcagtacgctaaggagaacggaaccaagcttctgctgactaacgacccgctagaagccgcccacggtggaaacgtgcttattactgacacctggatctccatgggacaggaagaagagaaaaagaagcggctgcaggcgttccagggatatcaggtcaccatgaaaaccgccaaggtcgccgcctccgactggaccttccttcactgcctgcctcggaagcctgaagaagtggacgacgaggtgttctactcgccgcggagcctcgtgttccctgaggccgagaatagaaagtggaccatcatggccgtgatggtgtcactcctcaccgactacagcccgcagcttcagaagcctaagttctagctcgagctagtgactgactaggatctggttaccactaaaccagcctcaagaacacccgaatggagtctctaagctacataataccaacttacacttacaaaatgttgtcccccaaaatgtagccattcgtatctgctcctaataaaaagaaagtttcttcacattctag

SEQ ID NO: 58 - RNA, 1368 nt, synthetic construct
  source 1..1368: mol_type = other RNA
tcaacacaacatatacaaaacaaacgaatctcaagcaatcaagcattctacttctattgcagcaatttaaatcatttcttttaaagcaaaagcaattttctgaaaattttcaccatttacgaacgatagccaccatgcttttcaatctccgcattctcctcaacaacgcagcctttagaaacggccacaacttcatggtccggaacttcagatgtggccagccgcttcagaacaaggtccagctcaagggccgggacctcctcaccctcaaaaactttaccggcgaagagatcaagtacatgctctggctttcggccgaccttaagttccgcatcaagcagaagggggaataccttccgctgcttcaaggaaagtccctcggcatgatctttgaaaagcgctcgaccaggacccgcctttccactgaaaccgggttcgcgcttctcggtggccacccctgcttcctcaccacccaagacattcacctcggagtgaacgaatcccttaccgataccgcaagagtgctttcgtcgatggccgatgccgtgcttgcgcgggtgtacaagcagtcagatctcgacactctcgccaaggaggcgtccattcctattatcaacggcctttccgacctttaccacccgattcagatcctcgccgattacctcaccctgcaagagcactactcgtcactcaagggtcttaccctctcctggatcggcgacggaaacaacatcctccattcgatcatgatgtccgccgccaaattcggcatgcacctccaagccgcgaccccgaagggttacgagcccgacgcttccgtgaccaagctcgccgaacagtacgctaaggaaaacggcaccaagctcctcctcactaacgaccctctcgaagcagcccatgggggcaacgtgctcattactgacacttggatctcgatgggccaggaagaggagaaaaagaagcggcttcaggcgttccagggatatcaggtcaccatgaaaaccgccaaggtcgctgcctcggactggaccttccttcactgccttccgcgcaagcctgaagaggtggacgatgaggtgttctactccccacggtcccttgtgttccccgaggccgagaataggaagtggaccatcatggccgtgatggtgtcgctcctcactgactactccccgcaacttcagaagcctaagttctagctcgagctagtgactgactaggatctggttaccactaaaccagcctcaagaacacccgaatggagtctctaagctacataataccaacttacacttacaaaatgttgtcccccaaaatgtagccattcgtatctgctcctaataaaaagaaagtttcttcacattctag

SEQ ID NO: 59 - RNA, 1368 nt, synthetic construct
  source 1..1368: mol_type = other RNA
tcaacacaacatatacaaaacaaacgaatctcaagcaatcaagcattctacttctattgcagcaatttaaatcatttcttttaaagcaaaagcaattttctgaaaattttcaccatttacgaacgatagccaccatgctgtttaatctgagaatacttctaaacaacgccgccttccggaatggccataactttatggttcggaatttccgctgcggccagccgctgcagaacaaggtccagctgaagggaagagacttgctgaccctcaagaacttcaccggagaagaaatcaagtatatgctgtggctgtccgccgacctgaaattccgcatcaagcagaagggcgaatatctgccgctgttgcaagggaagtccctggggatgatcttcgagaagaggtccaccagaacacggctttcaaccgaaaccgggtttgcactgctgggtggacacccctgttttctgaccactcaagatatccacctgggcgtgaacgagtcccttaccgacactgctagggtgttgtccagcatggccgatgccgtcctggctcgcgtgtacaagcagtccgacctggataccctggcaaaggaagcgtccattcccattatcaacgggctgtccgacctgtaccatccgattcaaatcctggcggactacctgactctgcaagagcattacagcagcttgaaggggcttactctctcgtggatcggcgacgggaacaacatcctgcactccatcatgatgtccgccgccaagttcgggatgcatttgcaagctgcgaccccgaaaggttacgagcccgatgctagcgtaactaagcttgccgaacagtacgccaaagagaatggtacaaaactgcttctgactaacgacccgctggaagcagcccacggcgggaacgtgctgataaccgacacctggatttcaatggggcaggaggaagagaagaagaagcgactgcaggcgttccaaggctatcaggttaccatgaaaaccgccaaagtggcagccagcgattggactttcctgcactgtctgccgcggaagcccgaggaagttgatgacgaagtattctactcaccccggagcctcgtgttccccgaggccgaaaaccggaagtggactattatggccgtgatggtgtcgctgttgaccgactacagcccgcaactgcagaagccgaagttttagctcgagctagtgactgactaggatctggttaccactaaaccagcctcaagaacacccgaatggagtctctaagctacataataccaacttacacttacaaaatgttgtcccccaaaatgtagccattcgtatctgctcctaataaaaagaaagtttcttcacattctag

SEQ ID NO: 60 - RNA, 1368 nt, synthetic construct
  source 1..1368: mol_type = other RNA
tcaacacaacatatacaaaacaaacgaatctcaagcaatcaagcattctacttctattgcagcaatttaaatcatttcttttaaagcaaaagcaattttctgaaaattttcaccatttacgaacgatagccaccatgcttttcaacctgaggatccttttgaacaacgccgcctttcgcaacggccacaactttatggtccgcaatttccgctgcgggcagccgctgcagaacaaggtccagctgaagggccgggatctgctgaccctgaagaacttcaccggggaggaaatcaagtacatgctttggctctccgccgatctgaagttcagaatcaagcagaagggagagtacctcccgttgctgcaaggaaagtcactcggaatgattttcgaaaagagaagcactaggacccgcctctcaactgaaaccgggttcgcgctgctcgggggccatccgtgtttcctgactacccaagacatccacctgggagtgaacgagtcgctgaccgacaccgcacgcgtgctgtcatccatggcggacgcagtgcttgcccgggtgtacaagcagtcggacctggacactcttgccaaggaggcatcaatccccatcattaacggactgtccgatctctaccacccgattcagatcctggctgactacctaaccctgcaagagcactactcaagcctgaaggggctgaccctgtcgtggatcggggacggcaacaacattctgcactccatcatgatgtcggcggctaagttcgggatgcatttgcaagcggcaactccgaagggttatgaacccgacgcctccgtgaccaagctggccgaacagtacgccaaggaaaacggaaccaagttgctgctgactaatgatcccctggaggcggcccacggggggaacgtgctgataaccgatacctggatctccatggggcaggaagaagagaagaaaaagcggctgcaggcattccagggataccaggtcaccatgaaaaccgcaaaagtggcagccagcgactggactttcctccattgcctgccgcgaaagccggaggaggtcgatgacgaggtgttctactccccgcggtcgctggtgttcccggaggcggaaaaccggaagtggaccattatggccgtgatggtgtcactcctgactgactacagcccgcaactgcagaagccgaagttctagctcgagctagtgactgactaggatctggttaccactaaaccagcctcaagaacacccgaatggagtctctaagctacataataccaacttacacttacaaaatgttgtcccccaaaatgtagccattcgtatctgctcctaataaaaagaaagtttcttcacattctag

SEQ ID NO: 61 - RNA, 1496 nt, synthetic construct
  source 1..1496: mol_type = other RNA
cttaagggggcgctgcctacggaggtggcagccatctccttctcggcatcaagcttaccatggtgccccaggccctgctcttggtcccgctgctggtgttccccctctgcttcggcaagttccccatctacaccatccccgacaagctggggccgtggagccccatcgacatccaccacctgtcctgccccaacaacctcgtggtcgaggacgagggctgcaccaacctgagcgggttctcctacatgcttttcaatctccgcatcctccttaacaacgccgcgtttagaaacggccacaacttcatggtccggaacttcagatgtggccagccgcttcaaaacaaggtccagctgaagggccgggatcttctgaccctgaagaactttactggcgaagagatcaagtacatgctctggctctccgcggacttgaagttccgcattaagcagaagggggaataccttccgctgcttcaaggaaagagcctcggcatgatctttgagaagcgctcaaccaggacccgcctttctactgaaactgggttcgcgctgctcggtggccacccctgcttcctgacgacccaggacatccacctcggagtgaacgaatccctcaccgataccgcccgggtgttatcgagcatggcagatgccgtgctggccagggtgtacaaacagtccgatctggacactctggccaaggaggcgtcaattcctattatcaacggccttagtgacctctaccatccgattcagatcctggccgattacctcaccctgcaagaacactacagctccctgaagggtctgacattgtcctggatcggcgacggcaacaacattctccattccatcatgatgtccgccgcaaaattcggcatgcatcttcaagccgccacgccgaagggttacgagcccgacgcttccgtgactaagctcgccgagcagtacgctaaggagaacggaaccaagcttctgctgactaacgacccactagaagcagcccacgggggcaacgtgcttattactgacacctggatctccatgggccaggaagaagagaaaaagaagcggctgcaggcgttccagggatatcaggtcaccatgaaaaccgccaaggtcgctgcctccgactggaccttcctgcactgcctgcctcgcaagcctgaagaagtggacgacgaggtgttctactcgccacggagcctcgtgttccccgaggccgagaatagaaagtggaccatcatggccgtgatggtgtcactgctcaccgactacagcccgcagcttcagaagcccaagttctagataagtgaatgcaaggctggccggaagcccttgcctgaaagcaagatttcagcctggaagagggcaaagtggacgggagtggacaggagtggatgcgataagatgtggtttgaagctgatgggtgccagccctgcattgctgagtcaatcaataaagagctttcttttgacccattctagatctag

SEQ ID NO: 62 - RNA, 1368 nt, synthetic construct
  source 1..1368: mol_type = other RNA
aggaaacttaagattattacatcaaaacaaaaagccgccaatgctgttcaacctgcgcatcctgctgaacaacgccgccttccgcaacggccacaacttcatggtgcgcaacttccgctgcggccagcccctgcagaacaaggtgcagctgaagggccgcgacctgctgaccctgaagaacttcaccggcgaggagatcaagtacatgctgtggctgagcgccgacctgaagttccgcatcaagcagaagggcgagtacctgcccctgctgcagggcaagagcctgggcatgatcttcgagaagcgcagcacccgcacccgcctgagcaccgagacaggcctggccctgctgggcggccacccctgcttcctgaccacccaggacatccacctgggcgtgaacgagagcctgaccgacaccgcccgcgtgctgagcagcatggccgacgccgtgctggcccgcgtgtacaagcagagcgacctggacaccctggccaaggaggccagcatccccatcatcaacggcctgagcgacctgtaccaccccatccagatcctggccgactacctgaccctgcaggagcactacagcagcctgaagggcctgaccctgagctggatcggcgacggcaacaacatcctgcacagcatcatgatgagcgccgccaagttcggcatgcacctgcaggccgccacccccaagggctacgagcccgacgccagcgtgaccaagctggccgagcagtacgccaaggagaacggcaccaagctgctgctgaccaacgaccccctggaggccgcccacggcggcaacgtgctgatcaccgacacctggatcagcatgggccaggaggaggagaagaagaagcgcctgcaggccttccagggctaccaggtgaccatgaagaccgccaaggtggccgccagcgactggaccttcctgcactgcctgccccgcaagcccgaggaggtggacgacgaggtgttctacagcccccgcagcctggtgttccccgaggccgagaaccgcaagtggaccatcatggccgtgatggtgagcctgctgaccgactacagcccccagctgcagaagcccaagttctgaacgccgaagcctgcagccatgcgaccccacgccaccccgtgcctcctgcctccgcgcagcctgcagcgggagaccctgtccccgccccagccgtcctcctggggtggaccctagtttaataaagattcaccaagtttcacgcaaaaaaaaaaaaaaaaaaaaaaaaaaaaaaaaaaaaaaaaaaaaaaaaaaaaaaaaaaaaaaaaaaaaaaaaaaaaaaaaaaaaaaaaaaaaaaaaaaaaaaaaaaaaaaaaaaaaaaaaa

SEQ ID NO: 63 - RNA, 1495 nt, synthetic construct
  source 1..1495: mol_type = other RNA
cttaagggggcgctgcctacggaggtggcagccatctccttctcggcatcaagcttaccatggtgccccaggccctgctcttggtcccgctgctggtgttccccctctgcttcggcaagttccccatctacaccatccccgacaagctggggccgtggagccccatcgacatccaccacctgtcctgccccaacaacctcgtggtcgaggacgagggctgcaccaacctgagcgggttctcctacatgctgttcaacctgcgcatcctgctgaacaacgccgccttccgcaacggccacaacttcatggtgcgcaacttccgctgcggccagcccctgcagaacaaggtgcagctgaagggccgcgacctgctgaccctgaagaacttcaccggcgaggagatcaagtacatgctgtggctgagcgccgacctgaagttccgcatcaagcagaagggcgagtacctgcccctgctgcagggcaagagcctgggcatgatcttcgagaagcgcagcacccgcacccgcctgagcaccgagacaggcctggccctgctgggcggccacccctgcttcctgaccacccaggacatccacctgggcgtgaacgagagcctgaccgacaccgcccgcgtgctgagcagcatggccgacgccgtgctggcccgcgtgtacaagcagagcgacctggacaccctggccaaggaggccagcatccccatcatcaacggcctgagcgacctgtaccaccccatccagatcctggccgactacctgaccctgcaggagcactacagcagcctgaagggcctgaccctgagctggatcggcgacggcaacaacatcctgcacagcatcatgatgagcgccgccaagttcggcatgcacctgcaggccgccacccccaagggctacgagcccgacgccagcgtgaccaagctggccgagcagtacgccaaggagaacggcaccaagctgctgctgaccaacgaccccctggaggccgcccacggcggcaacgtgctgatcaccgacacctggatcagcatgggccaggaggaggagaagaagaagcgcctgcaggccttccagggctaccaggtgaccatgaagaccgccaaggtggccgccagcgactggaccttcctgcactgcctgccccgcaagcccgaggaggtggacgacgaggtgttctacagcccccgcagcctggtgttccccgaggccgagaaccgcaagtggaccatcatggccgtgatggtgagcctgctgaccgactacagcccccagctgcagaagcccaagttctgaataagtgatgcaaggctggccggaagcccttgcctgaaagcaagatttcagcctggaagagggcaaagtggacgggagtggacaggagtggatgcgataagatgtggtttgaagctgatgggtgccagccctgcattgctgagtcaatcaataaagagctttcttttgacccattctagatctag

SEQ ID NO: 64 - RNA, 1368 nt, synthetic construct
  source 1..1368: mol_type = other RNA
aggaaacttaagattattacatcaaaacaaaaagccgccaatgcttttcaatctccgcatcctccttaacaacgccgcgtttagaaacggccacaacttcatggtccggaacttcagatgtggccagccgcttcaaaacaaggtccagctgaagggccgggatcttctgaccctgaagaactttactggcgaagagatcaagtacatgctctggctctccgcggacttgaagttccgcattaagcagaagggggaataccttccgctgcttcaaggaaagagcctcggcatgatctttgagaagcgctcaaccaggacccgcctttctactgaaactgggttcgcgctgctcggtggccacccctgcttcctgacgacccaggacatccacctcggagtgaacgaatccctcaccgataccgcccgggtgttatcgagcatggcagatgccgtgctggccagggtgtacaaacagtccgatctggacactctggccaaggaggcgtcaattcctattatcaacggccttagtgacctctaccatccgattcagatcctggccgattacctcaccctgcaagaacactacagctccctgaagggtctgacattgtcctggatcggcgacggcaacaacattctccattccatcatgatgtccgccgcaaaattcggcatgcatcttcaagccgccacgccgaagggttacgagcccgacgcttccgtgactaagctcgccgagcagtacgctaaggagaacggaaccaagcttctgctgactaacgacccactagaagcagcccacgggggcaacgtgcttattactgacacctggatctccatgggccaggaagaagagaaaaagaagcggctgcaggcgttccagggatatcaggtcaccatgaaaaccgccaaggtcgctgcctccgactggaccttcctgcactgcctgcctcgcaagcctgaagaagtggacgacgaggtgttctactcgccacggagcctcgtgttccccgaggccgagaatagaaagtggaccatcatggccgtgatggtgtcactgctcaccgactacagcccgcagcttcagaagcccaagttctagacgccgaagcctgcagccatgcgaccccacgccaccccgtgcctcctgcctccgcgcagcctgcagcgggagaccctgtccccgccccagccgtcctcctggggtggaccctagtttaataaagattcaccaagtttcacgcaaaaaaaaaaaaaaaaaaaaaaaaaaaaaaaaaaaaaaaaaaaaaaaaaaaaaaaaaaaaaaaaaaaaaaaaaaaaaaaaaaaaaaaaaaaaaaaaaaaaaaaaaaaaaaaaaaaaaaaaa

SEQ ID NO: 65 - RNA, 1495 nt, synthetic construct
  source 1..1495: mol_type = other RNA
cttaagggggcgctgcctacggaggtggcagccatctccttctcggcatcaagcttaccatggtgccccaggccctgctcttggtcccgctgctggtgttccccctctgcttcggcaagttccccatctacaccatccccgacaagctggggccgtggagccccatcgacatccaccacctgtcctgccccaacaacctcgtggtcgaggacgagggctgcaccaacctgagcgggttctcctacatgcttttcaacctgagaatcctcttgaacaatgctgcttttcggaatggccacaactttatggttcggaacttccgttgcggccagcctttacaaaacaaggtccagctgaagggccgggatttgctcacactaaagaactttactggagaagagatcaagtacatgctatggctgtcggccgacctgaagttccgtatcaagcagaagggagaataccttccgctgcttcaaggaaagagcctcggcatgatctttgagaagcgctcaaccaggacccgcctttctactgaaactgggttcgcgctgctcggtggccacccctgcttcctgacgacccaggacatccacctcggagtgaacgaatccctcaccgataccgcccgggtgttatcgagcatggcagatgccgtgctggccagggtgtacaaacagtccgatctcgataccttggcaaaggaggcttccattcccatcatcaacggcctgagcgacctgtaccacccaatccaaatcctggctgactacctgaccctgcaagagcactacagcagcctgaagggtctgaccctgtcatggattggcgatggaaacaatattctgcactccatcatgatgtccgccgcgaagttcggaatgcatctgcaagccgccactccaaaaggatacgaaccggatgcatccgtgaccaagttggcggaacagtacgcgaaggagaacggaaccaagctcctgctgactaacgacccgctcgaggctgcgcatgggggtaacgtgctgattacggacacctggatctccatggggcaggaggaagagaagaagaagagactgcaggcattccaggggtaccaggtcaccatgaaaaccgcaaaagtggcagcttcggactggactttcctgcattgcctgccgaggaagccggaggaagtcgacgacgaagtgttctactcgcctcggtccctggtgttccccgaggccgaaaaccggaagtggaccatcatggccgtgatggtgtccttgctgactgactatagcccgcagctgcagaagcctaagttctagataagtgatgcaaggctggccggaagcccttgcctgaaagcaagatttcagcctggaagagggcaaagtggacgggagtggacaggagtggatgcgataagatgtggtttgaagctgatgggtgccagccctgcattgctgagtcaatcaataaagagctttcttttgacccattctagatctag

SEQ ID NO: 66 - RNA, 1475 nt, synthetic construct
  source 1..1475: mol_type = other RNA
tgagtgtcgtacagcctccaggcccccccctcccgggagagccatagtggtctgcggaaccggtgagtacaccggaattgccgggaagactgggtcctttcttggataaacccactctatgcccggccatttgggcgtgcccccgcaagactgctagccgagtagtgttgggttgcgatgctgttcaacctgcgcatcctgctgaacaacgccgccttccgcaacggccacaacttcatggtgcgcaacttccgctgcggccagcccctgcagaacaaggtgcagctgaagggccgcgacctgctgaccctgaagaacttcaccggcgaggagatcaagtacatgctgtggctgagcgccgacctgaagttccgcatcaagcagaagggcgagtacctgcccctgctgcagggcaagagcctgggcatgatcttcgagaagcgcagcacccgcacccgcctgagcaccgagacaggcctggccctgctgggcggccacccctgcttcctgaccacccaggacatccacctgggcgtgaacgagagcctgaccgacaccgcccgcgtgctgagcagcatggccgacgccgtgctggcccgcgtgtacaagcagagcgacctggacaccctggccaaggaggccagcatccccatcatcaacggcctgagcgacctgtaccaccccatccagatcctggccgactacctgaccctgcaggagcactacagcagcctgaagggcctgaccctgagctggatcggcgacggcaacaacatcctgcacagcatcatgatgagcgccgccaagttcggcatgcacctgcaggccgccacccccaagggctacgagcccgacgccagcgtgaccaagctggccgagcagtacgccaaggagaacggcaccaagctgctgctgaccaacgaccccctggaggccgcccacggcggcaacgtgctgatcaccgacacctggatcagcatgggccaggaggaggagaagaagaagcgcctgcaggccttccagggctaccaggtgaccatgaagaccgccaaggtggccgccagcgactggaccttcctgcactgcctgccccgcaagcccgaggaggtggacgacgaggtgttctacagcccccgcagcctggtgttccccgaggccgagaaccgcaagtggaccatcatggccgtgatggtgagcctgctgaccgactacagcccccagctgcagaagcccaagttctgaataagtgatagagcggcaaaccctagctacactccatagctagtttcttttttttttgtttttttttttttttttttttttttttttttttttttttcctttcttttccttctttttttcctcttttcttggtggctccatcttagccctagtcacggctagctgtgaaaggtccgtgagccgcatgactgcagagagtgccgtaactggcctctctgcagatcatgttctag

SEQ ID NO: 67 - RNA, 1335 nt, synthetic construct
  source 1..1335: mol_type = other RNA
aggaaacttaagattattacatcaaaacaaaaagccgccaatgcttttcaatctccgcatcctccttaacaacgccgcgtttagaaacggccacaacttcatggtccggaacttcagatgtggccagccgcttcaaaacaaggtccagctgaagggccgggatcttctgaccctgaagaactttactggcgaagagatcaagtacatgctctggctctccgcggacttgaagttccgcattaagcagaagggggaataccttccgctgcttcaaggaaagagcctcggcatgatctttgagaagcgctcaaccaggacccgcctttctactgaaactgggttcgcgctgctcggtggccacccctgcttcctgacgacccaggacatccacctcggagtgaacgaatccctcaccgataccgcccgggtgttatcgagcatggcagatgccgtgctggccagggtgtacaaacagtccgatctggacactctggccaaggaggcgtcaattcctattatcaacggccttagtgacctctaccatccgattcagatcctggccgattacctcaccctgcaagaacactacagctccctgaagggtctgacattgtcctggatcggcgacggcaacaacattctccattccatcatgatgtccgccgcaaaattcggcatgcatcttcaagccgccacgccgaagggttacgagcccgacgcttccgtgactaagctcgccgagcagtacgctaaggagaacggaaccaagcttctgctgactaacgacccactagaagcagcccacgggggcaacgtgcttattactgacacctggatctccatgggccaggaagaagagaaaaagaagcggctgcaggcgttccagggatatcaggtcaccatgaaaaccgccaaggtcgctgcctccgactggaccttcctgcactgcctgcctcgcaagcctgaagaagtggacgacgaggtgttctactcgccacggagcctcgtgttccccgaggccgagaatagaaagtggaccatcatggccgtgatggtgtcactgctcaccgactacagcccgcagcttcagaagcccaagttctaggctggagcctcggtagccgttcctcctgcccgctgggcctcccaacgggccctcctcccctccttgcaccggcccttcctggtctttgaataaagtctgagtgggcagcaaaaaaaaaaaaaaaaaaaaaaaaaaaaaaaaaaaaaaaaaaaaaaaaaaaaaaaaaaaaaaaaaaaaaaaaaaaaaaaaaaaaaaaaaaaaaaaaaaaaaaaaaaaaaaaaaaaaaaaaa

SEQ ID NO: 68 - RNA, 1335 nt, synthetic construct
  source 1..1335: mol_type = other RNA
aggaaacttaagattattacatcaaaacaaaaagccgccaatgctgttcaacctgcgcatcctgctgaacaacgccgccttccgcaacggccacaacttcatggtgcgcaacttccgctgcggccagcccctgcagaacaaggtgcagctgaagggccgcgacctgctgaccctgaagaacttcaccggcgaggagatcaagtacatgctgtggctgagcgccgacctgaagttccgcatcaagcagaagggcgagtacctgcccctgctgcagggcaagagcctgggcatgatcttcgagaagcgcagcacccgcacccgcctgagcaccgagacaggcctggccctgctgggcggccacccctgcttcctgaccacccaggacatccacctgggcgtgaacgagagcctgaccgacaccgcccgcgtgctgagcagcatggccgacgccgtgctggcccgcgtgtacaagcagagcgacctggacaccctggccaaggaggccagcatccccatcatcaacggcctgagcgacctgtaccaccccatccagatcctggccgactacctgaccctgcaggagcactacagcagcctgaagggcctgaccctgagctggatcggcgacggcaacaacatcctgcacagcatcatgatgagcgccgccaagttcggcatgcacctgcaggccgccacccccaagggctacgagcccgacgccagcgtgaccaagctggccgagcagtacgccaaggagaacggcaccaagctgctgctgaccaacgaccccctggaggccgcccacggcggcaacgtgctgatcaccgacacctggatcagcatgggccaggaggaggagaagaagaagcgcctgcaggccttccagggctaccaggtgaccatgaagaccgccaaggtggccgccagcgactggaccttcctgcactgcctgccccgcaagcccgaggaggtggacgacgaggtgttctacagcccccgcagcctggtgttccccgaggccgagaaccgcaagtggaccatcatggccgtgatggtgagcctgctgaccgactacagcccccagctgcagaagcccaagttctgagctggagcctcggtagccgttcctcctgcccgctgggcctcccaacgggccctcctcccctccttgcaccggcccttcctggtctttgaataaagtctgagtgggcagcaaaaaaaaaaaaaaaaaaaaaaaaaaaaaaaaaaaaaaaaaaaaaaaaaaaaaaaaaaaaaaaaaaaaaaaaaaaaaaaaaaaaaaaaaaaaaaaaaaaaaaaaaaaaaaaaaaaaaaaaa

SEQ ID NO: 69 - RNA, 1335 nt, synthetic construct
  source 1..1335: mol_type = other RNA
aggaaacttaagattattacatcaaaacaaaaagccgccaatgcttttcaacctgagaatcctcttgaacaatgctgcttttcggaatggccacaactttatggttcggaacttccgttgcggccagcctttacaaaacaaggtccagctgaagggccgggatttgctcacactaaagaactttactggagaagagatcaagtacatgctatggctgtcggccgacctgaagttccgtatcaagcagaagggagaataccttccgctgcttcaaggaaagagcctcggcatgatctttgagaagcgctcaaccaggacccgcctttctactgaaactgggttcgcgctgctcggtggccacccctgcttcctgacgacccaggacatccacctcggagtgaacgaatccctcaccgataccgcccgggtgttatcgagcatggcagatgccgtgctggccagggtgtacaaacagtccgatctcgataccttggcaaaggaggcttccattcccatcatcaacggcctgagcgacctgtaccacccaatccaaatcctggctgactacctgaccctgcaagagcactacagcagcctgaagggtctgaccctgtcatggattggcgatggaaacaatattctgcactccatcatgatgtccgccgcgaagttcggaatgcatctgcaagccgccactccaaaaggatacgaaccggatgcatccgtgaccaagttggcggaacagtacgcgaaggagaacggaaccaagctcctgctgactaacgacccgctcgaggctgcgcatgggggtaacgtgctgattacggacacctggatctccatggggcaggaggaagagaagaagaagagactgcaggcattccaggggtaccaggtcaccatgaaaaccgcaaaagtggcagcttcggactggactttcctgcattgcctgccgaggaagccggaggaagtcgacgacgaagtgttctactcgcctcggtccctggtgttccccgaggccgaaaaccggaagtggaccatcatggccgtgatggtgtccttgctgactgactatagcccgcagctgcagaagcctaagttctaggctggagcctcggtagccgttcctcctgcccgctgggcctcccaacgggccctcctcccctccttgcaccggcccttcctggtctttgaataaagtctgagtgggcagcaaaaaaaaaaaaaaaaaaaaaaaaaaaaaaaaaaaaaaaaaaaaaaaaaaaaaaaaaaaaaaaaaaaaaaaaaaaaaaaaaaaaaaaaaaaaaaaaaaaaaaaaaaaaaaaaaaaaaaaaa

SEQ ID NO: 70 - RNA, 1346 nt, synthetic construct
  source 1..1346: mol_type = other RNA
aggaaacttaagaattattggttaaagaagtatattagtgctaatttccctccgtttgtcctagcttttctcttctgtcaaccccacacgcctttggcacaatgcttttcaatctccgcatcctccttaacaacgccgcgtttagaaacggccacaacttcatggtccggaacttcagatgtggccagccgcttcaaaacaaggtccagctgaagggccgggatcttctgaccctgaagaactttactggcgaagagatcaagtacatgctctggctctccgcggacttgaagttccgcattaagcagaagggggaataccttccgctgcttcaaggaaagagcctcggcatgatctttgagaagcgctcaaccaggacccgcctttctactgaaactgggttcgcgctgctcggtggccacccctgcttcctgacgacccaggacatccacctcggagtgaacgaatccctcaccgataccgcccgggtgttatcgagcatggcagatgccgtgctggccagggtgtacaaacagtccgatctggacactctggccaaggaggcgtcaattcctattatcaacggccttagtgacctctaccatccgattcagatcctggccgattacctcaccctgcaagaacactacagctccctgaagggtctgacattgtcctggatcggcgacggcaacaacattctccattccatcatgatgtccgccgcaaaattcggcatgcatcttcaagccgccacgccgaagggttacgagcccgacgcttccgtgactaagctcgccgagcagtacgctaaggagaacggaaccaagcttctgctgactaacgacccactagaagcagcccacgggggcaacgtgcttattactgacacctggatctccatgggccaggaagaagagaaaaagaagcggctgcaggcgttccagggatatcaggtcaccatgaaaaccgccaaggtcgctgcctccgactggaccttcctgcactgcctgcctcgcaagcctgaagaagtggacgacgaggtgttctactcgccacggagcctcgtgttccccgaggccgagaatagaaagtggaccatcatggccgtgatggtgtcactgctcaccgactacagcccgcagcttcagaagcccaagttctagctcgagacacatcacaaccacaaccttctcaggctaccctgagaaaaaaagacatgaagactcaggactcatcttttctgttggtgtaaaatcaacaccctaaggaacacaaatttctttaaacatttgacttcttgtctctgtgctgcaattaataaaaaatggaaagaatctatctag

SEQ ID NO: 71 - RNA, 1346 nt, synthetic construct
  source 1..1346: mol_type = other RNA
aggaaacttaagaattattggttaaagaagtatattagtgctaatttccctccgtttgtcctagcttttctcttctgtcaaccccacacgcctttggcacaatgctgttcaacctgcgcatcctgctgaacaacgccgccttccgcaacggccacaacttcatggtgcgcaacttccgctgcggccagcccctgcagaacaaggtgcagctgaagggccgcgacctgctgaccctgaagaacttcaccggcgaggagatcaagtacatgctgtggctgagcgccgacctgaagttccgcatcaagcagaagggcgagtacctgcccctgctgcagggcaagagcctgggcatgatcttcgagaagcgcagcacccgcacccgcctgagcaccgagacaggcctggccctgctgggcggccacccctgcttcctgaccacccaggacatccacctgggcgtgaacgagagcctgaccgacaccgcccgcgtgctgagcagcatggccgacgccgtgctggcccgcgtgtacaagcagagcgacctggacaccctggccaaggaggccagcatccccatcatcaacggcctgagcgacctgtaccaccccatccagatcctggccgactacctgaccctgcaggagcactacagcagcctgaagggcctgaccctgagctggatcggcgacggcaacaacatcctgcacagcatcatgatgagcgccgccaagttcggcatgcacctgcaggccgccacccccaagggctacgagcccgacgccagcgtgaccaagctggccgagcagtacgccaaggagaacggcaccaagctgctgctgaccaacgaccccctggaggccgcccacggcggcaacgtgctgatcaccgacacctggatcagcatgggccaggaggaggagaagaagaagcgcctgcaggccttccagggctaccaggtgaccatgaagaccgccaaggtggccgccagcgactggaccttcctgcactgcctgccccgcaagcccgaggaggtggacgacgaggtgttctacagcccccgcagcctggtgttccccgaggccgagaaccgcaagtggaccatcatggccgtgatggtgagcctgctgaccgactacagcccccagctgcagaagcccaagttctgactcgagacacatcacaaccacaaccttctcaggctaccctgagaaaaaaagacatgaagactcaggactcatcttttctgttggtgtaaaatcaacaccctaaggaacacaaatttctttaaacatttgacttcttgtctctgtgctgcaattaataaaaaatggaaagaatctatctag

SEQ ID NO: 72 - RNA, 1346 nt, synthetic construct
  source 1..1346: mol_type = other RNA
aggaaacttaagaattattggttaaagaagtatattagtgctaatttccctccgtttgtcctagcttttctcttctgtcaaccccacacgcctttggcacaatgcttttcaacctgagaatcctcttgaacaatgctgcttttcggaatggccacaactttatggttcggaacttccgttgcggccagcctttacaaaacaaggtccagctgaagggccgggatttgctcacactaaagaactttactggagaagagatcaagtacatgctatggctgtcggccgacctgaagttccgtatcaagcagaagggagaataccttccgctgcttcaaggaaagagcctcggcatgatctttgagaagcgctcaaccaggacccgcctttctactgaaactgggttcgcgctgctcggtggccacccctgcttcctgacgacccaggacatccacctcggagtgaacgaatccctcaccgataccgcccgggtgttatcgagcatggcagatgccgtgctggccagggtgtacaaacagtccgatctcgataccttggcaaaggaggcttccattcccatcatcaacggcctgagcgacctgtaccacccaatccaaatcctggctgactacctgaccctgcaagagcactacagcagcctgaagggtctgaccctgtcatggattggcgatggaaacaatattctgcactccatcatgatgtccgccgcgaagttcggaatgcatctgcaagccgccactccaaaaggatacgaaccggatgcatccgtgaccaagttggcggaacagtacgcgaaggagaacggaaccaagctcctgctgactaacgacccgctcgaggctgcgcatgggggtaacgtgctgattacggacacctggatctccatggggcaggaggaagagaagaagaagagactgcaggcattccaggggtaccaggtcaccatgaaaaccgcaaaagtggcagcttcggactggactttcctgcattgcctgccgaggaagccggaggaagtcgacgacgaagtgttctactcgcctcggtccctggtgttccccgaggccgaaaaccggaagtggaccatcatggccgtgatggtgtccttgctgactgactatagcccgcagctgcagaagcctaagttctagctcgagacacatcacaaccacaaccttctcaggctaccctgagaaaaaaagacatgaagactcaggactcatcttttctgttggtgtaaaatcaacaccctaaggaacacaaatttctttaaacatttgacttcttgtctctgtgctgcaattaataaaaaatggaaagaatctatctag

SEQ ID NO: 73 - RNA, 1222 nt, synthetic construct
  source 1..1222: mol_type = other RNA
attattacatcaaaacaaaaagccgccaccatgctgttcaacctgcgcatcctgctgaacaacgccgccttccgcaacggccacaacttcatggtgcgcaacttccgctgcggccagcccctgcagaacaaggtgcagctgaagggccgcgacctgctgaccctgaagaacttcaccggcgaggagatcaagtacatgctgtggctgagcgccgacctgaagttccgcatcaagcagaagggcgagtacctgcccctgctgcagggcaagagcctgggcatgatcttcgagaagcgcagcacccgcacccgcctgagcaccgagacaggcttcgccctgctgggcggccacccctgcttcctgaccacccaggacatccacctgggcgtgaacgagagcctgaccgacaccgcccgcgtgctgagcagcatggccgacgccgtgctggcccgcgtgtacaagcagagcgacctggacaccctggccaaggaggccagcatccccatcatcaacggcctgagcgacctgtaccaccccatccagatcctggccgactacctgaccctgcaggagcactacagcagcctgaagggcctgaccctgagctggatcggcgacggcaacaacatcctgcacagcatcatgatgagcgccgccaagttcggcatgcacctgcaggccgccacccccaagggctacgagcccgacgccagcgtgaccaagctggccgagcagtacgccaaggagaacggcaccaagctgctgctgaccaacgaccccctggaggccgcccacggcggcaacgtgctgatcaccgacacctggatcagcatgggccaggaggaggagaagaagaagcgcctgcaggccttccagggctaccaggtgaccatgaagaccgccaaggtggccgccagcgactggaccttcctgcactgcctgccccgcaagcccgaggaggtggacgacgaggtgttctacagcccccgcagcctggtgttccccgaggccgagaaccgcaagtggaccatcatggccgtgatggtgagcctgctgaccgactacagcccccagctgcagaagcccaagttctgaggtctctagtaatgagctggagcctcggtagccgttcctcctgcccgctgggcctcccaacgggccctcctcccctccttgcaccggcccttcctggtctttgaataaagtctgagtgggcatctag

SEQ ID NO: 74 - RNA, 1346 nt, synthetic construct
  source 1..1346: mol_type = other RNA
aggaaacttaagaattattggttaaagaagtatattagtgctaatttccctccgtttgtcctagcttttctcttctgtcaaccccacacgcctttggcacaatgctgttcaacctgcgcatcctgctgaacaacgccgccttccgcaacggccacaacttcatggtgcgcaacttccgctgcggccagcccctgcagaacaaggtgcagctgaagggccgcgacctgctgaccctgaagaacttcaccggcgaggagatcaagtacatgctgtggctgagcgccgacctgaagttccgcatcaagcagaagggcgagtacctgcccctgctgcagggcaagagcctgggcatgatcttcgagaagcgcagcacccgcacccgcctgagcaccgagacaggcttcgccctgctgggcggccacccctgcttcctgaccacccaggacatccacctgggcgtgaacgagagcctgaccgacaccgcccgcgtgctgagcagcatggccgacgccgtgctggcccgcgtgtacaagcagagcgacctggacaccctggccaaggaggccagcatccccatcatcaacggcctgagcgacctgtaccaccccatccagatcctggccgactacctgaccctgcaggagcactacagcagcctgaagggcctgaccctgagctggatcggcgacggcaacaacatcctgcacagcatcatgatgagcgccgccaagttcggcatgcacctgcaggccgccacccccaagggctacgagcccgacgccagcgtgaccaagctggccgagcagtacgccaaggagaacggcaccaagctgctgctgaccaacgaccccctggaggccgcccacggcggcaacgtgctgatcaccgacacctggatcagcatgggccaggaggaggagaagaagaagcgcctgcaggccttccagggctaccaggtgaccatgaagaccgccaaggtggccgccagcgactggaccttcctgcactgcctgccccgcaagcccgaggaggtggacgacgaggtgttctacagcccccgcagcctggtgttccccgaggccgagaaccgcaagtggaccatcatggccgtgatggtgagcctgctgaccgactacagcccccagctgcagaagcccaagttctgactcgagacacatcacaaccacaaccttctcaggctaccctgagaaaaaaagacatgaagactcaggactcatcttttctgttggtgtaaaatcaacaccctaaggaacacaaatttctttaaacatttgacttcttgtctctgtgctgcaattaataaaaaatggaaagaatctatctag

SEQ ID NO: 75 - RNA, 1368 nt, synthetic construct
  source 1..1368: mol_type = other RNA
aggaaacttaagattattacatcaaaacaaaaagccgccaatgctgttcaacctgcgcatcctgctgaacaacgccgccttccgcaacggccacaacttcatggtgcgcaacttccgctgcggccagcccctgcagaacaaggtgcagctgaagggccgcgacctgctgaccctgaagaacttcaccggcgaggagatcaagtacatgctgtggctgagcgccgacctgaagttccgcatcaagcagaagggcgagtacctgcccctgctgcagggcaagagcctgggcatgatcttcgagaagcgcagcacccgcacccgcctgagcaccgagacaggcttcgccctgctgggcggccacccctgcttcctgaccacccaggacatccacctgggcgtgaacgagagcctgaccgacaccgcccgcgtgctgagcagcatggccgacgccgtgctggcccgcgtgtacaagcagagcgacctggacaccctggccaaggaggccagcatccccatcatcaacggcctgagcgacctgtaccaccccatccagatcctggccgactacctgaccctgcaggagcactacagcagcctgaagggcctgaccctgagctggatcggcgacggcaacaacatcctgcacagcatcatgatgagcgccgccaagttcggcatgcacctgcaggccgccacccccaagggctacgagcccgacgccagcgtgaccaagctggccgagcagtacgccaaggagaacggcaccaagctgctgctgaccaacgaccccctggaggccgcccacggcggcaacgtgctgatcaccgacacctggatcagcatgggccaggaggaggagaagaagaagcgcctgcaggccttccagggctaccaggtgaccatgaagaccgccaaggtggccgccagcgactggaccttcctgcactgcctgccccgcaagcccgaggaggtggacgacgaggtgttctacagcccccgcagcctggtgttccccgaggccgagaaccgcaagtggaccatcatggccgtgatggtgagcctgctgaccgactacagcccccagctgcagaagcccaagttctgaacgccgaagcctgcagccatgcgaccccacgccaccccgtgcctcctgcctccgcgcagcctgcagcgggagaccctgtccccgccccagccgtcctcctggggtggaccctagtttaataaagattcaccaagtttcacgcaaaaaaaaaaaaaaaaaaaaaaaaaaaaaaaaaaaaaaaaaaaaaaaaaaaaaaaaaaaaaaaaaaaaaaaaaaaaaaaaaaaaaaaaaaaaaaaaaaaaaaaaaaaaaaaaaaaaaaaaa

SEQ ID NO: 76 - RNA, 1496 nt, synthetic construct
  source 1..1496: mol_type = other RNA
cttaagggggcgctgcctacggaggtggcagccatctccttctcggcatcaagcttaccatggtgccccaggccctgctcttggtcccgctgctggtgttccccctctgcttcggcaagttccccatctacaccatccccgacaagctggggccgtggagccccatcgacatccaccacctgtcctgccccaacaacctcgtggtcgaggacgagggctgcaccaacctgagcgggttctcctacatgctgttcaacctgcgcatcctgctgaacaacgccgccttccgcaacggccacaacttcatggtgcgcaacttccgctgcggccagcccctgcagaacaaggtgcagctgaagggccgcgacctgctgaccctgaagaacttcaccggcgaggagatcaagtacatgctgtggctgagcgccgacctgaagttccgcatcaagcagaagggcgagtacctgcccctgctgcagggcaagagcctgggcatgatcttcgagaagcgcagcacccgcacccgcctgagcaccgagacaggcttcgccctgctgggcggccacccctgcttcctgaccacccaggacatccacctgggcgtgaacgagagcctgaccgacaccgcccgcgtgctgagcagcatggccgacgccgtgctggcccgcgtgtacaagcagagcgacctggacaccctggccaaggaggccagcatccccatcatcaacggcctgagcgacctgtaccaccccatccagatcctggccgactacctgaccctgcaggagcactacagcagcctgaagggcctgaccctgagctggatcggcgacggcaacaacatcctgcacagcatcatgatgagcgccgccaagttcggcatgcacctgcaggccgccacccccaagggctacgagcccgacgccagcgtgaccaagctggccgagcagtacgccaaggagaacggcaccaagctgctgctgaccaacgaccccctggaggccgcccacggcggcaacgtgctgatcaccgacacctggatcagcatgggccaggaggaggagaagaagaagcgcctgcaggccttccagggctaccaggtgaccatgaagaccgccaaggtggccgccagcgactggaccttcctgcactgcctgccccgcaagcccgaggaggtggacgacgaggtgttctacagcccccgcagcctggtgttccccgaggccgagaaccgcaagtggaccatcatggccgtgatggtgagcctgctgaccgactacagcccccagctgcagaagcccaagttctgaataagtgaatgcaaggctggccggaagcccttgcctgaaagcaagatttcagcctggaagagggcaaagtggacgggagtggacaggagtggatgcgataagatgtggtttgaagctgatgggtgccagccctgcattgctgagtcaatcaataaagagctttcttttgacccattctagatctag

SEQ ID NO: 77 - RNA, 1380 nt, synthetic construct
  source 1..1380: mol_type = other RNA
tcaacacaacatatacaaaacaaacgaatctcaagcaatcaagcattctacttctattgcagcaatttaaatcatttcttttaaagcaaaagcaattttctgaaaattttcaccatttacgaacgatagccaccatgggcgtcttcaacctgcggatcctgctgaacaacgccgccttccggaacggccacaacttcatggtccgcaacttcagatgcggccagcccctgcagaacaaggtgcagctgaagggccgggacctgctgaccctgaagaacttcaccggcgaagagatcaagtacatgctgtggctgagcgccgacctgaagttccggatcaagcagaagggcgagtacctgcccctgctgcaaggcaagagcctgggcatgatcttcgagaagcggagcacccggacccggctgagcaccgagacaggctttgccctgctgggaggccacccctgctttctgaccacccaggacatccacctgggcgtgaacgagagcctgaccgacaccgccagagtgctgagcagcatggccgacgccgtgctggcccgggtgtacaagcagagcgacctggacaccctggccaaagaggccagcatccccatcatcaacggcctgagcgacctgtaccaccccatccagatcctggccgactacctgaccctgcaggaacactacagctccctgaagggcctgaccctgagctggatcggcgacggcaacaacatcctgcacagcatcatgatgagcgccgccaagttcggcatgcatctgcaggccgccacccccaagggctacgagcctgatgccagcgtgaccaagctggccgagcagtacgccaaagagaacggcaccaagctgctgctgaccaacgaccccctggaagccgcccacggcggcaacgtgctgatcaccgacacctggatcagcatgggccaggaagaggaaaagaagaagcggctgcaggccttccagggctaccaggtcacaatgaagaccgccaaggtggccgccagcgactggaccttcctgcactgcctgccccggaagcccgaagaggtggacgacgaggtgttctacagcccccggtccctggtgttccccgaggccgagaaccggaagtggaccattatggccgtgatggtgtccctgctgaccgactactccccccagctgcagaagcccaagttctagataagtgaactcgagctagtgactgactaggatctggttaccactaaaccagcctcaagaacacccgaatggagtctctaagctacataataccaacttacacttacaaaatgttgtcccccaaaatgtagccattcgtatctgctcctaataaaaagaaagtttcttcacattctag

SEQ ID NO: 78 - RNA, 1380 nt, synthetic construct
  source 1..1380: mol_type = other RNA
tcaacacaacatatacaaaacaaacgaatctcaagcaatcaagcattctacttctattgcagcaatttaaatcatttcttttaaagcaaaagcaattttctgaaaattttcaccatttacgaacgatagccaccatgggcgtcttcaacctgcggatcctgctgaacaacgccgccttccggaacggccacaacttcatggtccgcaacttcagatgcggccagcccctgcagaacagggtgcagctgaagggccgggacctgctgaccctgaagaacttcaccggcgaagagatcaggtacatgctgtggctgagcgccgacctgaagttccggatcaagcagaagggcgagtacctgcccctgctgcaaggcaagagcctgggcatgatcttcgagaagcggagcacccggacccggctgagcaccgagacaggctttgccctgctgggaggccacccctgctttctgaccacccaggacatccacctgggcgtgaacgagagcctgaccgacaccgccagagtgctgagcagcatggccgacgccgtgctggcccgggtgtacaagcagagcgacctggacaccctggccaaagaggccagcatccccatcatcaacggcctgagcgacctgtaccaccccatccagatcctggccgactacctgaccctgcaggaacactacagctccctgaagggcctgaccctgagctggatcggcgacggcaacaacatcctgcacagcatcatgatgagcgccgccaagttcggcatgcatctgcaggccgccacccccaagggctacgagcctgatgccagcgtgaccaagctggccgagcagtacgccaaagagaacggcaccaagctgctgctgaccaacgaccccctggaagccgcccacggcggcaacgtgctgatcaccgacacctggatcagcatgggccaggaagaggaaaagaagaagcggctgcaggccttccagggctaccaggtcacaatgaagaccgccaaggtggccgccagcgactggaccttcctgcactgcctgccccggaagcccgaagaggtggacgacgaggtgttctacagcccccggtccctggtgttccccgaggccgagaaccggaagtggaccattatggccgtgatggtgtccctgctgaccgactactccccccagctgcagaagcccaagttctagataagtgaactcgagctagtgactgactaggatctggttaccactaaaccagcctcaagaacacccgaatggagtctctaagctacataataccaacttacacttacaaaatgttgtcccccaaaatgtagccattcgtatctgctcctaataaaaagaaagtttcttcacattctag

SEQ ID NO: 79 - RNA, 1380 nt, synthetic construct
  source 1..1380: mol_type = other RNA
tcaacacaacatatacaaaacaaacgaatctcaagcaatcaagcattctacttctattgcagcaatttaaatcatttcttttaaagcaaaagcaattttctgaaaattttcaccatttacgaacgatagccaccatgctggtcttcaacctgcggatcctgctgaacaacgccgccttccggaacggccacaacttcatggtccgcaacttcagatgcggccagcccctgcagaacagggtgcagctgaagggccgggacctgctgaccctgaagaacttcaccggcgaagagatcaggtacatgctgtggctgagcgccgacctgaagttccggatcaagcagaagggcgagtacctgcccctgctgcaaggcaagagcctgggcatgatcttcgagaagcggagcacccggacccggctgagcaccgagacaggctttgccctgctgggaggccacccctgctttctgaccacccaggacatccacctgggcgtgaacgagagcctgaccgacaccgccagagtgctgagcagcatggccgacgccgtgctggcccgggtgtacaagcagagcgacctggacaccctggccaaagaggccagcatccccatcatcaacggcctgagcgacctgtaccaccccatccagatcctggccgactacctgaccctgcaggaacactacagctccctgaagggcctgaccctgagctggatcggcgacggcaacaacatcctgcacagcatcatgatgagcgccgccaagttcggcatgcatctgcaggccgccacccccaagggctacgagcctgatgccagcgtgaccaagctggccgagcagtacgccaaagagaacggcaccaagctgctgctgaccaacgaccccctggaagccgcccacggcggcaacgtgctgatcaccgacacctggatcagcatgggccaggaagaggaaaagaagaagcggctgcaggccttccagggctaccaggtcacaatgaagaccgccaaggtggccgccagcgactggaccttcctgcactgcctgccccggaagcccgaagaggtggacgacgaggtgttctacagcccccggtccctggtgttccccgaggccgagaaccggaagtggaccattatggccgtgatggtgtccctgctgaccgactactccccccagctgcagaagcccaagttctagataagtgaactcgagctagtgactgactaggatctggttaccactaaaccagcctcaagaacacccgaatggagtctctaagctacataataccaacttacacttacaaaatgttgtcccccaaaatgtagccattcgtatctgctcctaataaaaagaaagtttcttcacattctag

SEQ ID NO: 80 - RNA, 1377 nt, synthetic construct
  source 1..1377: mol_type = other RNA
tcaacacaacatatacaaaacaaacgaatctcaagcaatcaagcattctacttctattgcagcaatttaaatcatttcttttaaagcaaaagcaattttctgaaaattttcaccatttacgaacgatagccaccatgctgttcaacctgaggatcctgctgaacaacgcagctttcaggaacggccacaacttcatggtgaggaacttccggtgcggccagcccctgcagaacaaggtgcagctgaagggcagggacctgctgaccctgaagaacttcaccggagaggagatcaagtacatgctgtggctgagcgcagacctgaagttcaggatcaagcagaagggagagtacctgcccctgctgcaggggaagtccctgggcatgatcttcgagaagaggagtaccaggaccaggctgagcaccgaaaccggcttcgccctgctgggaggacacccctgcttcctgaccacccaggacatccacctgggcgtgaacgagagtctgaccgacaccgccagggtgctgtctagcatggccgacgccgtgctggccagggtgtacaagcagtcagacctggacaccctggctaaggaggccagcatccccatcatcaacggcctgagcgacctgtaccaccccatccagatcctggctgactacctgaccctgcaggagcactacagctctctgaagggcctgaccctgagctggatcggcgacgggaacaacatcctgcacagcatcatgatgagcgccgccaagttcggcatgcacctgcaggccgctacccccaagggttacgagcccgacgccagcgtgaccaagctggcagagcagtacgccaaggagaacggcaccaagctgctgctgaccaacgaccccctggaggccgcccacggaggcaacgtgctgatcaccgacacctggatcagcatgggacaggaggaggagaagaagaagcggctgcaggctttccagggttaccaggtgaccatgaagaccgccaaggtggctgccagcgactggaccttcctgcactgcctgcccaggaagcccgaggaggtggacgacgaggtgttctactctcccaggagcctggtgttccccgaggccgagaacaggaagtggaccatcatggctgtgatggtgtccctgctgaccgactacagcccccagctgcagaagcccaagttctgaataagtgaactcgagctagtgactgactaggatctggttaccactaaaccagcctcaagaacacccgaatggagtctctaagctacataataccaacttacacttacaaaatgttgtcccccaaaatgtagccattcgtatctgctcctaataaaaagaaagtttcttcacattctag

SEQ ID NO: 81 - RNA, 1377 nt, synthetic construct
  source 1..1377: mol_type = other RNA
tcaacacaacatatacaaaacaaacgaatctcaagcaatcaagcattctacttctattgcagcaatttaaatcatttcttttaaagcaaaagcaattttctgaaaattttcaccatttacgaacgatagccaccatgctgttcaacctgaggatcctgctgaacaacgcagctttcaggaacggccacaacttcatggtgaggaacttccggtgcggccagcccctgcagaacaaggtgcagctgaagggcagggacctgctgaccctgaagaacttcaccggagaggagatcaagtacatgctgtggctgagcgcagacctgaagttcaggatcaagcagaagggagagtacctgcccctgctgcaggggaagtccctgggcatgatcttcgagaagaggagtaccaggaccaggctgagcaccgaaaccggcttcgccctgctgggaggacacccctgcttcctgacgacccaggacatccacctcggagtgaacgaatccctcaccgataccgcccgggtgttatcaagcatggcagatgccgtgctggccagggtgtacaaacagtccgatctggacactctggctaaggaggccagcatccccatcatcaacggcctgagcgacctgtaccaccccatccagatcctggctgactacctgaccctgcaggagcactacagctctctgaagggcctgaccctgagctggatcggcgacgggaacaacatcctgcactccatcatgatgtccgccgcgaagttcggaatgcatctgcaagccgccacgccaaaaggatacgaaccggatgcgcccgtgacaaagttggcggaacagtacgctaaggagaacggaaccaagctgctgctgaccaacgaccccctggaggccgcccacggaggcaacgtgctgatcaccgacacctggatcagcatgggacaggaggaggagaagaagaagcggctgcaggctttccagggttaccaggtgaccatgaagaccgccaaggtggctgccagcgactggaccttcctgcactgcctgcccaggaagcccgaggaggtggacgacgaggtgttctactctcccaggagcctggtgttccccgaggccgagaacaggaagtggaccatcatggctgtgatggtgtccctgctgaccgactacagcccccagctgcagaagcccaagttctgaataagtgaactcgagctagtgactgactaggatctggttaccactaaaccagcctcaagaacacccgaatggagtctctaagctacataataccaacttacacttacaaaatgttgtcccccaaaatgtagccattcgtatctgctcctaataaaaagaaagtttcttcacattctag

SEQ ID NO: 82 - RNA, 1477 nt, synthetic construct
  source 1..1477: mol_type = other RNA
tcaacacaacatatacaaaacaaacgaatctcaagcaatcaagcattctacttctattgcagcaatttaaatcatttcttttaaagcaaaagcaattttctgaaaattttcaccatttacgaacgatagccaccatgctgttcaacctgcgcatcctgctgaacaacgccgccttccgcaacggccacaacttcatggtgcgcaacttccgctgcggccagcccctgcagaacaaggtgcagctgaagggccgcgacctgctgaccctgaagaacttcaccggcgaggagatcaagtacatgctgtggctgagcgccgacctgaagttccgcatcaagcagaagggcgagtacctgcccctgctgcagggcaagagcctgggcatgatcttcgagaagcgcagcacccgcacccgcctgagcaccgagacaggcttcgccctgctgggcggccacccctgcttcctgaccacccaggacatccacctgggcgtgaacgagagcctgaccgacaccgcccgcgtgctgagcagcatggccgacgccgtgctggcccgcgtgtacaagcagagcgacctggacaccctggccaaggaggccagcatccccatcatcaacggcctgagcgacctgtaccaccccatccagatcctggccgactacctgaccctgcaggagcactacagcagcctgaagggcctgaccctgagctggatcggcgacggcaacaacatcctgcacagcatcatgatgagcgccgccaagttcggcatgcacctgcaggccgccacccccaagggctacgagcccgacgccagcgtgaccaagctggccgagcagtacgccaaggagaacggcaccaagctgctgctgaccaacgaccccctggaggccgcccacggcggcaacgtgctgatcaccgacacctggatcagcatgggccaggaggaggagaagaagaagcgcctgcaggccttccagggctaccaggtgaccatgaagaccgccaaggtggccgccagcgactggaccttcctgcactgcctgccccgcaagcccgaggaggtggacgacgaggtgttctacagcccccgcagcctggtgttccccgaggccgagaaccgcaagtggaccatcatggccgtgatggtgagcctgctgaccgactacagcccccagctgcagaagcccaagttctgaataagtgaactcgagctagtgactgactaggatctggttaccactaaaccagcctcaagaacacccgaatggagtctctaagctacataataccaacttacacttacaaaatgttgtcccccaaaatgtagccattcgtatctgctcctaataaaaagaaagtttcttcacattctagaaaaaaaaaaaaaaaaaaaaaaaaaaaaaaaaaaaaaaaaaaaaaaaaaaaaaaaaaaaaaaaaaaaaaaaaaaaaaaaaaaaaaaaaaaaaaaaaaaaa

SEQ ID NO: 83 - RNA, 1371 nt, synthetic construct
  source 1..1371: mol_type = other RNA
aggaaacttaagtcaacacaacatatacaaaacaaacgaatctcaagcaatcaagcattctacttctattgcagcaatttaaatcatttcttttaaagcaaaagcaattttctgaaaattttcaccatttacgaacgatagccatgctgttcaacctgcgcatcctgctgaacaacgccgccttccgcaacggccacaacttcatggtgcgcaacttccgctgcggccagcccctgcagaacaaggtgcagctgaagggccgcgacctgctgaccctgaagaacttcaccggcgaggagatcaagtacatgctgtggctgagcgccgacctgaagttccgcatcaagcagaagggcgagtacctgcccctgctgcagggcaagagcctgggcatgatcttcgagaagcgcagcacccgcacccgcctgagcaccgagacaggcttcgccctgctgggcggccacccctgcttcctgaccacccaggacatccacctgggcgtgaacgagagcctgaccgacaccgcccgcgtgctgagcagcatggccgacgccgtgctggcccgcgtgtacaagcagagcgacctggacaccctggccaaggaggccagcatccccatcatcaacggcctgagcgacctgtaccaccccatccagatcctggccgactacctgaccctgcaggagcactacagcagcctgaagggcctgaccctgagctggatcggcgacggcaacaacatcctgcacagcatcatgatgagcgccgccaagttcggcatgcacctgcaggccgccacccccaagggctacgagcccgacgccagcgtgaccaagctggccgagcagtacgccaaggagaacggcaccaagctgctgctgaccaacgaccccctggaggccgcccacggcggcaacgtgctgatcaccgacacctggatcagcatgggccaggaggaggagaagaagaagcgcctgcaggccttccagggctaccaggtgaccatgaagaccgccaaggtggccgccagcgactggaccttcctgcactgcctgccccgcaagcccgaggaggtggacgacgaggtgttctacagcccccgcagcctggtgttccccgaggccgagaaccgcaagtggaccatcatggccgtgatggtgagcctgctgaccgactacagcccccagctgcagaagcccaagttctgactagtgactgactaggatctggttaccactaaaccagcctcaagaacacccgaatggagtctctaagctacataataccaacttacacttacaaaatgttgtcccccaaaatgtagccattcgtatctgctcctaataaaaagaaagtttcttcacattctag

SEQ ID NO: 84 - RNA, 1371 nt, synthetic construct
  source 1..1371: mol_type = other RNA
tcaacacaacatatacaaaacaaacgaatctcaagcaatcaagcattctacttctattgcagcaatttaaatcatttcttttaaagcaaaagcaattttctgaaaattttcaccatttacgaacgatagccaccatgcttttcaacttgagaatcctgctgaacaacgccgcctttcgcaacggtcacaattttatggtcagaaacttcagatgcggacagcccctccaaaacaaggtccagctgaagggccgcgatctcctcaccctgaagaacttcacgggggaggagatcaagtacatgctgtggctctccgctgacctgaagttcaggatcaagcagaagggagaatatctgccgctgctgcaagggaagtccctggggatgattttcgagaagcggagcacccggactcggctctccactgaaactggtttcgcccttctgggcggtcacccctgcttcctgaccactcaagacattcacctcggagtgaacgagtccttgactgacaccgcccgggtgctgtcgagcatggcagacgccgtgctagcccgcgtgtacaagcagtcagacctcgataccctggccaaggaggcttcgatcccgatcatcaacgggttgtccgacctgtaccacccgattcagattctcgccgactacctcaccctgcaagagcattacagctccctgaaggggcttaccctgtcctggattggcgacggaaacaacatcctgcactccattatgatgtcggcggccaagttcggcatgcacctccaagccgcgacccctaagggttacgaaccagacgcgtcagtgactaagctggccgaacagtacgcaaaggaaaatggcacgaagctgctcctgaccaacgatccgttggaagccgcccatggcggaaatgtgctcatcaccgacacctggatctcgatgggacaggaggaagagaagaagaagcggctgcaggcgttccagggctaccaggtcaccatgaaaactgccaaggtggccgccagcgactggaccttcctgcactgccttccgcgcaagcctgaggaggtggacgatgaagtgttctactctccacggtccctggtgttccccgaggcggagaaccgcaaatggaccatcatggctgtgatggtcagcctgctgaccgattacagccctcagttgcaaaagccgaagttttgataactcgagctagtgactgactaggatctggttaccactaaaccagcctcaagaacacccgaatggagtctctaagctacataataccaacttacacttacaaaatgttgtcccccaaaatgtagccattcgtatctgctcctaataaaaagaaagtttcttcacattctag

SEQ ID NO: 85 - RNA, 1471 nt, synthetic construct
  source 1..1471: mol_type = other RNA
tcaacacaacatatacaaaacaaacgaatctcaagcaatcaagcattctacttctattgcagcaatttaaatcatttcttttaaagcaaaagcaattttctgaaaattttcaccatttacgaacgatagccaccatgctgttcaacctccgcatcctcctcaacaacgccgcattcagaaacgggcacaacttcatggtcagaaacttccgctgcgggcaacccctacaaaacaaggtccagctcaaggggcgggacctcctgaccctgaagaacttcaccggcgaagagatcaagtacatgctgtggctctccgccgacctgaagttccgcatcaagcagaagggagagtacctcccgctgctgcaagggaagtcgctggggatgatcttcgagaagcggtcaaccagaacccggctgtcaaccgaaaccgggttcgcactgctggggggacacccgtgcttcctgaccacccaagacatccacctgggagtgaacgaatcgctgaccgacaccgcccgcgtgctgagctcaatggcggacgccgtgctggcccgcgtgtacaagcagtccgacctggacaccctggccaaggaagcgtccatcccgatcatcaacggactgtccgacctgtaccacccgatccagatcctggcagactacctgaccctgcaagaacactacagctccctgaagggcctgaccctgtcatggatcggggacgggaacaacatcctgcactccataatgatgtcagccgccaagttcggaatgcacctccaagccgcaaccccgaagggctacgaaccggacgcatcagtgaccaaactggccgagcagtacgccaaggaaaacggcaccaagctcctgctgaccaacgacccgctggaggccgcacacggggggaacgtgctgatcaccgacacctggatctccatgggacaggaggaggaaaagaagaagcggctgcaggcgttccaggggtaccaggtcaccatgaaaaccgcgaaggtcgcggcatcagactggaccttcctgcactgcctgccccggaagccggaagaggtggacgacgaggtgttctactcgccgcgctcgctggtgttccccgaggcggagaacaggaagtggaccatcatggcggtgatggtcagcctcctgaccgactactcgccgcagctgcagaagccgaagttctgataactcgagctagtgactgactaggatctggttaccactaaaccagcctcaagaacacccgaatggagtctctaagctacataataccaacttacacttacaaaatgttgtcccccaaaatgtagccattcgtatctgctcctaataaaaagaaagtttcttcacattctagaaaaaaaaaaaaaaaaaaaaaaaaaaaaaaaaaaaaaaaaaaaaaaaaaaaaaaaaaaaaaaaaaaaaaaaaaaaaaaaaaaaaaaaaaaaaaaaaaaaa

SEQ ID NO: 86 - RNA, 1771 nt, synthetic construct
  source 1..1771: mol_type = other RNA
ctccctcccccccccctaacgttactggccgaagccgcttggaataaggccggtgtgcgtttgtctatatgttattttccaccatattgccgtcttttggcaatgtgagggcccggaaacctggccctgtcttcttgacgagcattcctaggggtctttcccctctcgccaaaggaatgcaaggtctgttgaatgtcgtgaaggaagcagttcctctggaagcttcttgaagacaaacaacgtctgtagcgaccctttgcaggcagcggaaccccccacctggcgacaggtgcctctgcggccaaaagccacgtgtataagatacacctgcaaaggcggcacaaccccagtgccacgttgtgagttggatagttgtggaaagagtcaaatggctctcctcaagcgtattcaacaaggggctgaaggatgcccagaaggtaccccattgtatgggatctgatctggggcctcggtgcacatgctttacgtgtgtttagtcgaggttaaaaaacgtctaggccccccgaaccacggggacgtggttttcctttgaaaaacacgatgataatatgcttttcaatctccgcatcctccttaacaacgccgcgtttagaaacggccacaacttcatggtccggaacttcagatgtggccagccgcttcaaaacaaggtccagctgaagggccgggatcttctgaccctgaagaactttactggcgaagagatcaagtacatgctctggctctccgcggacttgaagttccgcattaagcagaagggggaataccttccgctgcttcaaggaaagagcctcggcatgatctttgagaagcgctcaaccaggacccgcctttctactgaaactgggttcgcgctgctcggtggccacccctgcttcctgacgacccaggacatccacctcggagtgaacgaatccctcaccgataccgcccgggtgttatcgagcatggcagatgccgtgctggccagggtgtacaaacagtccgatctggacactctggccaaggaggcgtcaattcctattatcaacggccttagtgacctctaccatccgattcagatcctggccgattacctcaccctgcaagaacactacagctccctgaagggtctgacattgtcctggatcggcgacggcaacaacattctccattccatcatgatgtccgccgcaaaattcggcatgcatcttcaagccgccacgccgaagggttacgagcccgacgcttccgtgactaagctcgccgagcagtacgctaaggagaacggaaccaagcttctgctgactaacgacccactagaagcagcccacgggggcaacgtgcttattactgacacctggatctccatgggccaggaagaagagaaaaagaagcggctgcaggcgttccagggatatcaggtcaccatgaaaaccgccaaggtcgctgcctccgactggaccttcctgcactgcctgcctcgcaagcctgaagaagtggacgacgaggtgttctactcgccacggagcctcgtgttccccgaggccgagaatagaaagtggaccatcatggccgtgatggtgtcactgctcaccgactacagcccgcagcttcagaagcccaagttctgaataagtagatagtgcagtcactggcacaacgcgttgcccggtaagccaatcgggtatacacggtcgtcatactgcagacagggttcttctactttgcaagatagtctagagtagtaaaataaatagtataagtctag

SEQ ID NO: 87 - RNA, 1771 nt, synthetic construct
  source 1..1771: mol_type = other RNA
ctccctcccccccccctaacgttactggccgaagccgcttggaataaggccggtgtgcgtttgtctatatgttattttccaccatattgccgtcttttggcaatgtgagggcccggaaacctggccctgtcttcttgacgagcattcctaggggtctttcccctctcgccaaaggaatgcaaggtctgttgaatgtcgtgaaggaagcagttcctctggaagcttcttgaagacaaacaacgtctgtagcgaccctttgcaggcagcggaaccccccacctggcgacaggtgcctctgcggccaaaagccacgtgtataagatacacctgcaaaggcggcacaaccccagtgccacgttgtgagttggatagttgtggaaagagtcaaatggctctcctcaagcgtattcaacaaggggctgaaggatgcccagaaggtaccccattgtatgggatctgatctggggcctcggtgcacatgctttacgtgtgtttagtcgaggttaaaaaacgtctaggccccccgaaccacggggacgtggttttcctttgaaaaacacgatgataatatgcttttcaacctgagaatcctcttgaacaatgctgcttttcggaatggccacaactttatggttcggaacttccgttgcggccagcctttacaaaacaaggtccagctgaagggccgggatttgctcacactaaagaactttactggagaagagatcaagtacatgctatggctgtcggccgacctgaagttccgtatcaagcagaagggagaataccttccgctgcttcaaggaaagagcctcggcatgatctttgagaagcgctcaaccaggacccgcctttctactgaaactgggttcgcgctgctcggtggccacccctgcttcctgacgacccaggacatccacctcggagtgaacgaatccctcaccgataccgcccgggtgttatcgagcatggcagatgccgtgctggccagggtgtacaaacagtccgatctcgataccttggcaaaggaggcttccattcccatcatcaacggcctgagcgacctgtaccacccaatccaaatcctggctgactacctgaccctgcaagagcactacagcagcctgaagggtctgaccctgtcatggattggcgatggaaacaatattctgcactccatcatgatgtccgccgcgaagttcggaatgcatctgcaagccgccactccaaaaggatacgaaccggatgcatccgtgaccaagttggcggaacagtacgcgaaggagaacggaaccaagctcctgctgactaacgacccgctcgaggctgcgcatgggggtaacgtgctgattacggacacctggatctccatggggcaggaggaagagaagaagaagagactgcaggcattccaggggtaccaggtcaccatgaaaaccgcaaaagtggcagcttcggactggactttcctgcattgcctgccgaggaagccggaggaagtcgacgacgaagtgttctactcgcctcggtccctggtgttccccgaggccgaaaaccggaagtggaccatcatggccgtgatggtgtccttgctgactgactatagcccgcagctgcagaagcctaagttctgaataagtagatagtgcagtcactggcacaacgcgttgcccggtaagccaatcgggtatacacggtcgtcatactgcagacagggttcttctactttgcaagatagtctagagtagtaaaataaatagtataagtctag

SEQ ID NO: 88 - RNA, 1771 nt, synthetic construct
  source 1..1771: mol_type = other RNA
ctccctcccccccccctaacgttactggccgaagccgcttggaataaggccggtgtgcgtttgtctatatgttattttccaccatattgccgtcttttggcaatgtgagggcccggaaacctggccctgtcttcttgacgagcattcctaggggtctttcccctctcgccaaaggaatgcaaggtctgttgaatgtcgtgaaggaagcagttcctctggaagcttcttgaagacaaacaacgtctgtagcgaccctttgcaggcagcggaaccccccacctggcgacaggtgcctctgcggccaaaagccacgtgtataagatacacctgcaaaggcggcacaaccccagtgccacgttgtgagttggatagttgtggaaagagtcaaatggctctcctcaagcgtattcaacaaggggctgaaggatgcccagaaggtaccccattgtatgggatctgatctggggcctcggtgcacatgctttacgtgtgtttagtcgaggttaaaaaacgtctaggccccccgaaccacggggacgtggttttcctttgaaaaacacgatgataatatgctgttcaacctgcgcatcctgctgaacaacgccgccttccgcaacggccacaacttcatggtgcgcaacttccgctgcggccagcccctgcagaacaaggtgcagctgaagggccgcgacctgctgaccctgaagaacttcaccggcgaggagatcaagtacatgctgtggctgagcgccgacctgaagttccgcatcaagcagaagggcgagtacctgcccctgctgcagggcaagagcctgggcatgatcttcgagaagcgcagcacccgcacccgcctgagcaccgagacaggcctggccctgctgggcggccacccctgcttcctgaccacccaggacatccacctgggcgtgaacgagagcctgaccgacaccgcccgcgtgctgagcagcatggccgacgccgtgctggcccgcgtgtacaagcagagcgacctggacaccctggccaaggaggccagcatccccatcatcaacggcctgagcgacctgtaccaccccatccagatcctggccgactacctgaccctgcaggagcactacagcagcctgaagggcctgaccctgagctggatcggcgacggcaacaacatcctgcacagcatcatgatgagcgccgccaagttcggcatgcacctgcaggccgccacccccaagggctacgagcccgacgccagcgtgaccaagctggccgagcagtacgccaaggagaacggcaccaagctgctgctgaccaacgaccccctggaggccgcccacggcggcaacgtgctgatcaccgacacctggatcagcatgggccaggaggaggagaagaagaagcgcctgcaggccttccagggctaccaggtgaccatgaagaccgccaaggtggccgccagcgactggaccttcctgcactgcctgccccgcaagcccgaggaggtggacgacgaggtgttctacagcccccgcagcctggtgttccccgaggccgagaaccgcaagtggaccatcatggccgtgatggtgagcctgctgaccgactacagcccccagctgcagaagcccaagttctgaataagtagatagtgcagtcactggcacaacgcgttgcccggtaagccaatcgggtatacacggtcgtcatactgcagacagggttcttctactttgcaagatagtctagagtagtaaaataaatagtataagtctag

SEQ ID NO: 89 - RNA, 1368 nt, synthetic construct; identical to SEQ ID NO: 34
  source 1..1368: mol_type = other RNA

SEQ ID NO: 90 - RNA, 1368 nt, synthetic construct; identical to SEQ ID NO: 34
  source 1..1368: mol_type = other RNA

SEQ ID NO: 91 - RNA, 1368 nt, synthetic construct; identical to SEQ ID NO: 34
  source 1..1368: mol_type = other RNA

SEQ ID NO: 92 - RNA, 1368 nt, synthetic construct; identical to SEQ ID NO: 34
  source 1..1368: mol_type = other RNA

SEQ ID NO: 93 - RNA, 1368 nt, synthetic construct; identical to SEQ ID NO: 34
  source 1..1368: mol_type = other RNA

SEQ ID NO: 94 - RNA, 1371 nt, synthetic construct
  source 1..1371: mol_type = other RNA
tcaacacaacatatacaaaacaaacgaatctcaagcaatcaagcattctacttctattgcagcaatttaaatcatttcttttaaagcaaaagcaattttctgaaaattttcaccatttacgaacgatagccaccatggtgttcaacctccgcatcctcctcaacaacgccgcattcagaaacgggcacaacttcatggtcagaaacttccgctgcgggcaacccctacaaaacaaggtccagctcaaggggcgggacctcctgaccctgaagaacttcaccggcgaagagatcaagtacatgctgtggctctccgccgacctgaagttccgcatcaagcagaagggagagtacctcccgctgctgcaagggaagtcgctggggatgatcttcgagaagcggtcaaccagaacccggctgtcaaccgaaaccgggttcgcactgctggggggacacccgtgcttcctgaccacccaagacatccacctgggagtgaacgaatcgctgaccgacaccgcccgcgtgctgagctcaatggcggacgccgtgctggcccgcgtgtacaagcagtccgacctggacaccctggccaaggaagcgtccatcccgatcatcaacggactgtccgacctgtaccacccgatccagatcctggcagactacctgaccctgcaagaacactacagctccctgaagggcctgaccctgtcatggatcggggacgggaacaacatcctgcactccataatgatgtcagccgccaagttcggaatgcacctccaagccgcaaccccgaagggctacgaaccggacgcatcagtgaccaaactggccgagcagtacgccaaggaaaacggcaccaagctcctgctgaccaacgacccgctggaggccgcacacggggggaacgtgctgatcaccgacacctggatctccatgggacaggaggaggaaaagaagaagcggctgcaggcgttccaggggtaccaggtcaccatgaaaaccgcgaaggtcgcggcatcagactggaccttcctgcactgcctgccccggaagccggaagaggtggacgacgaggtgttctactcgccgcgctcgctggtgttccccgaggcggagaacaggaagtggaccatcatggcggtgatggtcagcctcctgaccgactactcgccgcagctgcagaagccgaagttctgataactcgagctagtgactgactaggatctggttaccactaaaccagcctcaagaacacccgaatggagtctctaagctacataataccaacttacacttacaaaatgttgtcccccaaaatgtagccattcgtatctgctcctaataaaaagaaagtttcttcacattctag

SEQ ID NO: 95 - RNA, 1371 nt, synthetic construct
  source 1..1371: mol_type = other RNA
tcaacacaacatatacaaaacaaacgaatctcaagcaatcaagcattctacttctattgcagcaatttaaatcatttcttttaaagcaaaagcaattttctgaaaattttcaccatttacgaacgatagccaccatggtgttcaacctccgcatcctcctcaacaacgccgcattcagaaacgggcacaacttcatggtcagaaacttccgctgcgggcaacccctacaaaaccgggtccagctcaaggggcgggacctcctgaccctgaagaacttcaccggcgaagagatcaagtacatgctgtggctctccgccgacctgaagttccgcatcaagcagaagggagagtacctcccgctgctgcaagggaagtcgctggggatgatcttcgagaagcggtcaaccagaacccggctgtcaaccgaaaccgggttcgcactgctggggggacacccgtgcttcctgaccacccaagacatccacctgggagtgaacgaatcgctgaccgacaccgcccgcgtgctgagctcaatggcggacgccgtgctggcccgcgtgtacaagcagtccgacctggacaccctggccaaggaagcgtccatcccgatcatcaacggactgtccgacctgtaccacccgatccagatcctggcagactacctgaccctgcaagaacactacagctccctgaagggcctgaccctgtcatggatcggggacgggaacaacatcctgcactccataatgatgtcagccgccaagttcggaatgcacctccaagccgcaaccccgaagggctacgaaccggacgcatcagtgaccaaactggccgagcagtacgccaaggaaaacggcaccaagctcctgctgaccaacgacccgctggaggccgcacacggggggaacgtgctgatcaccgacacctggatctccatgggacaggaggaggaaaagaagaagcggctgcaggcgttccaggggtaccaggtcaccatgaaaaccgcgaaggtcgcggcatcagactggaccttcctgcactgcctgccccggaagccggaagaggtggacgacgaggtgttctactcgccgcgctcgctggtgttccccgaggcggagaacaggaagtggaccatcatggcggtgatggtcagcctcctgaccgactactcgccgcagctgcagaagccgaagttctgataactcgagctagtgactgactaggatctggttaccactaaaccagcctcaagaacacccgaatggagtctctaagctacataataccaacttacacttacaaaatgttgtcccccaaaatgtagccattcgtatctgctcctaataaaaagaaagtttcttcacattctag

SEQ ID NO: 96 - RNA, 1371 nt, synthetic construct
  source 1..1371: mol_type = other RNA
tcaacacaacatatacaaaacaaacgaatctcaagcaatcaagcattctacttctattgcagcaatttaaatcatttcttttaaagcaaaagcaattttctgaaaattttcaccatttacgaacgatagccaccatggtgttcaacctccgcatcctcctcaacaacgccgcattcagaaacgggcacaacttcatggtcagaaacttccgctgcgggcaacccctacaaaaccgggtccagctcaaggggcgggacctcctgaccctgaagaacttcaccggcgaagagatccggtacatgctgtggctctccgccgacctgaagttccgcatcaagcagaagggagagtacctcccgctgctgcaagggaagtcgctggggatgatcttcgagaagcggtcaaccagaacccggctgtcaaccgaaaccgggttcgcactgctggggggacacccgtgcttcctgaccacccaagacatccacctgggagtgaacgaatcgctgaccgacaccgcccgcgtgctgagctcaatggcggacgccgtgctggcccgcgtgtacaagcagtccgacctggacaccctggccaaggaagcgtccatcccgatcatcaacggactgtccgacctgtaccacccgatccagatcctggcagactacctgaccctgcaagaacactacagctccctgaagggcctgaccctgtcatggatcggggacgggaacaacatcctgcactccataatgatgtcagccgccaagttcggaatgcacctccaagccgcaaccccgaagggctacgaaccggacgcatcagtgaccaaactggccgagcagtacgccaaggaaaacggcaccaagctcctgctgaccaacgacccgctggaggccgcacacggggggaacgtgctgatcaccgacacctggatctccatgggacaggaggaggaaaagaagaagcggctgcaggcgttccaggggtaccaggtcaccatgaaaaccgcgaaggtcgcggcatcagactggaccttcctgcactgcctgccccggaagccggaagaggtggacgacgaggtgttctactcgccgcgctcgctggtgttccccgaggcggagaacaggaagtggaccatcatggcggtgatggtcagcctcctgaccgactactcgccgcagctgcagaagccgaagttctgataactcgagctagtgactgactaggatctggttaccactaaaccagcctcaagaacacccgaatggagtctctaagctacataataccaacttacacttacaaaatgttgtcccccaaaatgtagccattcgtatctgctcctaataaaaagaaagtttcttcacattctag

SEQ ID NO: 97 - RNA, 1371 nt, synthetic construct
  source 1..1371: mol_type = other RNA
tcaacacaacatatacaaaacaaacgaatctcaagcaatcaagcattctacttctattgcagcaatttaaatcatttcttttaaagcaaaagcaattttctgaaaattttcaccatttacgaacgatagccaccatgctggtcaacctccgcatcctcctcaacaacgccgcattcagaaacgggcacaacttcatggtcagaaacttccgctgcgggcaacccctacaaaacaaggtccagctcaaggggcgggacctcctgaccctgaagaacttcaccggcgaagagatcaagtacatgctgtggctctccgccgacctgaagttccgcatcaagcagaagggagagtacctcccgctgctgcaagggaagtcgctggggatgatcttcgagaagcggtcaaccagaacccggctgtcaaccgaaaccgggttcgcactgctggggggacacccgtgcttcctgaccacccaagacatccacctgggagtgaacgaatcgctgaccgacaccgcccgcgtgctgagctcaatggcggacgccgtgctggcccgcgtgtacaagcagtccgacctggacaccctggccaaggaagcgtccatcccgatcatcaacggactgtccgacctgtaccacccgatccagatcctggcagactacctgaccctgcaagaacactacagctccctgaagggcctgaccctgtcatggatcggggacgggaacaacatcctgcactccataatgatgtcagccgccaagttcggaatgcacctccaagccgcaaccccgaagggctacgaaccggacgcatcagtgaccaaactggccgagcagtacgccaaggaaaacggcaccaagctcctgctgaccaacgacccgctggaggccgcacacggggggaacgtgctgatcaccgacacctggatctccatgggacaggaggaggaaaagaagaagcggctgcaggcgttccaggggtaccaggtcaccatgaaaaccgcgaaggtcgcggcatcagactggaccttcctgcactgcctgccccggaagccggaagaggtggacgacgaggtgttctactcgccgcgctcgctggtgttccccgaggcggagaacaggaagtggaccatcatggcggtgatggtcagcctcctgaccgactactcgccgcagctgcagaagccgaagttctgataactcgagctagtgactgactaggatctggttaccactaaaccagcctcaagaacacccgaatggagtctctaagctacataataccaacttacacttacaaaatgttgtcccccaaaatgtagccattcgtatctgctcctaataaaaagaaagtttcttcacattctag

SEQ ID NO: 98 - RNA, 1471 nt, synthetic construct
  source 1..1471: mol_type = other RNA
tcaacacaacatatacaaaacaaacgaatctcaagcaatcaagcattctacttctattgcagcaatttaaatcatttcttttaaagcaaaagcaattttctgaaaattttcaccatttacgaacgatagccaccatgctggtcaacctccgcatcctcctcaacaacgccgcattcagaaacgggcacaacttcatggtcagaaacttccgctgcgggcaacccctacaaaaccgggtccagctcaaggggcgggacctcctgaccctgaagaacttcaccggcgaagagatcaagtacatgctgtggctctccgccgacctgaagttccgcatcaagcagaagggagagtacctcccgctgctgcaagggaagtcgctggggatgatcttcgagaagcggtcaaccagaacccggctgtcaaccgaaaccgggttcgcactgctggggggacacccgtgcttcctgaccacccaagacatccacctgggagtgaacgaatcgctgaccgacaccgcccgcgtgctgagctcaatggcggacgccgtgctggcccgcgtgtacaagcagtccgacctggacaccctggccaaggaagcgtccatcccgatcatcaacggactgtccgacctgtaccacccgatccagatcctggcagactacctgaccctgcaagaacactacagctccctgaagggcctgaccctgtcatggatcggggacgggaacaacatcctgcactccataatgatgtcagccgccaagttcggaatgcacctccaagccgcaaccccgaagggctacgaaccggacgcatcagtgaccaaactggccgagcagtacgccaaggaaaacggcaccaagctcctgctgaccaacgacccgctggaggccgcacacggggggaacgtgctgatcaccgacacctggatctccatgggacaggaggaggaaaagaagaagcggctgcaggcgttccaggggtaccaggtcaccatgaaaaccgcgaaggtcgcggcatcagactggaccttcctgcactgcctgccccggaagccggaagaggtggacgacgaggtgttctactcgccgcgctcgctggtgttccccgaggcggagaacaggaagtggaccatcatggcggtgatggtcagcctcctgaccgactactcgccgcagctgcagaagccgaagttctgataactcgagctagtgactgactaggatctggttaccactaaaccagcctcaagaacacccgaatggagtctctaagctacataataccaacttacacttacaaaatgttgtcccccaaaatgtagccattcgtatctgctcctaataaaaagaaagtttcttcacattctagaaaaaaaaaaaaaaaaaaaaaaaaaaaaaaaaaaaaaaaaaaaaaaaaaaaaaaaaaaaaaaaaaaaaaaaaaaaaaaaaaaaaaaaaaaaaaaaaaaaa

SEQ ID NO: 99 - RNA, 1371 nt, synthetic construct
  source 1..1371: mol_type = other RNA
tcaacacaacatatacaaaacaaacgaatctcaagcaatcaagcattctacttctattgcagcaatttaaatcatttcttttaaagcaaaagcaattttctgaaaattttcaccatttacgaacgatagccaccatgctggtcaacctccgcatcctcctcaacaacgccgcattcagaaacgggcacaacttcatggtcagaaacttccgctgcgggcaacccctacaaaaccgggtccagctcaaggggcgggacctcctgaccctgaagaacttcaccggcgaagagatccggtacatgctgtggctctccgccgacctgaagttccgcatcaagcagaagggagagtacctcccgctgctgcaagggaagtcgctggggatgatcttcgagaagcggtcaaccagaacccggctgtcaaccgaaaccgggttcgcactgctggggggacacccgtgcttcctgaccacccaagacatccacctgggagtgaacgaatcgctgaccgacaccgcccgcgtgctgagctcaatggcggacgccgtgctggcccgcgtgtacaagcagtccgacctggacaccctggccaaggaagcgtccatcccgatcatcaacggactgtccgacctgtaccacccgatccagatcctggcagactacctgaccctgcaagaacactacagctccctgaagggcctgaccctgtcatggatcggggacgggaacaacatcctgcactccataatgatgtcagccgccaagttcggaatgcacctccaagccgcaaccccgaagggctacgaaccggacgcatcagtgaccaaactggccgagcagtacgccaaggaaaacggcaccaagctcctgctgaccaacgacccgctggaggccgcacacggggggaacgtgctgatcaccgacacctggatctccatgggacaggaggaggaaaagaagaagcggctgcaggcgttccaggggtaccaggtcaccatgaaaaccgcgaaggtcgcggcatcagactggaccttcctgcactgcctgccccggaagccggaagaggtggacgacgaggtgttctactcgccgcgctcgctggtgttccccgaggcggagaacaggaagtggaccatcatggcggtgatggtcagcctcctgaccgactactcgccgcagctgcagaagccgaagttctgataactcgagctagtgactgactaggatctggttaccactaaaccagcctcaagaacacccgaatggagtctctaagctacataataccaacttacacttacaaaatgttgtcccccaaaatgtagccattcgtatctgctcctaataaaaagaaagtttcttcacattctag

SEQ ID NO: 100 - RNA, 1471 nt, synthetic construct
  source 1..1471: mol_type = other RNA
tcaacacaacatatacaaaacaaacgaatctcaagcaatcaagcattctacttctattgcagcaatttaaatcatttcttttaaagcaaaagcaattttctgaaaattttcaccatttacgaacgatagccaccatgctggtcaacctgcgcatcctgctgaacaacgccgccttccgcaacggccacaacttcatggtgcgcaacttccgctgcggccagcccctgcagaacaaggtgcagctgaagggccgcgacctgctgaccctgaagaacttcaccggcgaggagatcaagtacatgctgtggctgagcgccgacctgaagttccgcatcaagcagaagggcgagtacctgcccctgctgcagggcaagagcctgggcatgatcttcgagaagcgcagcacccgcacccgcctgagcaccgagacaggcttcgccctgctgggcggccacccctgcttcctgaccacccaggacatccacctgggcgtgaacgagagcctgaccgacaccgcccgcgtgctgagcagcatggccgacgccgtgctggcccgcgtgtacaagcagagcgacctggacaccctggccaaggaggccagcatccccatcatcaacggcctgagcgacctgtaccaccccatccagatcctggccgactacctgaccctgcaggagcactacagcagcctgaagggcctgaccctgagctggatcggcgacggcaacaacatcctgcacagcatcatgatgagcgccgccaagttcggcatgcacctgcaggccgccacccccaagggctacgagcccgacgccagcgtgaccaagctggccgagcagtacgccaaggagaacggcaccaagctgctgctgaccaacgaccccctggaggccgcccacggcggcaacgtgctgatcaccgacacctggatcagcatgggccaggaggaggagaagaagaagcgcctgcaggccttccagggctaccaggtgaccatgaagaccgccaaggtggccgccagcgactggaccttcctgcactgcctgccccgcaagcccgaggaggtggacgacgaggtgttctacagcccccgcagcctggtgttccccgaggccgagaaccgcaagtggaccatcatggccgtgatggtgagcctgctgaccgactacagcccccagctgcagaagcccaagttctgataactcgagctagtgactgactaggatctggttaccactaaaccagcctcaagaacacccgaatggagtctctaagctacataataccaacttacacttacaaaatgttgtcccccaaaatgtagccattcgtatctgctcctaataaaaagaaagtttcttcacattctagaaaaaaaaaaaaaaaaaaaaaaaaaaaaaaaaaaaaaaaaaaaaaaaaaaaaaaaaaaaaaaaaaaaaaaaaaaaaaaaaaaaaaaaaaaaaaaaaaaaa

SEQ ID NO: 101 - RNA, 1371 nt, synthetic construct
  source 1..1371: mol_type = other RNA
tcaacacaacatatacaaaacaaacgaatctcaagcaatcaagcattctacttctattgcagcaatttaaatcatttcttttaaagcaaaagcaattttctgaaaattttcaccatttacgaacgatagccaccatgctggtcaacctgcgcatcctgctgaacaacgccgccttccgcaacggccacaacttcatggtgcgcaacttccgctgcggccagcccctgcagaaccgggtgcagctgaagggccgcgacctgctgaccctgaagaacttcaccggcgaggagatcaagtacatgctgtggctgagcgccgacctgaagttccgcatcaagcagaagggcgagtacctgcccctgctgcagggcaagagcctgggcatgatcttcgagaagcgcagcacccgcacccgcctgagcaccgagacaggcttcgccctgctgggcggccacccctgcttcctgaccacccaggacatccacctgggcgtgaacgagagcctgaccgacaccgcccgcgtgctgagcagcatggccgacgccgtgctggcccgcgtgtacaagcagagcgacctggacaccctggccaaggaggccagcatccccatcatcaacggcctgagcgacctgtaccaccccatccagatcctggccgactacctgaccctgcaggagcactacagcagcctgaagggcctgaccctgagctggatcggcgacggcaacaacatcctgcacagcatcatgatgagcgccgccaagttcggcatgcacctgcaggccgccacccccaagggctacgagcccgacgccagcgtgaccaagctggccgagcagtacgccaaggagaacggcaccaagctgctgctgaccaacgaccccctggaggccgcccacggcggcaacgtgctgatcaccgacacctggatcagcatgggccaggaggaggagaagaagaagcgcctgcaggccttccagggctaccaggtgaccatgaagaccgccaaggtggccgccagcgactggaccttcctgcactgcctgccccgcaagcccgaggaggtggacgacgaggtgttctacagcccccgcagcctggtgttccccgaggccgagaaccgcaagtggaccatcatggccgtgatggtgagcctgctgaccgactacagcccccagctgcagaagcccaagttctgataactcgagctagtgactgactaggatctggttaccactaaaccagcctcaagaacacccgaatggagtctctaagctacataataccaacttacacttacaaaatgttgtcccccaaaatgtagccattcgtatctgctcctaataaaaagaaagtttcttcacattctag

SEQ ID NO: 102 - RNA, 1368 nt, synthetic construct
  source 1..1368: mol_type = other RNA
tcaacacaacatatacaaaacaaacgaatctcaagcaatcaagcattctacttctattgcagcaatttaaatcatttcttttaaagcaaaagcaattttctgaaaattttcaccatttacgaacgatagccaccatgcttgtcaatctccgcatcctccttaacaacgccgcgtttagaaacggccacaacttcatggtccggaacttcagatgtggccagccgcttcaaaacaaggtccagctgaagggccgggatcttctgaccctgaagaactttactggcgaagagatcaagtacatgctctggctctccgcggacttgaagttccgcattaagcagaagggggaataccttccgctgcttcaaggaaagagcctcggcatgatctttgagaagcgctcaaccaggacccgcctttctactgaaactgggttcgcgctgctcggtggccacccctgcttcctgacgacccaggacatccacctcggagtgaacgaatccctcaccgataccgcccgggtgttatcgagcatggcagatgccgtgctggccagggtgtacaaacagtccgatctggacactctggccaaggaggcgtcaattcctattatcaacggccttagtgacctctaccatccgattcagatcctggccgattacctcaccctgcaagaacactacagctccctgaagggtctgacattgtcctggatcggcgacggcaacaacattctccattccatcatgatgtccgccgcaaaattcggcatgcatcttcaagccgccacgccgaagggttacgagcccgacgcttccgtgactaagctcgccgagcagtacgctaaggagaacggaaccaagcttctgctgactaacgacccactagaagcagcccacgggggcaacgtgcttattactgacacctggatctccatgggccaggaagaagagaaaaagaagcggctgcaggcgttccagggatatcaggtcaccatgaaaaccgccaaggtcgctgcctccgactggaccttcctgcactgcctgcctcgcaagcctgaagaagtggacgacgaggtgttctactcgccacggagcctcgtgttccccgaggccgagaatagaaagtggaccatcatggccgtgatggtgtcactgctcaccgactacagcccgcagcttcagaagcccaagttctagctcgagctagtgactgactaggatctggttaccactaaaccagcctcaagaacacccgaatggagtctctaagctacataataccaacttacacttacaaaatgttgtcccccaaaatgtagccattcgtatctgctcctaataaaaagaaagtttcttcacattctag

SEQ ID NO: 103 - RNA, 1368 nt, synthetic construct
  source 1..1368: mol_type = other RNA
tcaacacaacatatacaaaacaaacgaatctcaagcaatcaagcattctacttctattgcagcaatttaaatcatttcttttaaagcaaaagcaattttctgaaaattttcaccatttacgaacgatagccaccatgcttgtcaatctccgcatcctccttaacaacgccgcgtttagaaacggccacaacttcatggtccggaacttcagatgtggccagccgcttcaaaaccgggtccagctgaagggccgggatcttctgaccctgaagaactttactggcgaagagatcaagtacatgctctggctctccgcggacttgaagttccgcattaagcagaagggggaataccttccgctgcttcaaggaaagagcctcggcatgatctttgagaagcgctcaaccaggacccgcctttctactgaaactgggttcgcgctgctcggtggccacccctgcttcctgacgacccaggacatccacctcggagtgaacgaatccctcaccgataccgcccgggtgttatcgagcatggcagatgccgtgctggccagggtgtacaaacagtccgatctggacactctggccaaggaggcgtcaattcctattatcaacggccttagtgacctctaccatccgattcagatcctggccgattacctcaccctgcaagaacactacagctccctgaagggtctgacattgtcctggatcggcgacggcaacaacattctccattccatcatgatgtccgccgcaaaattcggcatgcatcttcaagccgccacgccgaagggttacgagcccgacgcttccgtgactaagctcgccgagcagtacgctaaggagaacggaaccaagcttctgctgactaacgacccactagaagcagcccacgggggcaacgtgcttattactgacacctggatctccatgggccaggaagaagagaaaaagaagcggctgcaggcgttccagggatatcaggtcaccatgaaaaccgccaaggtcgctgcctccgactggaccttcctgcactgcctgcctcgcaagcctgaagaagtggacgacgaggtgttctactcgccacggagcctcgtgttccccgaggccgagaatagaaagtggaccatcatggccgtgatggtgtcactgctcaccgactacagcccgcagcttcagaagcccaagttctagctcgagctagtgactgactaggatctggttaccactaaaccagcctcaagaacacccgaatggagtctctaagctacataataccaacttacacttacaaaatgttgtcccccaaaatgtagccattcgtatctgctcctaataaaaagaaagtttcttcacattctag

SEQ ID NO: 104 - RNA, 1371 nt, synthetic construct
  source 1..1371: mol_type = other RNA
tcaacacaacatatacaaaacaaacgaatctcaagcaatcaagcattctacttctattgcagcaatttaaatcatttcttttaaagcaaaagcaattttctgaaaattttcaccatttacgaacgatagccaccatgggccttgtcaatctccgcatcctccttaacaacgccgcgtttagaaacggccacaacttcatggtccggaacttcagatgtggccagccgcttcaaaacaaggtccagctgaagggccgggatcttctgaccctgaagaactttactggcgaagagatcaagtacatgctctggctctccgcggacttgaagttccgcattaagcagaagggggaataccttccgctgcttcaaggaaagagcctcggcatgatctttgagaagcgctcaaccaggacccgcctttctactgaaactgggttcgcgctgctcggtggccacccctgcttcctgacgacccaggacatccacctcggagtgaacgaatccctcaccgataccgcccgggtgttatcgagcatggcagatgccgtgctggccagggtgtacaaacagtccgatctggacactctggccaaggaggcgtcaattcctattatcaacggccttagtgacctctaccatccgattcagatcctggccgattacctcaccctgcaagaacactacagctccctgaagggtctgacattgtcctggatcggcgacggcaacaacattctccattccatcatgatgtccgccgcaaaattcggcatgcatcttcaagccgccacgccgaagggttacgagcccgacgcttccgtgactaagctcgccgagcagtacgctaaggagaacggaaccaagcttctgctgactaacgacccactagaagcagcccacgggggcaacgtgcttattactgacacctggatctccatgggccaggaagaagagaaaaagaagcggctgcaggcgttccagggatatcaggtcaccatgaaaaccgccaaggtcgctgcctccgactggaccttcctgcactgcctgcctcgcaagcctgaagaagtggacgacgaggtgttctactcgccacggagcctcgtgttccccgaggccgagaatagaaagtggaccatcatggccgtgatggtgtcactgctcaccgactacagcccgcagcttcagaagcccaagttctagctcgagctagtgactgactaggatctggttaccactaaaccagcctcaagaacacccgaatggagtctctaagctacataataccaacttacacttacaaaatgttgtcccccaaaatgtagccattcgtatctgctcctaataaaaagaaagtttcttcacattctag

SEQ ID NO: 105 - RNA, 1485 nt, synthetic construct
  source 1..1485: mol_type = other RNA
tcaacacaacatatacaaaacaaacgaatctcaagcaatcaagcattctacttctattgcagcaatttaaatcatttcttttaaagcaaaagcaattttctgaaaattttcaccatttacgaacgatagccaccatgggccttgtcaatctccgcatcctccttaacaacgccgcgtttagaaacggccacaacttcatggtccggaacttcagatgtggccagccgcttcaaaaccgggtccagctgaagggccgggatcttctgaccctgaagaactttactggcgaagagatcaagtacatgctctggctctccgcggacttgaagttccgcattaagcagaagggggaataccttccgctgcttcaaggaaagagcctcggcatgatctttgagaagcgctcaaccaggacccgcctttctactgaaactgggttcgcgctgctcggtggccacccctgcttcctgacgacccaggacatccacctcggagtgaacgaatccctcaccgataccgcccgggtgttatcgagcatggcagatgccgtgctggccagggtgtacaaacagtccgatctggacactctggccaaggaggcgtcaattcctattatcaacggccttagtgacctctaccatccgattcagatcctggccgattacctcaccctgcaagaacactacagctccctgaagggtctgacattgtcctggatcggcgacggcaacaacattctccattccatcatgatgtccgccgcaaaattcggcatgcatcttcaagccgccacgccgaagggttacgagcccgacgcttccgtgactaagctcgccgagcagtacgctaaggagaacggaaccaagcttctgctgactaacgacccactagaagcagcccacgggggcaacgtgcttattactgacacctggatctccatgggccaggaagaagagaaaaagaagcggctgcaggcgttccagggatatcaggtcaccatgaaaaccgccaaggtcgctgcctccgactggaccttcctgcactgcctgcctcgcaagcctgaagaagtggacgacgaggtgttctactcgccacggagcctcgtgttccccgaggccgagaatagaaagtggaccatcatggccgtgatggtgtcactgctcaccgactacagcccgcagcttcagaagcccaagttctagctcgagctagtgactgactaggatctggttaccactaaaccagcctcaagaacacccgaatggagtctctaagctacataataccaacttacacttacaaaatgttgtcccccaaaatgtagccattcgtatctgctcctaataaaaagaaagtttcttcacattctagaaaaaaaaaaaaaaaaaaaaaaaaaaaaaaaaaaaaaaaaaaaaaaaaaaaaaaaaaaaaaaaaaaaaaaaaaaaaaaaaaaaaaaaaaaaaaaaaaaaaaaaaaaaaaaaaaa

SEQ ID NO: 106 - RNA, 1374 nt, synthetic construct
  source 1..1374: mol_type = other RNA
tcaacacaacatatacaaaacaaacgaatctcaagcaatcaagcattctacttctattgcagcaatttaaatcatttcttttaaagcaaaagcaattttctgaaaattttcaccatttacgaacgatagccaccatgggcggacttgtcaatctccgcatcctccttaacaacgccgcgtttagaaacggccacaacttcatggtccggaacttcagatgtggccagccgcttcaaaacaaggtccagctgaagggccgggatcttctgaccctgaagaactttactggcgaagagatcaagtacatgctctggctctccgcggacttgaagttccgcattaagcagaagggggaataccttccgctgcttcaaggaaagagcctcggcatgatctttgagaagcgctcaaccaggacccgcctttctactgaaactgggttcgcgctgctcggtggccacccctgcttcctgacgacccaggacatccacctcggagtgaacgaatccctcaccgataccgcccgggtgttatcgagcatggcagatgccgtgctggccagggtgtacaaacagtccgatctggacactctggccaaggaggcgtcaattcctattatcaacggccttagtgacctctaccatccgattcagatcctggccgattacctcaccctgcaagaacactacagctccctgaagggtctgacattgtcctggatcggcgacggcaacaacattctccattccatcatgatgtccgccgcaaaattcggcatgcatcttcaagccgccacgccgaagggttacgagcccgacgcttccgtgactaagctcgccgagcagtacgctaaggagaacggaaccaagcttctgctgactaacgacccactagaagcagcccacgggggcaacgtgcttattactgacacctggatctccatgggccaggaagaagagaaaaagaagcggctgcaggcgttccagggatatcaggtcaccatgaaaaccgccaaggtcgctgcctccgactggaccttcctgcactgcctgcctcgcaagcctgaagaagtggacgacgaggtgttctactcgccacggagcctcgtgttccccgaggccgagaatagaaagtggaccatcatggccgtgatggtgtcactgctcaccgactacagcccgcagcttcagaagcccaagttctagctcgagctagtgactgactaggatctggttaccactaaaccagcctcaagaacacccgaatggagtctctaagctacataataccaacttacacttacaaaatgttgtcccccaaaatgtagccattcgtatctgctcctaataaaaagaaagtttcttcacattctag

SEQ ID NO: 107 - RNA, 1377 nt, synthetic construct
  source 1..1377: mol_type = other RNA
tcaacacaacatatacaaaacaaacgaatctcaagcaatcaagcattctacttctattgcagcaatttaaatcatttcttttaaagcaaaagcaattttctgaaaattttcaccatttacgaacgatagccatggcccttttcaatctccgcatcctccttaacaacgccgcgtttagaaacggccacaacttcatggtccggaacttcagatgtggccagccgcttcaaggcaaggtccagctgaagggccgggatcttctgaccctgaagaactttactggcgaagagatcaagtacatgctctggctctccgcggacttgaagttccgcattaagcagaagggggaataccttccgctgcttcaaggaaagagcctcggcatgatctttgagaagcgctcaaccaggacccgcctttctactgaaactgggttcgcgctgctcggtggccacccctgcttcctgacgacccaggacatccacctcggagtgaacgaatccctcaccgataccgcccgggtgttatcgagcatggcagatgccgtgctggccagggtgtacaaacagtccgatctggacactctggccaaggaggcgtcaattcctattatcaacggccttagtgacctctaccatccgattcagatcctggccgattacctcaccctgcaagaacactacagctccctgaagggtctgacattgtcctggatcggcgacggcaacaacattctccattccatcatgatgtccgccgcaaaattcggcatgcatcttcaagccgccacgccgaagggttacgagcccgacgcttccgtgactaagctcgccgagcagtacgctaaggagaacggaaccaagcttctgctgactaacgacccactagaagcagcccacgggggcaacgtgcttattactgacacctggatctccatgggccaggaagaagagaaaaagaagcggctgcaggcgttccagggatatcaggtcaccatgaaaaccgccaaggtcgctgcctccgactggaccttcctgcactgcctgcctcgcaagcctgaagaagtggacgacgaggtgttctactcgccacggagcctcgtgttccccgaggccgagaatagaaagtggaccatcatggccgtgatggtgtcactgctcaccgactacagcccgcagcttcagaagcccaagttctagataagtgaactcgagctagtgactgactaggatctggttaccactaaaccagcctcaagaacacccgaatggagtctctaagctacataataccaacttacacttacaaaatgttgtcccccaaaatgtagccattcgtatctgctcctaataaaaagaaagtttcttcacattctag

SEQ ID NO: 108 - RNA, 1377 nt, synthetic construct
  source 1..1377: mol_type = other RNA
tcaacacaacatatacaaaacaaacgaatctcaagcaatcaagcattctacttctattgcagcaatttaaatcatttcttttaaagcaaaagcaattttctgaaaattttcaccatttacgaacgatagccatggcccttttcaatctccgcatcctccttaacaacgccgcgtttagaaacggccacaacttcatggtccggaacttcagatgtggccagccgcttcaaggccgggtccagctgaagggccgggatcttctgaccctgaagaactttactggcgaagagatcaagtacatgctctggctctccgcggacttgaagttccgcattaagcagaagggggaataccttccgctgcttcaaggaaagagcctcggcatgatctttgagaagcgctcaaccaggacccgcctttctactgaaactgggttcgcgctgctcggtggccacccctgcttcctgacgacccaggacatccacctcggagtgaacgaatccctcaccgataccgcccgggtgttatcgagcatggcagatgccgtgctggccagggtgtacaaacagtccgatctggacactctggccaaggaggcgtcaattcctattatcaacggccttagtgacctctaccatccgattcagatcctggccgattacctcaccctgcaagaacactacagctccctgaagggtctgacattgtcctggatcggcgacggcaacaacattctccattccatcatgatgtccgccgcaaaattcggcatgcatcttcaagccgccacgccgaagggttacgagcccgacgcttccgtgactaagctcgccgagcagtacgctaaggagaacggaaccaagcttctgctgactaacgacccactagaagcagcccacgggggcaacgtgcttattactgacacctggatctccatgggccaggaagaagagaaaaagaagcggctgcaggcgttccagggatatcaggtcaccatgaaaaccgccaaggtcgctgcctccgactggaccttcctgcactgcctgcctcgcaagcctgaagaagtggacgacgaggtgttctactcgccacggagcctcgtgttccccgaggccgagaatagaaagtggaccatcatggccgtgatggtgtcactgctcaccgactacagcccgcagcttcagaagcccaagttctagataagtgaactcgagctagtgactgactaggatctggttaccactaaaccagcctcaagaacacccgaatggagtctctaagctacataataccaacttacacttacaaaatgttgtcccccaaaatgtagccattcgtatctgctcctaataaaaagaaagtttcttcacattctag

SEQ ID NO: 109 - RNA, 1377 nt, synthetic construct
  source 1..1377: mol_type = other RNA
tcaacacaacatatacaaaacaaacgaatctcaagcaatcaagcattctacttctattgcagcaatttaaatcatttcttttaaagcaaaagcaattttctgaaaattttcaccatttacgaacgatagccatggcccttttcaatctccgcatcctccttaacaacgccgcgtttagaaacggccacaacttcatggtccggaacttcagatgtggccagccgcttcaaggccgggtccagctgaagggccgggatcttctgaccctgaagaactttactggcgaagagatcaggtacatgctctggctctccgcggacttgaagttccgcattaagcagaagggggaataccttccgctgcttcaaggaaagagcctcggcatgatctttgagaagcgctcaaccaggacccgcctttctactgaaactgggttcgcgctgctcggtggccacccctgcttcctgacgacccaggacatccacctcggagtgaacgaatccctcaccgataccgcccgggtgttatcgagcatggcagatgccgtgctggccagggtgtacaaacagtccgatctggacactctggccaaggaggcgtcaattcctattatcaacggccttagtgacctctaccatccgattcagatcctggccgattacctcaccctgcaagaacactacagctccctgaagggtctgacattgtcctggatcggcgacggcaacaacattctccattccatcatgatgtccgccgcaaaattcggcatgcatcttcaagccgccacgccgaagggttacgagcccgacgcttccgtgactaagctcgccgagcagtacgctaaggagaacggaaccaagcttctgctgactaacgacccactagaagcagcccacgggggcaacgtgcttattactgacacctggatctccatgggccaggaagaagagaaaaagaagcggctgcaggcgttccagggatatcaggtcaccatgaaaaccgccaaggtcgctgcctccgactggaccttcctgcactgcctgcctcgcaagcctgaagaagtggacgacgaggtgttctactcgccacggagcctcgtgttccccgaggccgagaatagaaagtggaccatcatggccgtgatggtgtcactgctcaccgactacagcccgcagcttcagaagcccaagttctagataagtgaactcgagctagtgactgactaggatctggttaccactaaaccagcctcaagaacacccgaatggagtctctaagctacataataccaacttacacttacaaaatgttgtcccccaaaatgtagccattcgtatctgctcctaataaaaagaaagtttcttcacattctag

SEQ ID NO: 110 - RNA, 1377 nt, synthetic construct
  source 1..1377: mol_type = other RNA
tcaacacaacatatacaaaacaaacgaatctcaagcaatcaagcattctacttctattgcagcaatttaaatcatttcttttaaagcaaaagcaattttctgaaaattttcaccatttacgaacgatagccatggcccttgtcaatctccgcatcctccttaacaacgccgcgtttagaaacggccacaacttcatggtccggaacttcagatgtggccagccgcttcaaggcagggtccagctgaagggccgggatcttctgaccctgaagaactttactggcgaagagatcaagtacatgctctggctctccgcggacttgaagttccgcattaagcagaagggggaataccttccgctgcttcaaggaaagagcctcggcatgatctttgagaagcgctcaaccaggacccgcctttctactgaaactgggttcgcgctgctcggtggccacccctgcttcctgacgacccaggacatccacctcggagtgaacgaatccctcaccgataccgcccgggtgttatcgagcatggcagatgccgtgctggccagggtgtacaaacagtccgatctggacactctggccaaggaggcgtcaattcctattatcaacggccttagtgacctctaccatccgattcagatcctggccgattacctcaccctgcaagaacactacagctccctgaagggtctgacattgtcctggatcggcgacggcaacaacattctccattccatcatgatgtccgccgcaaaattcggcatgcatcttcaagccgccacgccgaagggttacgagcccgacgcttccgtgactaagctcgccgagcagtacgctaaggagaacggaaccaagcttctgctgactaacgacccactagaagcagcccacgggggcaacgtgcttattactgacacctggatctccatgggccaggaagaagagaaaaagaagcggctgcaggcgttccagggatatcaggtcaccatgaaaaccgccaaggtcgctgcctccgactggaccttcctgcactgcctgcctcgcaagcctgaagaagtggacgacgaggtgttctactcgccacggagcctcgtgttccccgaggccgagaatagaaagtggaccatcatggccgtgatggtgtcactgctcaccgactacagcccgcagcttcagaagcccaagttctaagtgaatagactcgagctagtgactgactaggatctggttaccactaaaccagcctcaagaacacccgaatggagtctctaagctacataataccaacttacacttacaaaatgttgtcccccaaaatgtagccattcgtatctgctcctaataaaaagaaagtttcttcacattctag

SEQ ID NO: 111 - RNA, 1496 nt, synthetic construct
  source 1..1496: mol_type = other RNA
tcaacacaacatatacaaaacaaacgaatctcaagcaatcaagcattctacttctattgcagcaatttaaatcatttcttttaaagcaaaagcaattttctgaaaattttcaccatttacgaacgatagccatggcccttttcaatctccgcatcctccttaacaacgccgcgtttagaaacggccacaacttcatggtccggaacttcagatgtggccagccgcttcaagtcaaggtccagctgaagggccgggatcttctgaccctgaagaactttactggcgaagagatcaagtacatgctctggctctccgcggacttgaagttccgcattaagcagaagggggaataccttccgctgcttcaaggaaagagcctcggcatgatctttgagaagcgctcaaccaggacccgcctttctactgaaactgggttcgcgctgctcggtggccacccctgcttcctgacgacccaggacatccacctcggagtgaacgaatccctcaccgataccgcccgggtgttatcgagcatggcagatgccgtgctggccagggtgtacaaacagtccgatctggacactctggccaaggaggcgtcaattcctattatcaacggccttagtgacctctaccatccgattcagatcctggccgattacctcaccctgcaagaacactacagctccctgaagggtctgacattgtcctggatcggcgacggcaacaacattctccattccatcatgatgtccgccgcaaaattcggcatgcatcttcaagccgccacgccgaagggttacgagcccgacgcttccgtgactaagctcgccgagcagtacgctaaggagaacggaaccaagcttctgctgactaacgacccactagaagcagcccacgggggcaacgtgcttattactgacacctggatctccatgggccaggaagaagagaaaaagaagcggctgcaggcgttccagggatatcaggtcaccatgaaaaccgccaaggtcgctgcctccgactggaccttcctgcactgcctgcctcgcaagcctgaagaagtggacgacgaggtgttctactcgccacggagcctcgtgttccccgaggccgagaatagaaagtggaccatcatggccgtgatggtgtcactgctcaccgactacagcccgcagcttcagaagcccaagttctagataagtgaactcgagctagtgactgactaggatctggttaccactaaaccagcctcaagaacacccgaatggagtctctaagctacataataccaacttacacttacaaaatgttgtcccccaaaatgtagccattcgtatctgctcctaataaaaagaaagtttcttcacattctagaaaaaaaaaaaaaaaaaaaaaaaaaaaaaaaaaaaaaaaaaaaaaaaaaaaaaaaaaaaaaaaaaaaaaaaaaaaaaaaaaaaaaaaaaaaaaaaaaaaaaaaaaaaaaaaaaaaaaaa

SEQ ID NO: 112 - RNA, 1377 nt, synthetic construct
  source 1..1377: mol_type = other RNA
tcaacacaacatatacaaaacaaacgaatctcaagcaatcaagcattctacttctattgcagcaatttaaatcatttcttttaaagcaaaagcaattttctgaaaattttcaccatttacgaacgatagccatggcccttttcaatctccgcatcctccttaacaacgccgcgtttagaaacggccacaacttcatggtccggaacttcagatgtggccagccgcttcaagtcagggtccagctgaagggccgggatcttctgaccctgaagaactttactggcgaagagatcaagtacatgctctggctctccgcggacttgaagttccgcattaagcagaagggggaataccttccgctgcttcaaggaaagagcctcggcatgatctttgagaagcgctcaaccaggacccgcctttctactgaaactgggttcgcgctgctcggtggccacccctgcttcctgacgacccaggacatccacctcggagtgaacgaatccctcaccgataccgcccgggtgttatcgagcatggcagatgccgtgctggccagggtgtacaaacagtccgatctggacactctggccaaggaggcgtcaattcctattatcaacggccttagtgacctctaccatccgattcagatcctggccgattacctcaccctgcaagaacactacagctccctgaagggtctgacattgtcctggatcggcgacggcaacaacattctccattccatcatgatgtccgccgcaaaattcggcatgcatcttcaagccgccacgccgaagggttacgagcccgacgcttccgtgactaagctcgccgagcagtacgctaaggagaacggaaccaagcttctgctgactaacgacccactagaagcagcccacgggggcaacgtgcttattactgacacctggatctccatgggccaggaagaagagaaaaagaagcggctgcaggcgttccagggatatcaggtcaccatgaaaaccgccaaggtcgctgcctccgactggaccttcctgcactgcctgcctcgcaagcctgaagaagtggacgacgaggtgttctactcgccacggagcctcgtgttccccgaggccgagaatagaaagtggaccatcatggccgtgatggtgtcactgctcaccgactacagcccgcagcttcagaagcccaagttctagataagtgaactcgagctagtgactgactaggatctggttaccactaaaccagcctcaagaacacccgaatggagtctctaagctacataataccaacttacacttacaaaatgttgtcccccaaaatgtagccattcgtatctgctcctaataaaaagaaagtttcttcacattctag

SEQ ID NO: 113 - RNA, 1282 nt, synthetic construct
  source 1..1282: mol_type = other RNA
ggcagaaaaatttgctacattgtttcacaaacttcaaatattattcatttatttagatctattattacatcaaaacaaaaagccgccaccatgctgttcaacctgcgcatcctgctgaacaacgccgccttccgcaacggccacaacttcatggtgcgcaacttccgctgcggccagcccctgcagaacaaggtgcagctgaagggccgcgacctgctgaccctgaagaacttcaccggcgaggagatcaagtacatgctgtggctgagcgccgacctgaagttccgcatcaagcagaagggcgagtacctgcccctgctgcagggcaagagcctgggcatgatcttcgagaagcgcagcacccgcacccgcctgagcaccgagacaggcttcgccctgctgggcggccacccctgcttcctgaccacccaggacatccacctgggcgtgaacgagagcctgaccgacaccgcccgcgtgctgagcagcatggccgacgccgtgctggcccgcgtgtacaagcagagcgacctggacaccctggccaaggaggccagcatccccatcatcaacggcctgagcgacctgtaccaccccatccagatcctggccgactacctgaccctgcaggagcactacagcagcctgaagggcctgaccctgagctggatcggcgacggcaacaacatcctgcacagcatcatgatgagcgccgccaagttcggcatgcacctgcaggccgccacccccaagggctacgagcccgacgccagcgtgaccaagctggccgagcagtacgccaaggagaacggcaccaagctgctgctgaccaacgaccccctggaggccgcccacggcggcaacgtgctgatcaccgacacctggatcagcatgggccaggaggaggagaagaagaagcgcctgcaggccttccagggctaccaggtgaccatgaagaccgccaaggtggccgccagcgactggaccttcctgcactgcctgccccgcaagcccgaggaggtggacgacgaggtgttctacagcccccgcagcctggtgttccccgaggccgagaaccgcaagtggaccatcatggccgtgatggtgagcctgctgaccgactacagcccccagctgcagaagcccaagttctgaggtctctagtaatgagctggagcctcggtagccgttcctcctgcccgctgggcctcccaacgggccctcctcccctccttgcaccggcccttcctggtctttgaataaagtctgagtgggcatctag

SEQ ID NO: 114 - RNA, 1285 nt, synthetic construct
  source 1..1285: mol_type = other RNA
ggcagaaaaatttgctacattgtttcacaaacttcaaatattattcatttatttagatctattattacatcaaaacaaaaagccgccaccatgggagtattcaacctgcgcatcctgctgaacaacgccgccttccgcaacggccacaacttcatggtgcgcaacttccgctgcggccagcccctgcagaacaaggtgcagctgaagggccgcgacctgctgaccctgaagaacttcaccggcgaggagatcaagtacatgctgtggctgagcgccgacctgaagttccgcatcaagcagaagggcgagtacctgcccctgctgcagggcaagagcctgggcatgatcttcgagaagcgcagcacccgcacccgcctgagcaccgagacaggcttcgccctgctgggcggccacccctgcttcctgaccacccaggacatccacctgggcgtgaacgagagcctgaccgacaccgcccgcgtgctgagcagcatggccgacgccgtgctggcccgcgtgtacaagcagagcgacctggacaccctggccaaggaggccagcatccccatcatcaacggcctgagcgacctgtaccaccccatccagatcctggccgactacctgaccctgcaggagcactacagcagcctgaagggcctgaccctgagctggatcggcgacggcaacaacatcctgcacagcatcatgatgagcgccgccaagttcggcatgcacctgcaggccgccacccccaagggctacgagcccgacgccagcgtgaccaagctggccgagcagtacgccaaggagaacggcaccaagctgctgctgaccaacgaccccctggaggccgcccacggcggcaacgtgctgatcaccgacacctggatcagcatgggccaggaggaggagaagaagaagcgcctgcaggccttccagggctaccaggtgaccatgaagaccgccaaggtggccgccagcgactggaccttcctgcactgcctgccccgcaagcccgaggaggtggacgacgaggtgttctacagcccccgcagcctggtgttccccgaggccgagaaccgcaagtggaccatcatggccgtgatggtgagcctgctgaccgactacagcccccagctgcagaagcccaagttctgaggtctctagtaatgagctggagcctcggtagccgttcctcctgcccgctgggcctcccaacgggccctcctcccctccttgcaccggcccttcctggtctttgaataaagtctgagtgggcatctag

SEQ ID NO: 115 - RNA, 1285 nt, synthetic construct
  source 1..1285: mol_type = other RNA
ggcagaaaaatttgctacattgtttcacaaacttcaaatattattcatttatttagatctattattacatcaaaacaaaaagccgccaccatgggagtattcaacctgcgcatcctgctgaacaacgccgccttccgcaacggccacaacttcatggtgcgcaacttccgctgcggccagcccctgcagaaccgggtgcagctgaagggccgcgacctgctgaccctgaagaacttcaccggcgaggagatccggtacatgctgtggctgagcgccgacctgaagttccgcatcaagcagaagggcgagtacctgcccctgctgcagggcaagagcctgggcatgatcttcgagaagcgcagcacccgcacccgcctgagcaccgagacaggcttcgccctgctgggcggccacccctgcttcctgaccacccaggacatccacctgggcgtgaacgagagcctgaccgacaccgcccgcgtgctgagcagcatggccgacgccgtgctggcccgcgtgtacaagcagagcgacctggacaccctggccaaggaggccagcatccccatcatcaacggcctgagcgacctgtaccaccccatccagatcctggccgactacctgaccctgcaggagcactacagcagcctgaagggcctgaccctgagctggatcggcgacggcaacaacatcctgcacagcatcatgatgagcgccgccaagttcggcatgcacctgcaggccgccacccccaagggctacgagcccgacgccagcgtgaccaagctggccgagcagtacgccaaggagaacggcaccaagctgctgctgaccaacgaccccctggaggccgcccacggcggcaacgtgctgatcaccgacacctggatcagcatgggccaggaggaggagaagaagaagcgcctgcaggccttccagggctaccaggtgaccatgaagaccgccaaggtggccgccagcgactggaccttcctgcactgcctgccccgcaagcccgaggaggtggacgacgaggtgttctacagcccccgcagcctggtgttccccgaggccgagaaccgcaagtggaccatcatggccgtgatggtgagcctgctgaccgactacagcccccagctgcagaagcccaagttctgaggtctctagtaatgagctggagcctcggtagccgttcctcctgcccgctgggcctcccaacgggccctcctcccctccttgcaccggcccttcctggtctttgaataaagtctgagtgggcatctag

SEQ ID NO: 116 - RNA, 1285 nt, synthetic construct
  source 1..1285: mol_type = other RNA
ggcagaaaaatttgctacattgtttcacaaacttcaaatattattcatttatttagatctattattacatcaaaacaaaaagccgccaccatgctggtattcaacctgcgcatcctgctgaacaacgccgccttccgcaacggccacaacttcatggtgcgcaacttccgctgcggccagcccctgcagaaccgggtgcagctgaagggccgcgacctgctgaccctgaagaacttcaccggcgaggagatccggtacatgctgtggctgagcgccgacctgaagttccgcatcaagcagaagggcgagtacctgcccctgctgcagggcaagagcctgggcatgatcttcgagaagcgcagcacccgcacccgcctgagcaccgagacaggcttcgccctgctgggcggccacccctgcttcctgaccacccaggacatccacctgggcgtgaacgagagcctgaccgacaccgcccgcgtgctgagcagcatggccgacgccgtgctggcccgcgtgtacaagcagagcgacctggacaccctggccaaggaggccagcatccccatcatcaacggcctgagcgacctgtaccaccccatccagatcctggccgactacctgaccctgcaggagcactacagcagcctgaagggcctgaccctgagctggatcggcgacggcaacaacatcctgcacagcatcatgatgagcgccgccaagttcggcatgcacctgcaggccgccacccccaagggctacgagcccgacgccagcgtgaccaagctggccgagcagtacgccaaggagaacggcaccaagctgctgctgaccaacgaccccctggaggccgcccacggcggcaacgtgctgatcaccgacacctggatcagcatgggccaggaggaggagaagaagaagcgcctgcaggccttccagggctaccaggtgaccatgaagaccgccaaggtggccgccagcgactggaccttcctgcactgcctgccccgcaagcccgaggaggtggacgacgaggtgttctacagcccccgcagcctggtgttccccgaggccgagaaccgcaagtggaccatcatggccgtgatggtgagcctgctgaccgactacagcccccagctgcagaagcccaagttctgaggtctctagtaatgagctggagcctcggtagccgttcctcctgcccgctgggcctcccaacgggccctcctcccctccttgcaccggcccttcctggtctttgaataaagtctgagtgggcatctag

SEQ ID NO: 117 - RNA, 1225 nt, synthetic construct
  source 1..1225: mol_type = other RNA
attattacatcaaaacaaaaagccgccaccatgggagtattcaacctgcgcatcctgctgaacaacgccgccttccgcaacggccacaacttcatggtgcgcaacttccgctgcggccagcccctgcagaacaaggtgcagctgaagggccgcgacctgctgaccctgaagaacttcaccggcgaggagatcaagtacatgctgtggctgagcgccgacctgaagttccgcatcaagcagaagggcgagtacctgcccctgctgcagggcaagagcctgggcatgatcttcgagaagcgcagcacccgcacccgcctgagcaccgagacaggcttcgccctgctgggcggccacccctgcttcctgaccacccaggacatccacctgggcgtgaacgagagcctgaccgacaccgcccgcgtgctgagcagcatggccgacgccgtgctggcccgcgtgtacaagcagagcgacctggacaccctggccaaggaggccagcatccccatcatcaacggcctgagcgacctgtaccaccccatccagatcctggccgactacctgaccctgcaggagcactacagcagcctgaagggcctgaccctgagctggatcggcgacggcaacaacatcctgcacagcatcatgatgagcgccgccaagttcggcatgcacctgcaggccgccacccccaagggctacgagcccgacgccagcgtgaccaagctggccgagcagtacgccaaggagaacggcaccaagctgctgctgaccaacgaccccctggaggccgcccacggcggcaacgtgctgatcaccgacacctggatcagcatgggccaggaggaggagaagaagaagcgcctgcaggccttccagggctaccaggtgaccatgaagaccgccaaggtggccgccagcgactggaccttcctgcactgcctgccccgcaagcccgaggaggtggacgacgaggtgttctacagcccccgcagcctggtgttccccgaggccgagaaccgcaagtggaccatcatggccgtgatggtgagcctgctgaccgactacagcccccagctgcagaagcccaagttctgaggtctctagtaatgagctggagcctcggtagccgttcctcctgcccgctgggcctcccaacgggccctcctcccctccttgcaccggcccttcctggtctttgaataaagtctgagtgggcatctag

SEQ ID NO: 118 - RNA, 1225 nt, synthetic construct
  source 1..1225: mol_type = other RNA
attattacatcaaaacaaaaagccgccaccatgggagtattcaacctgcgcatcctgctgaacaacgccgccttccgcaacggccacaacttcatggtgcgcaacttccgctgcggccagcccctgcagaaccgggtgcagctgaagggccgcgacctgctgaccctgaagaacttcaccggcgaggagatccggtacatgctgtggctgagcgccgacctgaagttccgcatcaagcagaagggcgagtacctgcccctgctgcagggcaagagcctgggcatgatcttcgagaagcgcagcacccgcacccgcctgagcaccgagacaggcttcgccctgctgggcggccacccctgcttcctgaccacccaggacatccacctgggcgtgaacgagagcctgaccgacaccgcccgcgtgctgagcagcatggccgacgccgtgctggcccgcgtgtacaagcagagcgacctggacaccctggccaaggaggccagcatccccatcatcaacggcctgagcgacctgtaccaccccatccagatcctggccgactacctgaccctgcaggagcactacagcagcctgaagggcctgaccctgagctggatcggcgacggcaacaacatcctgcacagcatcatgatgagcgccgccaagttcggcatgcacctgcaggccgccacccccaagggctacgagcccgacgccagcgtgaccaagctggccgagcagtacgccaaggagaacggcaccaagctgctgctgaccaacgaccccctggaggccgcccacggcggcaacgtgctgatcaccgacacctggatcagcatgggccaggaggaggagaagaagaagcgcctgcaggccttccagggctaccaggtgaccatgaagaccgccaaggtggccgccagcgactggaccttcctgcactgcctgccccgcaagcccgaggaggtggacgacgaggtgttctacagcccccgcagcctggtgttccccgaggccgagaaccgcaagtggaccatcatggccgtgatggtgagcctgctgaccgactacagcccccagctgcagaagcccaagttctgaggtctctagtaatgagctggagcctcggtagccgttcctcctgcccgctgggcctcccaacgggccctcctcccctccttgcaccggcccttcctggtctttgaataaagtctgagtgggcatctag

SEQ ID NO: 119 - RNA, 1225 nt, synthetic construct
  source 1..1225: mol_type = other RNA
attattacatcaaaacaaaaagccgccaccatgctggtattcaacctgcgcatcctgctgaacaacgccgccttccgcaacggccacaacttcatggtgcgcaacttccgctgcggccagcccctgcagaaccgggtgcagctgaagggccgcgacctgctgaccctgaagaacttcaccggcgaggagatccggtacatgctgtggctgagcgccgacctgaagttccgcatcaagcagaagggcgagtacctgcccctgctgcagggcaagagcctgggcatgatcttcgagaagcgcagcacccgcacccgcctgagcaccgagacaggcttcgccctgctgggcggccacccctgcttcctgaccacccaggacatccacctgggcgtgaacgagagcctgaccgacaccgcccgcgtgctgagcagcatggccgacgccgtgctggcccgcgtgtacaagcagagcgacctggacaccctggccaaggaggccagcatccccatcatcaacggcctgagcgacctgtaccaccccatccagatcctggccgactacctgaccctgcaggagcactacagcagcctgaagggcctgaccctgagctggatcggcgacggcaacaacatcctgcacagcatcatgatgagcgccgccaagttcggcatgcacctgcaggccgccacccccaagggctacgagcccgacgccagcgtgaccaagctggccgagcagtacgccaaggagaacggcaccaagctgctgctgaccaacgaccccctggaggccgcccacggcggcaacgtgctgatcaccgacacctggatcagcatgggccaggaggaggagaagaagaagcgcctgcaggccttccagggctaccaggtgaccatgaagaccgccaaggtggccgccagcgactggaccttcctgcactgcctgccccgcaagcccgaggaggtggacgacgaggtgttctacagcccccgcagcctggtgttccccgaggccgagaaccgcaagtggaccatcatggccgtgatggtgagcctgctgaccgactacagcccccagctgcagaagcccaagttctgaggtctctagtaatgagctggagcctcggtagccgttcctcctgcccgctgggcctcccaacgggccctcctcccctccttgcaccggcccttcctggtctttgaataaagtctgagtgggcatctag

SEQ ID NO: 120 - RNA, 1376 nt, synthetic construct
  source 1..1376: mol_type = other RNA
tcaacacaacatatacaaaacaaacgaatctcaagcaatcaagcattctacttctattgcagcaatttaaatcatttcttttaaagcaaaagcaattttctgaaaattttcaccatttacgaacgatagccaccatgttgttcaacttgaggatcttgttgaacaacgccgccttcaggaacggacacaacttcatggtaaggaacttcaggtgcggacagcccttgcagaacaaagtacagttgaaaggaagggacttgttgacattgaaaaacttcacaggagaagaaatcaaatacatgttgtggttgtcggccgacttgaaattcaggatcaaacagaaaggagaatacttgcccttgttgcagggaaaatcgttgggaatgatcttcgaaaaaaggtcgacaaggacaaggttgtcgacagaaacaggattcgccttgttgggaggacacccctgcttcttgacaacacaggacatccacttgggagtaaacgaatcgttgacagacacagccagggtattgtcgtcgatggccgacgccgtattggccagggtatacaaacagtcggacttggacacattggccaaagaagcctcgatccccatcatcaacggattgtcggacttgtaccaccccatccagatcttggccgactacttgacattgcaggaacactactcgtcgttgaaaggattgacattgtcgtggatcggagacggaaacaacatcttgcactcgatcatgatgtcggccgccaaattcggaatgcacttgcaggccgccacacccaaaggatacgaacccgacgcctcggtaacaaaattggccgaacagtacgccaaagaaaacggaacaaaattgttgttgacaaacgaccccttggaagccgcccacggaggaaacgtattgatcacagacacatggatctcgatgggacaggaagaagaaaaaaaaaaaaggttgcaggccttccagggataccaggtaacaatgaaaacagccaaagtagccgcctcggactggacattcttgcactgcttgcccaggaaacccgaagaagtagacgacgaagtattctactcgcccaggtcgttggtattccccgaagccgaaaacaggaaatggacaatcatggccgtaatggtatcgttgttgacagactactcgccccagttgcagaaacccaaattctgaatagtgaactcgagctagtgactgactaggatctggttaccactaaaccagcctcaagaacacccgaatggagtctctaagctacataataccaacttacacttacaaaatgttgtcccccaaaatgtagccattcgtatctgctcctaataaaaagaaagtttcttcacattctag

SEQ ID NO: 121 - RNA, 1222 nt, synthetic construct
  source 1..1222: mol_type = other RNA
attattacatcaaaacaaaaagccgccaccatgctgttcaacctgcgcatcctgctgaacaacgccgccttccgcaacggccacaacttcatggtgcgcaacttccgctgcggccagcccctgcagggcaaggtgcagctgaagggccgcgacctgctgaccctgaagaacttcaccggcgaggagatcaagtacatgctgtggctgagcgccgacctgaagttccgcatcaagcagaagggcgagtacctgcccctgctgcagggcaagagcctgggcatgatcttcgagaagcgcagcacccgcacccgcctgagcaccgagacaggcttcgccctgctgggcggccacccctgcttcctgaccacccaggacatccacctgggcgtgaacgagagcctgaccgacaccgcccgcgtgctgagcagcatggccgacgccgtgctggcccgcgtgtacaagcagagcgacctggacaccctggccaaggaggccagcatccccatcatcaacggcctgagcgacctgtaccaccccatccagatcctggccgactacctgaccctgcaggagcactacagcagcctgaagggcctgaccctgagctggatcggcgacggcaacaacatcctgcacagcatcatgatgagcgccgccaagttcggcatgcacctgcaggccgccacccccaagggctacgagcccgacgccagcgtgaccaagctggccgagcagtacgccaaggagaacggcaccaagctgctgctgaccaacgaccccctggaggccgcccacggcggcaacgtgctgatcaccgacacctggatcagcatgggccaggaggaggagaagaagaagcgcctgcaggccttccagggctaccaggtgaccatgaagaccgccaaggtggccgccagcgactggaccttcctgcactgcctgccccgcaagcccgaggaggtggacgacgaggtgttctacagcccccgcagcctggtgttccccgaggccgagaaccgcaagtggaccatcatggccgtgatggtgagcctgctgaccgactacagcccccagctgcagaagcccaagttctgaggtctctagtaatgagctggagcctcggtagccgttcctcctgcccgctgggcctcccaacgggccctcctcccctccttgcaccggcccttcctggtctttgaataaagtctgagtgggcatctag

SEQ ID NO: 122 - RNA, 1222 nt, synthetic construct
  source 1..1222: mol_type = other RNA
attattacatcaaaacaaaaagccgccaccatgctgttcaacctgcgcatcctgctgaacaacgccgccttccgcaacggccacaacttcatggtgcgcaacttccgctgcggccagcccctgcagggccgggtgcagctgaagggccgcgacctgctgaccctgaagaacttcaccggcgaggagatcaagtacatgctgtggctgagcgccgacctgaagttccgcatcaagcagaagggcgagtacctgcccctgctgcagggcaagagcctgggcatgatcttcgagaagcgcagcacccgcacccgcctgagcaccgagacaggcttcgccctgctgggcggccacccctgcttcctgaccacccaggacatccacctgggcgtgaacgagagcctgaccgacaccgcccgcgtgctgagcagcatggccgacgccgtgctggcccgcgtgtacaagcagagcgacctggacaccctggccaaggaggccagcatccccatcatcaacggcctgagcgacctgtaccaccccatccagatcctggccgactacctgaccctgcaggagcactacagcagcctgaagggcctgaccctgagctggatcggcgacggcaacaacatcctgcacagcatcatgatgagcgccgccaagttcggcatgcacctgcaggccgccacccccaagggctacgagcccgacgccagcgtgaccaagctggccgagcagtacgccaaggagaacggcaccaagctgctgctgaccaacgaccccctggaggccgcccacggcggcaacgtgctgatcaccgacacctggatcagcatgggccaggaggaggagaagaagaagcgcctgcaggccttccagggctaccaggtgaccatgaagaccgccaaggtggccgccagcgactggaccttcctgcactgcctgccccgcaagcccgaggaggtggacgacgaggtgttctacagcccccgcagcctggtgttccccgaggccgagaaccgcaagtggaccatcatggccgtgatggtgagcctgctgaccgactacagcccccagctgcagaagcccaagttctgaggtctctagtaatgagctggagcctcggtagccgttcctcctgcccgctgggcctcccaacgggccctcctcccctccttgcaccggcccttcctggtctttgaataaagtctgagtgggcatctag

SEQ ID NO: 123 - RNA, 1222 nt, synthetic construct
  source 1..1222: mol_type = other RNA
attattacatcaaaacaaaaagccgccaccatgctgttcaacctgcgcatcctgctgaacaacgccgccttccgcaacggccacaacttcatggtgcgcaacttccgctgcggccagcccctgcagggccgggtgcagctgaagggccgcgacctgctgaccctgaagaacttcaccggcgaggagatccggtacatgctgtggctgagcgccgacctgaagttccgcatcaagcagaagggcgagtacctgcccctgctgcagggcaagagcctgggcatgatcttcgagaagcgcagcacccgcacccgcctgagcaccgagacaggcttcgccctgctgggcggccacccctgcttcctgaccacccaggacatccacctgggcgtgaacgagagcctgaccgacaccgcccgcgtgctgagcagcatggccgacgccgtgctggcccgcgtgtacaagcagagcgacctggacaccctggccaaggaggccagcatccccatcatcaacggcctgagcgacctgtaccaccccatccagatcctggccgactacctgaccctgcaggagcactacagcagcctgaagggcctgaccctgagctggatcggcgacggcaacaacatcctgcacagcatcatgatgagcgccgccaagttcggcatgcacctgcaggccgccacccccaagggctacgagcccgacgccagcgtgaccaagctggccgagcagtacgccaaggagaacggcaccaagctgctgctgaccaacgaccccctggaggccgcccacggcggcaacgtgctgatcaccgacacctggatcagcatgggccaggaggaggagaagaagaagcgcctgcaggccttccagggctaccaggtgaccatgaagaccgccaaggtggccgccagcgactggaccttcctgcactgcctgccccgcaagcccgaggaggtggacgacgaggtgttctacagcccccgcagcctggtgttccccgaggccgagaaccgcaagtggaccatcatggccgtgatggtgagcctgctgaccgactacagcccccagctgcagaagcccaagttctgaggtctctagtaatgagctggagcctcggtagccgttcctcctgcccgctgggcctcccaacgggccctcctcccctccttgcaccggcccttcctggtctttgaataaagtctgagtgggcatctag

SEQ ID NO: 124 - RNA, 1282 nt, synthetic construct
  source 1..1282: mol_type = other RNA
ggcagaaaaatttgctacattgtttcacaaacttcaaatattattcatttatttagatctattattacatcaaaacaaaaagccgccaccatgctgttcaacctgcgcatcctgctgaacaacgccgccttccgcaacggccacaacttcatggtgcgcaacttccgctgcggccagcccctgcagggcaaggtgcagctgaagggccgcgacctgctgaccctgaagaacttcaccggcgaggagatcaagtacatgctgtggctgagcgccgacctgaagttccgcatcaagcagaagggcgagtacctgcccctgctgcagggcaagagcctgggcatgatcttcgagaagcgcagcacccgcacccgcctgagcaccgagacaggcttcgccctgctgggcggccacccctgcttcctgaccacccaggacatccacctgggcgtgaacgagagcctgaccgacaccgcccgcgtgctgagcagcatggccgacgccgtgctggcccgcgtgtacaagcagagcgacctggacaccctggccaaggaggccagcatccccatcatcaacggcctgagcgacctgtaccaccccatccagatcctggccgactacctgaccctgcaggagcactacagcagcctgaagggcctgaccctgagctggatcggcgacggcaacaacatcctgcacagcatcatgatgagcgccgccaagttcggcatgcacctgcaggccgccacccccaagggctacgagcccgacgccagcgtgaccaagctggccgagcagtacgccaaggagaacggcaccaagctgctgctgaccaacgaccccctggaggccgcccacggcggcaacgtgctgatcaccgacacctggatcagcatgggccaggaggaggagaagaagaagcgcctgcaggccttccagggctaccaggtgaccatgaagaccgccaaggtggccgccagcgactggaccttcctgcactgcctgccccgcaagcccgaggaggtggacgacgaggtgttctacagcccccgcagcctggtgttccccgaggccgagaaccgcaagtggaccatcatggccgtgatggtgagcctgctgaccgactacagcccccagctgcagaagcccaagttctgaggtctctagtaatgagctggagcctcggtagccgttcctcctgcccgctgggcctcccaacgggccctcctcccctccttgcaccggcccttcctggtctttgaataaagtctgagtgggcatctag

SEQ ID NO: 125 - RNA, 21 nt, synthetic construct
  source 1..21: mol_type = other RNA
cacaaagagtaaagaagaaca

SEQ ID NO: 126 - RNA, 21 nt, synthetic construct
  source 1..21: mol_type = other RNA
aacactaaaagtagaagaaaa

SEQ ID NO: 127 - RNA, 21 nt, synthetic construct
  source 1..21: mol_type = other RNA
ctcagaaagataagatcagcc

SEQ ID NO: 128 - DNA, 1065 bp, synthetic construct; identical to SEQ ID NO: 2
  source 1..1065: mol_type = other DNA

SEQ ID NO: 129 - DNA, 1065 bp, synthetic construct
  source 1..1065: mol_type = other DNA
atgctctttaatctgcgcatcttactgaacaacgccgcattccggaacggtcacaacttcatggtccgcaatttccgctgtggccagccgcttcaaaacaaggtccagctgaagggacgggatctgctgacactgaagaacttcaccggagaagagatcaagtacatgctgtggctcagcgcagacttgaagttccggatcaagcagaagggagaatacttgcccctgctgcaaggaaagtcgctgggaatgatttttgagaagcggtcaactcgcaccagactctccaccgaaactggtttcgcactgcttggcgggcacccttgcttcctgacgactcaggacatccacctcggcgtgaacgaatcgctaaccgataccgccagagtgctttcttccatggccgacgcggtgctggccagggtgtacaagcagtccgacctcgataccttggcaaaggaggcttccattcccatcatcaacggcctgagcgacctgtaccacccaatccaaatcctggctgactacctgaccctgcaagagcactacagcagcctgaagggtctgaccctgtcatggattggcgatggaaacaatattctgcactccatcatgatgtccgccgcgaagttcggaatgcatctgcaagccgccactccaaaaggatacgaaccggatgcgtccgtgaccaagttggcggaacagtacgcgaaggagaacggaaccaagcttctgctgactaacgaccccctcgaggctgcgcatgggggcaacgtgctgattaccgacacctggatctccatggggcaggaggaagagaagaagaagagactgcaggcattccaggggtaccaggtcaccatgaaaaccgcaaaagtggcagcttcggactggactttcctgcattgcctgccgaggaagccggaggaagtcgacgacgaagtgttctactcgcctcggtccctggtgttccccgaggccgaaaaccggaagtggaccatcatggccgtgatggtgtccttgctgactgactatagcccgcagctgcagaagcctaagttctag

SEQ ID NO: 130 - DNA, 1065 bp, synthetic construct
  source 1..1065: mol_type = other DNA
atgctgtttaacctacgtattttgctcaacaatgcagcctttagaaacggacataactttatggttcgaaactttcgctgcgggcagccactgcagaacaaggtccagctgaaagggagagatttgctcacgctgaagaactttactggcgaagaaatcaagtatatgctgtggttgtccgcggacctcaagtttcggattaagcagaaaggggagtatctgccactgctgcaaggaaagagcctcggcatgatcttcgagaagcggagcactcggaccaggctgagtaccgaaactggcttcgcattgttgggtggacatccatgttttctgacaacgcaggacattcatctgggcgtgaacgagagtctgacggacacagctcgcgttctgtcctctatggctgatgcggtgttggcccgggtctataagcagtccgatttggacaccttggctaaggaagctagcataccgattatcaatgggctgtccgacctgtatcaccctattcaaatcctggccgactacctcacactgcaagaacactatagctcattgaagggactgaccctgagctggataggggacggaaacaacatcctacatagcattatgatgtccgctgccaagtttggcatgcatcttcaagccgccacgccaaagggttatgagcccgacgcgtcagtgacaaagctggccgagcagtacgctaaggagaatggtaccaaattactgctgactaatgatccactggaggctgcacatggcggcaatgtactgatcaccgacacatggatctcgatgggccaggaggaagaaaagaagaagaggcttcaggccttccaaggctaccaggtcaccatgaaaacagctaaggttgcagcatctgattggacctttctgcactgtctgccaaggaagcccgaagaggtggacgatgaagtattctatagcccacggagtttggtgttccctgaggctgaaaataggaagtggacaattatggccgtaatggtgtccctgttaaccgactactctccgcaactgcagaaacctaagttttag

SEQ ID NO: 131 - DNA, 1065 bp, synthetic construct
  source 1..1065: mol_type = other DNA
atgctgtttaacttaaggatcctgctgaacaacgccgcttttcgtaacggtcataactttatggtccggaactttagatgtggccagccgctgcagaacaaggttcagctgaaggggagggatctgctgaccttgaagaactttaccggcgaagagatcaagtacatgttgtggctgagcgccgatctgaagtttaggattaagcagaagggggagtatttgccactgctgcaaggaaaatccttggggatgatcttcgagaagcgctccactagaacccggctaagcacagaaaccggcttcgcacttctgggtggacatccctgttttctgacgacgcaggatatacacctgggcgtgaatgagagtctgacggacacagctagggtgttgagcagcatggccgatgcagtactggcccgcgtttataagcagagcgacttggacacactggccaaggaagcgtcaattccgattatcaatgggctgtcagacctgtatcatcccattcaaatcttggctgactatctgaccctgcaagaacattacagctccctgaagggcctcacgttgtcctggattggcgacggaaacaacattctgcattcgatcatgatgagcgctgctaagtttggcatgcacctccaagccgctacacctaagggatatgagcctgatgccagcgtaaccaagctggccgaacagtacgcgaaggagaatggcacgaaactgctgttgacaaatgacccactggaggcagctcacggtggcaacgtgctgatcaccgacacgtggatatctatgggacaggaagaagagaagaagaagcggctgcaggcattccaagggtatcaggtcaccatgaaaacggccaaggttgctgcatccgactggacatttctgcattgcttgccccgcaaaccagaagaagtagacgacgaagtcttttattccccacggtcgctggtgttccccgaggcggagaatcgaaagtggacgattatggccgtgatggtgtccctgctgactgattactctccccaactgcaaaagcctaagttttag

SEQ ID NO: 132 - DNA, 1065 bp, synthetic construct
  source 1..1065: mol_type = other DNA
atgcttttcaacctgaggatcctcctgaacaacgccgcctttcgcaatggtcacaactttatggtccggaacttcagatgcggccagccgctgcagaacaaggtccagctgaagggacgggatctgctgactctgaagaacttcaccggagaagagatcaagtacatgctgtggctgtcggccgacctgaagttcaggatcaagcagaagggagaatacctcccgctgctgcaaggaaagtccctgggcatgattttcgagaagcgctcgaccagaactcggttgtccaccgaaaccgggtttgcgctgctgggcggacatccttgcttcctgacgactcaggatattcacctgggagtgaacgagtcgctgaccgacaccgccagagtgctgagctcgatggccgacgccgtgttggcacgcgtgtacaagcagtccgatctggataccctggccaaagaagcttccatcccgatcattaacgggctgagcgacctctaccaccccattcaaatcctggccgactacctgactctgcaagaacactacagctcgctgaaggggttgactctgtcctggatcggcgacggaaacaacatcctgcactccatcatgatgtcggccgcaaagttcggcatgcatttgcaagccgccaccccaaagggctacgaaccagacgcgagcgtcaccaagctggccgaacagtacgcgaaggaaaatggtactaagctgctgctgaccaacgacccattggaagctgcccatggtggaaacgtgctgatcaccgacacctggatctcgatgggccaggaagaggagaagaagaagcggctgcaggcgttccaggggtatcaggtcaccatgaaaacagccaaagtggcagcgtcagactggaccttcctccactgtctgcctcgcaagccagaggaggtggacgacgaggtgttctactcccctcggtccctcgtgttccctgaggctgagaaccggaagtggaccattatggccgtgatggtgtcactcctgactgattactccccgcaactgcagaagcccaagttctag

SEQ ID NO: 133 - DNA, 1065 bp, synthetic construct
  source 1..1065: mol_type = other DNA
atgctgtttaacctgaggatcctattgaacaatgctgcttttcgtaatggccataactttatggttcggaactttagatgcgggcagccactgcagaacaaggtccagttgaaaggccgcgatctgttgacattgaagaactttaccggcgaagagattaagtatatgctgtggctgtctgctgacctcaagtttcgaatcaagcagaagggcgaatatctccccctgctgcaaggaaagtctctcggcatgatctttgagaagcggagtacccgaacacggctgagcaccgaaacgggcttcgcactgctggggggccatccctgttttctgacaacgcaggacatccacttgggggttaacgaatcattgactgataccgcccgcgtactgtcatccatggccgacgctgtgctggctagggtgtacaagcagtcagatctggatacactggccaaggaagctagcataccaatcatcaatggactgagtgacctttatcacccgattcaaatactagccgattatctgaccctgcaagagcattactcctcgctgaaaggcctcacgctgtcctggatcggcgacggcaacaacattctgcatagtattatgatgtctgctgccaaattcggcatgcatctgcaagctgctacgccgaagggttatgaacccgacgcgtcagttacgaagctcgctgagcagtatgcaaaggagaatggcacaaagctgttgcttaccaacgatcccctggaagctgctcatggcggcaatgtgctgattactgacacctggatttcaatgggccaggaggaggagaagaagaagaggttacaggcttttcaaggttaccaagtcacgatgaaaaccgctaaggtcgcagccagcgactggacattcctgcactgtctgccaagaaagccggaagaagtggacgacgaggtgttctattccccgcggtctttggtgtttccggaggccgaaaacaggaaatggaccattatggccgtgatggtatcgttgctgacggactacagccctcagttgcaaaagcccaagttctag

SEQ ID NO: 134 - DNA, 1065 bp, synthetic construct
  source 1..1065: mol_type = other DNA
atgctctttaacctccgcatcctcctcaacaacgccgccttccggaatgggcataacttcatggtccggaacttcagatgcggccagcccctgcaaaacaaggtccagttgaagggacgggacctccttacgctgaagaactttaccggagaagagattaagtacatgctgtggttgtccgctgacctcaagttccgcattaagcagaagggagaatatctgccgctgctgcaaggaaagagcctgggcatgatcttcgaaaagcgctccactagaacccggctgtcgactgagactggattcgccttgctcggtggacacccgtgcttcctgacgacccaggacatccacctgggagtgaacgagtcacttacggataccgcgagggtgctgtcctcaatggccgacgcagtgctcgcgcgcgtgtacaagcagtcagatctggataccctggccaaggaagccagcattcccatcatcaacggactgagcgacctttaccacccaatccagatcctcgccgactacttaaccctgcaagagcactacagctccctgaagggactgactctgtcctggatcggggatggaaacaacatcctgcactccatcatgatgtctgccgctaagtttgggatgcatctgcaagccgcaacccctaagggatacgagcccgacgcctcggtgaccaaacttgcggaacagtacgccaaggaaaacggtaccaagctgctgctgaccaacgaccctctggaagcggcccacggaggaaatgtgctgattaccgacacctggatttcgatgggccaggaggaggagaagaagaagagactgcaggcgttccagggatatcaggtcaccatgaaaaccgccaaggtcgccgccagcgactggaccttcctgcactgtctccctcggaaaccggaagaagtggatgacgaggtgttctactccccgcgctcgctggtgttcccggaggctgaaaacaggaagtggacaatcatggccgtgatggtgtccctgttgaccgactactccccacaactgcagaagcccaagttctag

SEQ ID NO: 135 - DNA, 1065 bp, synthetic construct
  source 1..1065: mol_type = other DNA
atgcttttcaatctgcgcatcctcctgaacaacgccgccttccgcaatggacacaactttatggtccgcaacttccgctgtgggcagccgctgcagaacaaggtccagctcaaggggagagatctcctgaccctgaagaacttcactggagaggagatcaagtacatgctgtggctgtccgccgacctgaaatttcggattaagcagaagggcgaatacctcccactgctgcaaggaaagtctttgggcatgatcttcgaaaagagaagcacccggacccggttgagcaccgaaactgggttcgcgctcctcggtggacacccgtgcttcctgaccacccaagatattcatctgggtgtcaacgaaagcctgaccgacaccgccagggtgctgtcatccatggctgacgcagtgctcgcccgggtgtacaagcagtcagacctggacaccctcgccaaggaagcttcgatccctatcatcaacggactttccgacctgtaccaccccatccaaattctggccgactacctgactctgcaagaacactatagctcgctgaaaggacttactctgtcctggatcggggacggcaacaacattctccattccatcatgatgtccgctgccaagttcggaatgcaccttcaagcagcgactcccaagggatacgaacctgatgcctccgtgactaagctggcagagcagtacgccaaggagaacggtacaaagctgctgctcacgaacgaccccctggaggcggcccacggcggaaacgtgctgattaccgatacctggatctcaatgggccaggaagaggagaagaagaagcggctccaggcgtttcaaggctaccaggtcaccatgaaaaccgcgaaggtcgccgcctccgactggactttcttgcactgcctgccgcggaagcccgaggaagtggatgacgaagtgttctactcgccgagatcgttggtgttccctgaggccgaaaacaggaagtggaccatcatggccgtgatggtgtccctgctgactgattacagcccacagctgcagaagcctaagttctag

SEQ ID NO: 136 - DNA, 1065 bp, synthetic construct
  source 1..1065: mol_type = other DNA
atgcttttcaatctccgcatcctccttaacaacgccgcgtttagaaacggccacaacttcatggtccggaacttcagatgtggccagccgcttcaaaacaaggtccagctgaagggccgggatcttctgaccctgaagaactttactggcgaagagatcaagtacatgctctggctctccgcggacttgaagttccgcattaagcagaagggggaataccttccgctgcttcaaggaaagagcctcggcatgatctttgagaagcgctcaaccaggacccgcctttctactgaaactgggttcgcgctgctcggtggccacccctgcttcctgacgacccaggacatccacctcggagtgaacgaatccctcaccgataccgcccgggtgttatcgagcatggcagatgccgtgctggccagggtgtacaaacagtccgatctggacactctggccaaggaggcgtcaattcctattatcaacggccttagtgacctctaccatccgattcagatcctggccgattacctcaccctgcaagaacactacagctccctgaagggtctgacattgtcctggatcggcgacggcaacaacattctccattccatcatgatgtccgccgcaaaattcggcatgcatcttcaagccgccacgccgaagggttacgagcccgacgcttccgtgactaagctcgccgagcagtacgctaaggagaacggaaccaagcttctgctgactaacgacccactagaagcagcccacgggggcaacgtgcttattactgacacctggatctccatgggccaggaagaagagaaaaagaagcggctgcaggcgttccagggatatcaggtcaccatgaaaaccgccaaggtcgctgcctccgactggaccttcctgcactgcctgcctcgcaagcctgaagaagtggacgacgaggtgttctactcgccacggagcctcgtgttccccgaggccgagaatagaaagtggaccatcatggccgtgatggtgtcactgctcaccgactacagcccgcagcttcagaagcccaagttctag

SEQ ID NO: 137 - DNA, 1065 bp, synthetic construct
  source 1..1065: mol_type = other DNA
atgcttttcaacctgagaatcctcctgaacaacgccgccttccgcaatggtcataacttcatggtccgcaactttcgctgcggacagcctctccaaaacaaggtccagctcaaggggcgcgacctcctcacactgaagaacttcactggagaagaaatcaagtacatgctgtggctgagcgccgatctgaagttccggatcaagcagaagggagagtaccttcctctgctgcaagggaagtccttgggaatgattttcgagaagcggtccacccggaccaggctgagcactgaaactggcttcgccctgctgggaggccacccttgtttcctgaccactcaggacatccacctgggcgtgaacgagtccctgaccgatactgccagagtgctgtcctccatggccgacgccgtgctcgcccgggtgtacaagcagtcagacctcgatacgctggccaaggaagcctccattcccattatcaatggtctgtcggacctctaccatccaatccaaatcctcgccgactacctgactctgcaagaacactacagctcactcaagggcctcaccctctcctggatcggcgacggaaacaacatccttcactcgattatgatgtcggccgcgaagttcgggatgcacctccaagctgccactccaaaaggctacgagccggatgcctcagtgactaagttggcggaacagtatgcgaaggagaacggtaccaagctcctgctgactaacgacccgctggaggccgcccacgggggaaacgtgctcatcaccgatacttggatttccatgggacaggaggaagagaagaagaagcggttgcaggcatttcagggctaccaggtcaccatgaaaactgccaaagtcgccgccagcgactggaccttcctgcactgcctgccccgcaagcctgaagaagtggacgacgaggtgttctactctccccggtccctcgtgttccctgaggccgaaaacaggaagtggaccatcatggctgtgatggtgtccctcctgaccgactacagccctcagctccaaaaacccaagttttag

SEQ ID NO: 138 - DNA, 1065 bp, synthetic construct
  source 1..1065: mol_type = other DNA
atgcttttcaacctgagaatcctcttgaacaatgctgcttttcggaatggccacaactttatggttcggaacttccgttgcggccagcctttacaaaacaaggtccagctgaagggccgggatttgctcacactgaagaactttactggggaggagattaagtatatgctgtggctgtccgctgacctgaagtttaggatcaagcagaagggcgaatatctgccgctgctgcaagggaaaagtctgggcatgatttttgaaaagcgctctacccggaccagactgtctacggaaacaggctttgccctgctgggcggccacccctgttttctgacaacgcaggacatccatctgggcgtgaacgaatcactgaccgatactgctcgggtactcagttctatggctgacgcagtgctggctagggtgtacaagcagagcgacttggacacactggctaaggaggccagcatccccattatcaatggcctgtctgatttgtaccatcccattcaaatcctggctgattatctgacactacaagagcattactcaagtctgaagggtttgactctctcctggatcggcgacggcaacaacattttacattccattatgatgagtgctgctaagtttggcatgcatttgcaagctgctaccccaaagggctatgaacctgacgctagcgtaaccaagttggccgaacagtatgctaaagagaatggcaccaagctgctcctgacgaatgaccccctggaagctgctcatggcggaaacgtacttataactgatacatggattagcatgggccaggaagaggagaagaagaagagactgcaggccttccaaggctatcaggtcaccatgaaaactgccaaggttgcagctagcgactggaccttcctgcactgtttgccgaggaaacccgaggaggtggacgatgaagtcttttattctccccgctccttggtgtttcccgaggctgaaaatcgaaagtggacgataatggcagtgatggtgtccctactgaccgactattctccacaactgcagaagcctaaattctag

SEQ ID NO: 139 - DNA, 1065 bp, synthetic construct
  source 1..1065: mol_type = other DNA
atgcttttcaatctgaggatcctgctgaacaacgctgcttttcgcaacggtcataactttatggttcgcaattttcgttgtggccagccgctgcagaacaaggttcagctgaagggcagagatctgctgactctgaagaacttcactggggaagaaatcaagtatatgttatggctgtccgcggatctgaaatttcgaatcaagcagaagggcgaatatcttcccctgctgcaagggaaatccttgggcatgatttttgagaagaggagcactaggactagattgtcaacagaaacaggctttgctttgttgggcggacatccctgctttctgacgacacaggatatccacctcggcgtaaacgagtccctcaccgacactgctagggtactgagcagcatggccgacgctgtgctagcccgggtttacaagcagtcagacctggacacccttgccaaggaagcttctattccaattatcaacggcctgagtgacctgtatcaccctattcaaatactcgccgactatttgacgcttcaagaacattacagcagcctcaagggcttaaccttgagttggataggcgacggcaacaatatcctgcattccattatgatgtctgccgctaagtttggcatgcatctacaagccgcaacacccaagggctatgaacccgacgctagcgtgaccaagctggccgagcagtatgctaaggaaaatggcacaaagctccttcttaccaacgatcccctggaggctgctcacggcggcaacgtgctgattaccgatacatggattagcatgggccaggaggaggagaaaaagaagcggctccaggcttttcaaggctatcaggtcaccatgaaaactgcaaaggtcgctgcctccgactggactttcctgcattgtctaccccgcaagcctgaggaagtggacgatgaggtgttctactccccacggagtctggtgttcccggaagcagagaatcggaagtggaccatcatggctgtcatggtgtcgctcttgactgactattctccccaactgcaaaaacccaagttttag

SEQ ID NO: 140 - DNA, 1065 bp, synthetic construct; identical to SEQ ID NO: 139
  source 1..1065: mol_type = other DNA

SEQ ID NO: 141 - DNA, 1065 bp, synthetic construct
  source 1..1065: mol_type = other DNA
atgctttttaatctccgcatcctccttaacaacgccgcgtttagaaacggccacaacttcatggtccggaacttcagatgtggccagccgcttcaaaacaaggtccagctgaagggccgggatcttctgaccctgaagaactttactggcgaagagatcaagtacatgctctggctctccgcggacttgaagttccgcattaagcagaagggggaataccttccgctgcttcaaggaaagagcctcggcatgatctttgagaagcgctcaaccaggacccgcctttctactgaaactgggttcgcgctgctcggtggccacccctgcttcctgacgacccaggacatccacctcggagtgaacgaatccctcaccgataccgcccgggtgttatcgagcatggcagatgccgtgctggccagggtgtacaaacagtccgatctggacactctggccaaggaggcgtcaattcccatcatcaacggcctgagcgacctgtaccacccaatccaaatcctggctgactacctgaccctgcaagagcactacagcagcctgaagggtctgaccctgtcatggattggcgatggaaacaatattctgcactccatcatgatgtccgccgcgaagttcggaatgcatctgcaagccgccacgccaaaaggatacgaaccggatgcgtccgtgacgaagttggcggaacagtacgcgaaggagaacggaaccaagcttctgctgactaacgaccccctcgaggctgcgcatgggggcaacgtgctgattaccgacacctggatctccatggggcaggaggaagagaagaagaagagactgcaggcattccaggggtaccaggtcaccatgaaaaccgcaaaagtggcagcttcggactggactttcctgcattgcctgccgaggaagccggaggaagtcgacgacgaagtgttctactcgcctcggtccctggtgttccccgaggccgaaaaccggaagtggaccatcatggccgtgatggtgtccttgctgactgactatagcccgcagctgcagaagcctaagttctag

SEQ ID NO: 142 - DNA, 1065 bp, synthetic construct
  source 1..1065: mol_type = other DNA
atgcttttcaacctgagaatcctcttgaacaatgctgcttttcggaatggccacaactttatggttcggaacttccgttgcggccagcctttacaaaacaaggtccagctgaagggccgggatttgctcacactgaagaactttactggagaagagatcaagtacatgctgtggctgtcggccgacctgaagttcaggatcaagcagaagggagaataccttccgctgcttcaaggaaagagcctcggcatgatctttgagaagcgctcaaccaggacccgcctttctactgaaactgggttcgcgctgctcggtggccacccctgcttcctgacgacccaggacatccacctcggagtgaacgaatccctcaccgataccgcccgggtgttatcgagcatggcagatgccgtgctggccagggtgtacaaacagtccgatctcgataccttggcaaaggaggcttccattcccatcatcaacggcctgagcgacctgtaccacccaatccaaatcctggctgactacctgaccctgcaagagcactacagcagcctgaagggtctgaccctgtcatggattggcgatggaaacaatattctgcactccatcatgatgtccgccgcgaagttcggaatgcatctgcaagccgccactccaaaaggatacgaaccggatgcgtccgtgaccaagttggcggaacagtacgcgaaggagaacggaaccaagcttctgctgactaacgaccccctcgaggctgcgcatgggggcaacgtgctgattaccgacacctggatctccatggggcaggaggaagagaagaagaagagactgcaggcattccaggggtaccaggtcaccatgaaaaccgcaaaagtggcagcttcggactggactttcctgcattgcctgccgaggaagccggaggaagtcgacgacgaagtgttctactcgcctcggtccctggtgttccccgaggccgaaaaccggaagtggaccatcatggccgtgatggtgtccttgctgactgactatagcccgcagctgcagaagcctaagttctag

SEQ ID NO: 143 - DNA, 1065 bp, synthetic construct
  source 1..1065: mol_type = other DNA
atgcttttcaacctgagaatcctcttgaacaatgctgcttttcggaatggccacaactttatggttcggaacttccgttgcggccagcctttacaaaacaaggtccagctgaagggccgggatttgctcacactaaagaactttactggagaagagatcaagtacatgctatggctgtcggccgacctgaagttccgtatcaagcagaagggagaataccttccgctgcttcaaggaaagagcctcggcatgatctttgagaagcgctcaaccaggacccgcctttctactgaaactgggttcgcgctgctcggtggccacccctgcttcctgacgacccaggacatccacctcggagtgaacgaatccctcaccgataccgcccgggtgttatcgagcatggcagatgccgtgctggccagggtgtacaaacagtccgatctcgataccttggcaaaggaggcttccattcccatcatcaacggcctgagcgacctgtaccacccaatccaaatcctggctgactacctgaccctgcaagagcactacagcagcctgaagggtctgaccctgtcatggattggcgatggaaacaatattctgcactccatcatgatgtccgccgcgaagttcggaatgcatctgcaagccgccactccaaaaggatacgaaccggatgcatccgtgaccaagttggcggaacagtacgcgaaggagaacggaaccaagctcctgctgactaacgacccgctcgaggctgcgcatgggggtaacgtgctgattacggacacctggatctccatggggcaggaggaagagaagaagaagagactgcaggcattccaggggtaccaggtcaccatgaaaaccgcaaaagtggcagcttcggactggactttcctgcattgcctgccgaggaagccggaggaagtcgacgacgaagtgttctactcgcctcggtccctggtgttccccgaggccgaaaaccggaagtggaccatcatggccgtgatggtgtccttgctgactgactatagcccgcagctgcagaagcctaagttctag

SEQ ID NO: 144 - DNA, 1065 bp, synthetic construct
  source 1..1065: mol_type = other DNA
atgcttttcaacctgagaatcctcttgaacaatgctgcttttcggaatggccacaactttatggttcggaacttccgttgcggccagcctttacaaaacaaggtccagctgaagggccgggatttgctcacactaaagaactttactggagaagagatcaagtacatgctatggctgtcggccgacctgaagttccgtatcaagcagaagggagaataccttccgctgcttcaaggaaagagcctcggcatgatctttgagaagcgctcaaccaggacccgcctttctactgaaactgggttcgcgctgctcggtggccacccctgcttcctgacgacccaggacatccacctcggagtgaacgaatccctcaccgataccgcccgggtgttatcgagcatggcagatgccgtgctggccagggtgtacaaacagtccgatctcgataccttggcaaaggaggcttccattcccatcatcaacggcctgagcgacctgtaccacccaatccaaatcctggctgactacctgaccctgcaagagcactacagcagcctgaagggtctgaccctgtcatggattggcgatggaaacaatattctgcactccatcatgatgtccgccgcgaagttcggaatgcatctgcaagccgccactccaaaaggatacgaaccggatgcgtccgtgaccaagttggcggaacagtacgcgaaggagaacggaaccaagcttctgctgactaacgaccccctcgaggctgcgcatgggggcaacgtgctgattaccgacacctggatctccatggggcaggaggaagagaagaagaagagactgcaggcattccaggggtaccaggtcaccatgaaaaccgcaaaagtggcagcttcggactggactttcctgcattgcctgccgaggaagccggaggaagtcgacgacgaagtgttctactcgcctcggtccctggtgttccccgaggccgaaaaccggaagtggaccatcatggccgtgatggtgtccttgctgactgactatagcccgcagctgcagaagcctaagttctag

SEQ ID NO: 145 - DNA, 1065 bp, synthetic construct
  source 1..1065: mol_type = other DNA
atgctgttcaacctgcgaatcctgctgaacaacgccgcttttcggaacgggcacaactttatggtgaggaactttcgctgcggacagcccctccagaataaggtccagctgaagggcagggacctgctgaccctgaaaaatttcacaggggaggaaatcaagtatatgctgtggctgtcagctgatctgaagttccggatcaagcagaagggcgaatatctgcctctgctccagggcaaaagcctggggatgatcttcgaaaagcgcagtactcggaccagactgtcaaccgagactggattcgctctgctgggaggacacccttgttttctgaccactcaggacattcacctgggagtgaacgagtccctgaccgacactgctcgcgtcctgagctctatggccgacgctgtgctggctcgagtctacaaacagtccgacctggataccctggccaaggaagcttctatcccaattattaacggcctgtcagacctgtatcaccccatccagattctggccgattacctgaccctccaggagcactattctagtctgaaagggctgacactgagttggattggggacggaaacaatatcctgcactctattatgatgtcagccgccaagtttggaatgcacctccaggctgcaaccccaaaaggctacgaacccgatgcctcagtgacaaagctggctgaacagtacgccaaagagaacggcactaagctgctgctgaccaacgaccctctggaggccgctcacggaggcaacgtgctgatcaccgatacctggattagtatgggacaggaggaagagaagaagaagcggctccaggccttccagggctaccaggtgacaatgaaaaccgctaaggtcgcagccagcgattggacctttctgcactgcctgcccagaaagcccgaagaggtggacgacgaggtcttctactctcccagaagcctggtgtttcccgaagctgagaataggaagtggacaattatggcagtgatggtcagcctgctgactgattattcacctcagctccagaaaccaaagttctga

SEQ ID NO: 146 - DNA, 1065 bp, synthetic construct
  source 1..1065: mol_type = other DNA
atgctgttcaacctgcgcatcctgctgaacaacgccgccttccgcaacggccacaacttcatggtgcgcaacttccgctgcggccagcccctgcagaacaaggtgcagctgaagggccgcgacctgctgaccctgaagaacttcaccggcgaggagatcaagtacatgctgtggctgagcgccgacctgaagttccgcatcaagcagaagggcgagtacctgcccctgctgcagggcaagagcctgggcatgatcttcgagaagcgcagcacccgcacccgcctgagcaccgagacaggcctggccctgctgggcggccacccctgcttcctgaccacccaggacatccacctgggcgtgaacgagagcctgaccgacaccgcccgcgtgctgagcagcatggccgacgccgtgctggcccgcgtgtacaagcagagcgacctggacaccctggccaaggaggccagcatccccatcatcaacggcctgagcgacctgtaccaccccatccagatcctggccgactacctgaccctgcaggagcactacagcagcctgaagggcctgaccctgagctggatcggcgacggcaacaacatcctgcacagcatcatgatgagcgccgccaagttcggcatgcacctgcaggccgccacccccaagggctacgagcccgacgccagcgtgaccaagctggccgagcagtacgccaaggagaacggcaccaagctgctgctgaccaacgaccccctggaggccgcccacggcggcaacgtgctgatcaccgacacctggatcagcatgggccaggaggaggagaagaagaagcgcctgcaggccttccagggctaccaggtgaccatgaagaccgccaaggtggccgccagcgactggaccttcctgcactgcctgccccgcaagcccgaggaggtggacgacgaggtgttctacagcccccgcagcctggtgttccccgaggccgagaaccgcaagtggaccatcatggccgtgatggtgagcctgctgaccgactacagcccccagctgcagaagcccaagttctga

SEQ ID NO: 147 - DNA, 1065 bp, synthetic construct
  source 1..1065: mol_type = other DNA
atgctgttcaacctgcgaatcctgctgaacaacgccgcttttcggaacgggcacaactttatggtgaggaactttcgctgcggacagcccctccagaataaggtccagctgaagggcagggacctgctgaccctgaaaaatttcacaggggaggaaatcaagtatatgctgtggctgtcagctgatctgaagttccggatcaagcagaagggcgaatatctgcctctgctccagggcaaaagcctggggatgatcttcgaaaagcgcagtactcggaccagactgtcaaccgagactggattcgctctgctgggaggacacccttgttttctgaccactcaggacattcacctgggagtgaacgagtccctgaccgacactgctcgcgtcctgagctctatggccgacgctgtgctagctcgagtctacaaacagtccgacctggataccctggccaaggaagcttctatcccaattattaacggcctgtcagacctgtatcaccccatccagattctggccgattacctgaccctccaggagcactattctagtctgaaagggctgacactgagttggattggggacggaaacaatatcctgcactctattatgatgtcagccgccaagtttggaatgcacctccaggctgcaaccccaaaaggctacgaacccgatgcctcagtgacaaagctggctgaacagtacgccaaagagaacggcactaagctgctgctgaccaacgaccctctggaggccgctcacggaggcaacgtgctgatcaccgatacctggattagtatgggacaggaggaagagaagaagaagcggctccaggccttccagggctaccaggtgacaatgaaaaccgctaaggtcgcagccagcgattggacctttctgcactgcctgcccagaaagcccgaagaggtggacgacgaggtcttctactctcccagaagcctggtgtttcccgaagctgagaataggaagtggacaattatggcagtgatggtcagcctgctgactgattattcacctcagctccagaaaccaaagttctga

SEQ ID NO: 148 - DNA, 1065 bp, synthetic construct
  source 1..1065: mol_type = other DNA
atgctgttcaacctgcgaatcctgctgaacaatgccgcttttcggaacgggcacaatttcatggtgaggaactttcgctgcggacagcccctccagaacaaggtccagctgaagggcagggacctgctgaccctgaaaaatttcacaggggaggaaatcaagtacatgctgtggctgtcagccgatctgaagttccggatcaagcagaagggcgaatatctgcctctgctccagggcaaaagcctggggatgatcttcgaaaagcgcagtactcggaccagactgtcaacagagactggattcgcactgctgggaggacacccatgttttctgaccacacaggacattcatctgggagtgaacgagtccctgaccgacacagcacgcgtcctgagctccatggctgatgcagtgctggctcgagtctacaaacagtctgacctggataccctggccaaggaagcttctatcccaatcattaatggcctgagtgacctgtatcaccccatccagattctggccgattacctgaccctccaggagcattattctagtctgaaagggctgacactgagctggattggggacggaaacaatatcctgcactccattatgatgagcgccgccaagtttggaatgcacctccaggctgcaaccccaaaaggctacgaacccgatgcctccgtgacaaagctggcagaacagtatgccaaagagaacggcactaagctgctgctgaccaatgaccctctggaggccgctcacggaggcaacgtgctgatcactgatacctggattagtatgggacaggaggaagagaagaagaagcggctccaggccttccagggctaccaggtgacaatgaaaactgctaaggtcgcagccagcgactggacctttctgcattgcctgcccagaaagcctgaagaggtggacgatgaggtcttctactcacccagaagcctggtgtttcctgaagctgagaataggaagtggacaatcatggcagtgatggtcagcctgctgactgattattcccctcagctccagaaaccaaagttctga

SEQ ID NO: 149 - DNA, 1065 bp, synthetic construct
  source 1..1065: mol_type = other DNA
atgcttttcaaccttcgcattctcctcaacaacgccgcgtttagaaacggacacaacttcatggtccgcaacttccgctgcggacagccgctgcagaacaaggtccagctcaagggtcgggatctcctgacgctgaagaactttaccggcgaagagattaagtacatgctgtggctgtccgccgaccttaagttccggatcaagcagaagggcgaataccttcccctgctgcaaggaaagtccctgggcatgatcttcgagaagcgcagtaccagaaccagactctccactgaaaccgggttcgcgctgcttggcggccacccgtgtttcctcactacgcaagacatccatcttggcgtgaacgagtcccttaccgacaccgccagggtgctgtcaagcatggccgacgccgtccttgcgcgcgtgtacaagcagtcagaccttgatactctggccaaggaagcctccatccctattatcaacggcctatccgacctttaccacccgatccagatcctcgctgactacctgaccctgcaagaacactacagcagcctcaagggactgactctgtcctggatcggcgacgggaacaacatcctgcactcaatcatgatgagcgcagccaagttcggcatgcatctccaagccgctacacccaagggttatgaaccggacgcctctgtgaccaagttggcagaacagtacgccaaggagaacggtactaagctccttttaaccaacgaccccctcgaagcagcccatggcgggaatgtgctcattaccgatacctggatttcgatgggccaggaggaggagaagaagaagcggctgcaggcgttccagggctaccaggtcaccatgaaaactgccaaagtggccgcctcggattggacctttctccactgcctgcctcggaagcctgaggaggtggacgacgaagtgttctactccccacggtccctcgtgttccccgaggccgaaaataggaagtggaccatcatggccgtgatggtgtccctcttgaccgattacagcccgcagcttcagaagcctaaattctag

SEQ ID NO: 150 - DNA, 1065 bp, synthetic construct
  source 1..1065: mol_type = other DNA
atgcttttcaatcttcgcatcctgttgaacaacgccgccttccgcaatggtcacaacttcatggtccggaacttcagatgtggacagcctctccaaaacaaggtccagctgaagggaagggacctcttaaccctcaaaaactttactggagaggagatcaagtacatgctgtggcttagcgccgaccttaagttccggatcaagcagaagggagagtacctcccgctgctgcaaggaaagagtcttggaatgatcttcgagaagcggtccaccagaactcgcctctccactgaaaccggattcgcactcctgggtggacacccgtgctttctgaccacccaagacatccacctcggagtgaacgagagcctcacggacaccgcgagagtgctgtcatccatggccgacgccgtgcttgcacgggtctacaagcagtccgatctggacactcttgccaaggaagcctccattcctatcattaacggtctgtcggatctgtaccacccgattcagatccttgcggactacctcacacttcaagaacactattcaagcctaaagggtctgaccctgtcctggatcggagatggaaacaacattctccattccatcatgatgagcgctgccaagttcggaatgcatctccaagcagcgactcctaagggttacgagccggacgcctcagtgactaagctggccgagcagtacgccaaggagaacggtaccaaactgttgcttactaacgacccgcttgaagcggcccatggaggaaacgtgctgattaccgacacctggatttcgatgggacaggaagaggagaagaagaagcggctccaggcgttccagggataccaggtcaccatgaaaacggccaaagtggccgctagcgattggacctttctgcactgcctcccgcgcaagcctgaagaagtggacgacgaagtgttctactcccctcgctctcttgtgttcccggaagccgaaaacaggaagtggaccatcatggccgtgatggtgtccctcctgaccgattacagcccgcagctgcagaagcctaagttctag

SEQ ID NO: 151 - DNA, 1065 bp, synthetic construct
  source 1..1065: mol_type = other DNA
atgcttttcaatctccgcatcctcctcaacaacgccgcgtttagaaacggccacaacttcatggtccggaacttcagatgtggccagccgcttcagaacaaggtccagctcaagggccgggatcttctgaccctgaagaactttactggcgaagaaatcaagtacatgctctggctctccgccgacttgaagttccgcattaagcagaagggggaataccttccgctgctgcaaggaaagtcgctcggcatgatctttgagaagcgctcaacccgcaccaggctgtccactgaaaccgggttcgcgctgcttggtggccacccctgcttcctgaccacccaagacattcacctcggagtgaacgaatcgctcactgatactgcccgggtgctgtcgtcgatggccgatgcagtgctggccagggtgtacaaacagtccgatctggacactctggccaaggaggcgtccatccctattatcaacggcctttccgacctctaccacccgattcagatccttgccgattacctcaccctgcaagaacactactcgtcactgaagggtctgaccttgtcctggatcggcgacggcaacaacatcctccattccattatgatgtccgccgccaaattcggcatgcatcttcaagccgcaacccctaagggttacgagccggacgcttccgtgaccaagctcgccgagcagtacgctaaggagaacggaaccaagcttctgctgactaacgaccccctagaggcagcccacgggggcaacgtgcttattactgacacctggatctccatgggacaggaagaagagaagaagaagcggttacaggcgttccagggctatcaggtcaccatgaaaaccgccaaggtcgctgcctcggactggaccttcctgcattgcctgcctcgcaagcccgaagaagtggacgacgaggtgttctactcgccacggtcccttgtgttccctgaggccgagaatagaaagtggaccattatggccgtgatggtgtcccttctcaccgactactcgccgcaactgcagaaacccaagttctag

SEQ ID NO: 152 - DNA, 1065 bp, synthetic construct
  source 1..1065: mol_type = other DNA
atgcttttcaatcttcgcatcctcctcaacaacgccgccttccggaacggtcacaacttcatggtccggaacttccgctgcggccagccgctccaaaacaaagtgcagcttaagggccgcgatctcctgaccctgaagaacttcaccggagaggaaatcaagtacatgctgtggctctcggcggacctgaagtttaggattaagcagaagggggagtatctgccgctgctccaagggaagtcccttggcatgatcttcgaaaagaggtccacccggactcggctcagcaccgaaacaggttttgcacttctggggggccacccgtgcttcctgacgacccaggacatccatctgggtgtcaacgagagtttgaccgacactgccagagtgctgtcatccatggcggacgcggtgctcgcgagagtgtacaagcagtccgatcttgacaccctggcaaaagaggcttcaatcccgatcattaacggactctcggatctgtaccaccctatccaaatcttggccgactacctgaccctgcaagaacactacagctccctgaagggcctgactctttcctggattggcgatggaaacaacattctccattctattatgatgtccgccgccaagttcggcatgcaccttcaagccgccaccccgaagggctacgaacctgacgcctccgtgactaagctagccgaacagtacgctaaggagaacggcactaagcttctccttaccaacgatccgctggaggcggcccatggcggaaatgtgcttatcaccgacacctggattagcatggggcaggaagaagagaagaagaaacggctccaggcattccagggctaccaggtcaccatgaaaactgccaaggtcgccgctagcgactggaccttcctccactgtctgcctcgcaagcctgaagaagtggacgacgaggtgttctactccccgcgctccctcgtgtttcctgaggccgagaacagaaagtggaccatcatggccgtgatggtgtcattacttacggactacagcccgcagctgcagaagccgaagttctag

SEQ ID NO: 153 - DNA, 1065 bp, synthetic construct
  source 1..1065: mol_type = other DNA
atgctttttaacttgagaatccttctgaacaacgccgctttccgcaacggtcataacttcatggtccggaacttcagatgtggccagcccctccaaaacaaagtgcagctgaagggccgggaccttcttacgctgaagaatttcaccggcgaagaaatcaagtacatgctctggctgtccgccgatcttaagttccgcattaagcagaagggggaatacctcccgctgctgcaagggaagtcgctgggcatgatttttgagaagcggtcaactcgcacccgcctgtccactgaaactggattcgcactgctcggtggccatccctgcttcctgaccacccaagacatccacctcggcgtgaacgagtccctgactgacaccgcccgggtcttatcctcgatggccgatgctgtgcttgcgagggtgtacaagcagtccgacctcgacacactcgcgaaggaggcctccatccccatcatcaacggcctgtccgacctttaccacccaattcagatcctcgccgattacctgaccctgcaagagcactactcgtcgctcaaggggcttaccctctcgtggattggcgacggcaacaacatccttcactccatcatgatgtcggcagcgaagttcggcatgcatctgcaagccgccacgcctaagggttatgaaccggatgcctcagtgaccaagctcgccgaacagtacgcgaaagagaatggaaccaagctacttctgaccaacgaccccctggaggccgctcacggcggcaacgtcctcattaccgatacttggatttcgatgggacaggaagaggaaaagaagaagagactgcaggcgttccagggataccaggtcaccatgaaaactgccaaagtggcagcctccgactggaccttccttcactgcctgccgaggaagcctgaagaggtggacgacgaggtgttctactccccgcgctccttggtgtttcctgaggccgaaaaccggaagtggactatcatggccgtgatggtgtccctcctcaccgactactcgccgcaactgcagaagcctaagttctag

SEQ ID NO: 154 - DNA, 1065 bp, synthetic construct
  source 1..1065: mol_type = other DNA
atgttattcaaccttagaattctccttaacaacgccgccttccggaatgggcataactttatggtccgcaatttccgctgtggacagcctctgcaaaacaaggtccagctcaagggccgggatctgctgactctcaagaacttcactggggaagaaatcaagtacatgctctggctgagcgccgacctcaagttccgcatcaagcagaagggagagtacctcccgctgctccaagggaagtccctgggcatgatcttcgagaagagatccacccgcaccagactttccactgagactggcttcgccttgctgggaggccacccatgcttcctgacgacccaggacattcaccttggcgtgaacgagtccctgactgacaccgcaagggtgttgtcctcgatggccgacgccgtgcttgcccgggtgtacaagcagagcgatcttgacaccctggctaaggaagcttccattcccatcatcaacggtctgagcgacctgtaccacccgattcagatcctggcggactacctaaccctgcaagagcactatagctccctgaagggcctcacactttcatggatcggcgacggcaacaacatcctgcactctattatgatgagcgctgccaaattcggcatgcacctccaagccgccacgcctaaaggctacgagcccgacgcctcggtgaccaagcttgcggagcagtacgcgaaggaaaacggcaccaagctgcttctcaccaacgatcctctggaagcggcccatggtggcaacgtgctcattaccgacacttggatctccatgggacaggaggaggaaaagaagaagcggctccaggcgtttcagggttaccaggtcaccatgaaaaccgccaaggtcgcagcctccgactggaccttccttcattgccttccgcgcaagcccgaagaagtggacgatgaagtgttttactcacctcggtcactcgtgttcccggaagcagagaacaggaaatggaccattatggccgtgatggtgtccctgctcaccgattacagtccgcaactgcagaagcccaagttctag

SEQ ID NO: 155 - DNA, 1065 bp, synthetic construct
  source 1..1065: mol_type = other DNA
atgcttttcaatctccgcatcctccttaacaacgccgcgtttagaaacggccacaacttcatggtccggaacttcagatgtggccagccgcttcaaaacaaggtccagctgaagggccgggatcttctgaccctgaagaactttactggcgaagagatcaagtacatgctctggctctccgcggacttgaagttccgcattaagcagaagggggaataccttccgctgcttcaaggaaagagcctcggcatgatctttgagaagcgctcaaccaggacccgcctttctactgaaactgggttcgcgctgctcggtggccacccctgcttcctgacgacccaggacatccacctcggagtgaacgaatccctcaccgataccgcccgggtgttatcgagcatggcagatgccgtgctggccagggtgtacaaacagtccgatctggacactctggccaaggaggcgtcaattcctattatcaacggccttagtgacctctaccatccgattcaaatcctggccgattacctcaccctgcaagaacactacagctccctgaagggtctgacattgtcctggatcggcgacggcaacaacattctccattccatcatgatgtccgccgcaaaattcggcatgcatcttcaagccgccacgcctaagggttacgaacccgacgcttccgtgactaagctcgccgagcagtacgctaaggagaacggaaccaagctgctgctgactaacgacccgctagaagcagcccacgggggcaacgtgcttattactgacacctggatctccatgggccaggaggaagagaaaaagaagcggctgcaggcgttccagggatatcaggtcaccatgaaaaccgccaaggtcgctgcctccgactggaccttcctgcactgcctgcctcgcaagcctgaagaagtggacgacgaggtgttctactcgccacggagcctcgtgttccccgaggccgagaatagaaagtggaccatcatggccgtgatggtgtcacttctcaccgactacagcccgcagcttcagaagcccaagttctag

SEQ ID NO: 156 - DNA, 1065 bp, synthetic construct
  source 1..1065: mol_type = other DNA
atgcttttcaatctccgcatcctccttaacaacgccgcgtttagaaacggccacaacttcatggtccggaacttcagatgtggccagccgcttcaaaacaaggtccagcttaagggccgggatctcctcacccttaaaaacttcaccggcgaagagatcaagtacatgctctggctctccgcggaccttaagttccgcattaagcagaagggggaataccttccgctgcttcaaggaaagagcctcggcatgatctttgagaagcgctcaaccaggaccaggctttctactgaaactgggttcgcgcttctcggcggtcatccctgcttcctcacgacccaagacatccacctcggagtgaacgaatccctcacggatactgcccgcgtgctttcgagcatggcagacgccgtgctcgcccgggtgtacaaacagtccgatctcgacactctcgccaaggaggcgtcaattcctattatcaacggtcttagtgacctttaccacccgatccagatcctcgccgattacctcacactccaagaacactacagctcccttaagggtcttaccctctcctggatcggcgacggcaacaacattctccactccatcatgatgtccgccgcaaagttcggcatgcatcttcaagccgccaccccgaagggctacgagcctgatgcttccgtgactaagctcgccgagcagtacgctaaggagaacggaaccaagcttcttctcactaacgacccactcgaagcagcccatgggggcaacgtgcttatcactgacacctggatctccatgggccaggaagaagagaagaagaagcggctccaggcgttccagggatatcaggtcaccatgaaaaccgccaaggtcgctgcctccgactggacctttctccactgcctccctcgcaaacctgaagaagtggacgacgaggtgttctactcgccccggagcctcgtgttccccgaggccgagaatagaaagtggaccattatggccgtgatggtgtcactcctcaccgactacagcccgcagcttcagaagcccaagttctag

SEQ ID NO: 157 - DNA, 1065 bp, synthetic construct
  source 1..1065: mol_type = other DNA
atgcttttcaatctccgcatcctccttaacaacgccgcgtttagaaacggacataacttcatggtccggaacttcagatgtggacagccgcttcaaaacaaggtccagctgaagggtcgggatcttctgaccctgaagaactttaccggagaagagatcaagtacatgctctggctctccgcggacttgaagttccgcattaagcagaagggagaatacctcccgctgcttcaaggaaagagcctcggaatgatttttgagaagcgctcaaccaggacccgcctttctactgaaactggattcgcgctgctgggtggacacccctgcttcctgacgacccaggacatccacctcggagtgaacgaatccctcactgataccgcccgggtgttatcgagcatggcagatgccgtgctggccagggtgtacaaacagtccgatctggacactctggccaaggaggcgtcaattcctatcatcaacggacttagtgacctctaccatccgattcaaatcctggccgactacctcaccctgcaagaacactacagctccctgaagggtctgacattgtcctggatcggagatggaaacaacattctccactccatcatgatgtccgccgcaaaattcggaatgcatcttcaagccgccacgcctaagggttacgaacccgacgcttccgtgactaagctcgccgagcagtacgctaaggagaacggtaccaagcttctcctgaccaacgacccactagaagcagcccacggtggaaacgtgcttattactgacacttggatctccatgggacaggaggaagagaaaaagaagcggctgcaggcgttccagggatatcaggtcaccatgaaaaccgccaaggtcgctgcctccgactggaccttcctgcactgcctgcctcgcaagcctgaagaagtggacgacgaggtgttctactcgccgcggagcctcgtgttccccgaggccgagaatagaaagtggaccatcatggccgtgatggtgtcactgctcaccgactacagcccgcagcttcagaagcccaagttctag

SEQ ID NO: 158 - DNA, 1065 bp, synthetic construct
  source 1..1065: mol_type = other DNA
atgcttttcaacctccgcattctcctcaacaacgctgccttccggaatggacataacttcatggtccggaacttcagatgcggacagccgcttcagaacaaggtccagcttaaggggagagatctccttaccctcaaaaacttcactggcgaagaaatcaagtacatgctctggcttagtgcggatctcaagttccgcatcaagcagaagggagaatacctcccgctccttcaaggaaagagcctcggcatgatttttgagaagaggtccaccagaactcgcctttcaaccgagactgggttcgccctgcttggcggtcacccctgcttcctcactacccaagacatccacctcggcgtgaacgagagccttaccgacaccgcccgcgtgctctcctcaatggccgacgctgtgctcgcccgggtgtacaagcagtccgaccttgatactctcgccaaggaggcctccatcccaattatcaacgggctctctgatctctaccaccctatccaaatcctcgcggactacctcaccctccaagagcactatagctcgctcaagggcctcaccctttcctggattggcgacggcaacaacattcttcactcgatcatgatgtccgccgccaagttcggcatgcatctccaagccgcgacccccaagggctacgagcctgacgcatccgtgaccaagctcgccgagcagtacgcgaaggaaaatggcaccaagcttcttctcaccaacgacccccttgaggccgctcatggcggcaacgtgctcatcactgacacttggatcagcatgggccaggaggaggaaaagaagaagcgccttcaggcattccagggttaccaggtcaccatgaaaaccgccaaagtggccgcctccgactggacctttcttcactgtctcccgcggaagcctgaagaagtggatgacgaagtgttttactcccctcggtcactcgtgttcccggaagcagaaaacaggaagtggaccattatggcggtcatggtgtccctcctcaccgactacagcccgcagcttcagaaacccaagttctag

SEQ ID NO: 159 - DNA, 1065 bp, synthetic construct
  source 1..1065: mol_type = other DNA
atgcttttcaatctccgcatcctccttaacaacgcagcgtttagaaacggtcacaacttcatggtccggaacttccgctgtggacagccgcttcaaaacaaggtccagctgaagggtcgggaccttctgaccctgaagaactttactggagaagagatcaagtacatgctttggctgtccgcggacttgaagttccgcattaagcagaagggagaataccttccgctgctccaaggaaagagcctgggaatgatctttgagaagcgctcaaccaggacccgcctttctactgaaactggattcgcgctgctgggtggtcacccttgcttcctgacgacccaggacattcacctcggagtgaacgagtccctcactgataccgccagagtgttatcgagcatggcagatgccgtgctggctagggtgtacaaacagtccgatctggacaccctggccaaggaggcatcaattcctattatcaacggacttagtgacctctaccatccgattcaaatcctggccgattacctcaccctgcaagaacactacagctccctgaagggtctgacattgtcctggatcggagatggaaacaacattctccattccatcatgatgtccgcggccaagttcggaatgcatctccaagccgccacgccgaaaggatacgagccggacgcttccgtgactaagctcgccgagcagtacgctaaggagaacggaaccaagcttctgctgactaacgacccgctagaagccgcccacggtggaaacgtgcttattactgacacctggatctccatgggacaggaagaagagaaaaagaagcggctgcaggcgttccagggatatcaggtcaccatgaaaaccgccaaggtcgccgcctccgactggaccttccttcactgcctgcctcggaagcctgaagaagtggacgacgaggtgttctactcgccgcggagcctcgtgttccctgaggccgagaatagaaagtggaccatcatggccgtgatggtgtcactcctcaccgactacagcccgcagcttcagaagcctaagttctag

SEQ ID NO: 160 - DNA, 1065 bp, synthetic construct
  source 1..1065: mol_type = other DNA
atgcttttcaatctccgcattctcctcaacaacgcagcctttagaaacggccacaacttcatggtccggaacttcagatgtggccagccgcttcagaacaaggtccagctcaagggccgggacctcctcaccctcaaaaactttaccggcgaagagatcaagtacatgctctggctttcggccgaccttaagttccgcatcaagcagaagggggaataccttccgctgcttcaaggaaagtccctcggcatgatctttgaaaagcgctcgaccaggacccgcctttccactgaaaccgggttcgcgcttctcggtggccacccctgcttcctcaccacccaagacattcacctcggagtgaacgaatcccttaccgataccgcaagagtgctttcgtcgatggccgatgccgtgcttgcgcgggtgtacaagcagtcagatctcgacactctcgccaaggaggcgtccattcctattatcaacggcctttccgacctttaccacccgattcagatcctcgccgattacctcaccctgcaagagcactactcgtcactcaagggtcttaccctctcctggatcggcgacggaaacaacatcctccattcgatcatgatgtccgccgccaaattcggcatgcacctccaagccgcgaccccgaagggttacgagcccgacgcttccgtgaccaagctcgccgaacagtacgctaaggaaaacggcaccaagctcctcctcactaacgaccctctcgaagcagcccatgggggcaacgtgctcattactgacacttggatctcgatgggccaggaagaggagaaaaagaagcggcttcaggcgttccagggatatcaggtcaccatgaaaaccgccaaggtcgctgcctcggactggaccttccttcactgccttccgcgcaagcctgaagaggtggacgatgaggtgttctactccccacggtcccttgtgttccccgaggccgagaataggaagtggaccatcatggccgtgatggtgtcgctcctcactgactactccccgcaacttcagaagcctaagttctag

SEQ ID NO: 161 - DNA, 1065 bp, synthetic construct
  source 1..1065: mol_type = other DNA
atgctgtttaatctgagaatacttctaaacaacgccgccttccggaatggccataactttatggttcggaatttccgctgcggccagccgctgcagaacaaggtccagctgaagggaagagacttgctgaccctcaagaacttcaccggagaagaaatcaagtatatgctgtggctgtccgccgacctgaaattccgcatcaagcagaagggcgaatatctgccgctgttgcaagggaagtccctggggatgatcttcgagaagaggtccaccagaacacggctttcaaccgaaaccgggtttgcactgctgggtggacacccctgttttctgaccactcaagatatccacctgggcgtgaacgagtcccttaccgacactgctagggtgttgtccagcatggccgatgccgtcctggctcgcgtgtacaagcagtccgacctggataccctggcaaaggaagcgtccattcccattatcaacgggctgtccgacctgtaccatccgattcaaatcctggcggactacctgactctgcaagagcattacagcagcttgaaggggcttactctctcgtggatcggcgacgggaacaacatcctgcactccatcatgatgtccgccgccaagttcgggatgcatttgcaagctgcgaccccgaaaggttacgagcccgatgctagcgtaactaagcttgccgaacagtacgccaaagagaatggtacaaaactgcttctgactaacgacccgctggaagcagcccacggcgggaacgtgctgataaccgacacctggatttcaatggggcaggaggaagagaagaagaagcgactgcaggcgttccaaggctatcaggttaccatgaaaaccgccaaagtggcagccagcgattggactttcctgcactgtctgccgcggaagcccgaggaagttgatgacgaagtattctactcaccccggagcctcgtgttccccgaggccgaaaaccggaagtggactattatggccgtgatggtgtcgctgttgaccgactacagcccgcaactgcagaagccgaagttttag

SEQ ID NO: 162 - DNA, 1065 bp, synthetic construct
  source 1..1065: mol_type = other DNA
atgcttttcaacctgaggatccttttgaacaacgccgcctttcgcaacggccacaactttatggtccgcaatttccgctgcgggcagccgctgcagaacaaggtccagctgaagggccgggatctgctgaccctgaagaacttcaccggggaggaaatcaagtacatgctttggctctccgccgatctgaagttcagaatcaagcagaagggagagtacctcccgttgctgcaaggaaagtcactcggaatgattttcgaaaagagaagcactaggacccgcctctcaactgaaaccgggttcgcgctgctcgggggccatccgtgtttcctgactacccaagacatccacctgggagtgaacgagtcgctgaccgacaccgcacgcgtgctgtcatccatggcggacgcagtgcttgcccgggtgtacaagcagtcggacctggacactcttgccaaggaggcatcaatccccatcattaacggactgtccgatctctaccacccgattcagatcctggctgactacctaaccctgcaagagcactactcaagcctgaaggggctgaccctgtcgtggatcggggacggcaacaacattctgcactccatcatgatgtcggcggctaagttcgggatgcatttgcaagcggcaactccgaagggttatgaacccgacgcctccgtgaccaagctggccgaacagtacgccaaggaaaacggaaccaagttgctgctgactaatgatcccctggaggcggcccacggggggaacgtgctgataaccgatacctggatctccatggggcaggaagaagagaagaaaaagcggctgcaggcattccagggataccaggtcaccatgaaaaccgcaaaagtggcagccagcgactggactttcctccattgcctgccgcgaaagccggaggaggtcgatgacgaggtgttctactccccgcggtcgctggtgttcccggaggcggaaaaccggaagtggaccattatggccgtgatggtgtcactcctgactgactacagcccgcaactgcagaagccgaagttctag

SEQ ID NO: 163 - DNA, 1074 bp, synthetic construct
  source 1..1074: mol_type = other DNA
atgcttttcaatctccgcatcctccttaacaacgccgcgtttagaaacggccacaacttcatggtccggaacttcagatgtggccagccgcttcaaaacaaggtccagctgaagggccgggatcttctgaccctgaagaactttactggcgaagagatcaagtacatgctctggctctccgcggacttgaagttccgcattaagcagaagggggaataccttccgctgcttcaaggaaagagcctcggcatgatctttgagaagcgctcaaccaggacccgcctttctactgaaactgggttcgcgctgctcggtggccacccctgcttcctgacgacccaggacatccacctcggagtgaacgaatccctcaccgataccgcccgggtgttatcgagcatggcagatgccgtgctggccagggtgtacaaacagtccgatctggacactctggccaaggaggcgtcaattcctattatcaacggccttagtgacctctaccatccgattcagatcctggccgattacctcaccctgcaagaacactacagctccctgaagggtctgacattgtcctggatcggcgacggcaacaacattctccattccatcatgatgtccgccgcaaaattcggcatgcatcttcaagccgccacgccgaagggttacgagcccgacgcttccgtgactaagctcgccgagcagtacgctaaggagaacggaaccaagcttctgctgactaacgacccactagaagcagcccacgggggcaacgtgcttattactgacacctggatctccatgggccaggaagaagagaaaaagaagcggctgcaggcgttccagggatatcaggtcaccatgaaaaccgccaaggtcgctgcctccgactggaccttcctgcactgcctgcctcgcaagcctgaagaagtggacgacgaggtgttctactcgccacggagcctcgtgttccccgaggccgagaatagaaagtggaccatcatggccgtgatggtgtcactgctcaccgactacagcccgcagcttcagaagcccaagttctagataagtgaa

SEQ ID NO: 164 - DNA, 1073 bp, synthetic construct
  source 1..1073: mol_type = other DNA
atgctgttcaacctgcgcatcctgctgaacaacgccgccttccgcaacggccacaacttcatggtgcgcaacttccgctgcggccagcccctgcagaacaaggtgcagctgaagggccgcgacctgctgaccctgaagaacttcaccggcgaggagatcaagtacatgctgtggctgagcgccgacctgaagttccgcatcaagcagaagggcgagtacctgcccctgctgcagggcaagagcctgggcatgatcttcgagaagcgcagcacccgcacccgcctgagcaccgagacaggcctggccctgctgggcggccacccctgcttcctgaccacccaggacatccacctgggcgtgaacgagagcctgaccgacaccgcccgcgtgctgagcagcatggccgacgccgtgctggcccgcgtgtacaagcagagcgacctggacaccctggccaaggaggccagcatccccatcatcaacggcctgagcgacctgtaccaccccatccagatcctggccgactacctgaccctgcaggagcactacagcagcctgaagggcctgaccctgagctggatcggcgacggcaacaacatcctgcacagcatcatgatgagcgccgccaagttcggcatgcacctgcaggccgccacccccaagggctacgagcccgacgccagcgtgaccaagctggccgagcagtacgccaaggagaacggcaccaagctgctgctgaccaacgaccccctggaggccgcccacggcggcaacgtgctgatcaccgacacctggatcagcatgggccaggaggaggagaagaagaagcgcctgcaggccttccagggctaccaggtgaccatgaagaccgccaaggtggccgccagcgactggaccttcctgcactgcctgccccgcaagcccgaggaggtggacgacgaggtgttctacagcccccgcagcctggtgttccccgaggccgagaaccgcaagtggaccatcatggccgtgatggtgagcctgctgaccgactacagcccccagctgcagaagcccaagttctgaataagtga

SEQ ID NO: 165 - DNA, 1073 bp, synthetic construct; identical to SEQ ID NO: 164
  source 1..1073: mol_type = other DNA

SEQ ID NO: 166 - DNA, 1074 bp, synthetic construct; identical to SEQ ID NO: 163
  source 1..1074: mol_type = other DNA

SEQ ID NO: 167 - DNA, 1073 bp, synthetic construct
  source 1..1073: mol_type = other DNA
atgcttttcaacctgagaatcctcttgaacaatgctgcttttcggaatggccacaactttatggttcggaacttccgttgcggccagcctttacaaaacaaggtccagctgaagggccgggatttgctcacactaaagaactttactggagaagagatcaagtacatgctatggctgtcggccgacctgaagttccgtatcaagcagaagggagaataccttccgctgcttcaaggaaagagcctcggcatgatctttgagaagcgctcaaccaggacccgcctttctactgaaactgggttcgcgctgctcggtggccacccctgcttcctgacgacccaggacatccacctcggagtgaacgaatccctcaccgataccgcccgggtgttatcgagcatggcagatgccgtgctggccagggtgtacaaacagtccgatctcgataccttggcaaaggaggcttccattcccatcatcaacggcctgagcgacctgtaccacccaatccaaatcctggctgactacctgaccctgcaagagcactacagcagcctgaagggtctgaccctgtcatggattggcgatggaaacaatattctgcactccatcatgatgtccgccgcgaagttcggaatgcatctgcaagccgccactccaaaaggatacgaaccggatgcatccgtgaccaagttggcggaacagtacgcgaaggagaacggaaccaagctcctgctgactaacgacccgctcgaggctgcgcatgggggtaacgtgctgattacggacacctggatctccatggggcaggaggaagagaagaagaagagactgcaggcattccaggggtaccaggtcaccatgaaaaccgcaaaagtggcagcttcggactggactttcctgcattgcctgccgaggaagccggaggaagtcgacgacgaagtgttctactcgcctcggtccctggtgttccccgaggccgaaaaccggaagtggaccatcatggccgtgatggtgtccttgctgactgactatagcccgcagctgcagaagcctaagttctagataagtga

SEQ ID NO: 168 - DNA, 1073 bp, synthetic construct; identical to SEQ ID NO: 164
  source 1..1073: mol_type = other DNA

SEQ ID NO: 169 - DNA, 1074 bp, synthetic construct; identical to SEQ ID NO: 163
  source 1..1074: mol_type = other DNA

SEQ ID NO: 170 - DNA, 1073 bp, synthetic construct; identical to SEQ ID NO: 164
  source 1..1073: mol_type = other DNA

SEQ ID NO: 171 - DNA, 1073 bp, synthetic construct; identical to SEQ ID NO: 167
  source 1..1073: mol_type = other DNA

SEQ ID NO: 172 - DNA, 1074 bp, synthetic construct; identical to SEQ ID NO: 163
  source 1..1074: mol_type = other DNA

SEQ ID NO: 173 - DNA, 1073 bp, synthetic construct; identical to SEQ ID NO: 164
  source 1..1073: mol_type = other DNA

SEQ ID NO: 174 - DNA, 1073 bp, synthetic construct; identical to SEQ ID NO: 167
  source 1..1073: mol_type = other DNA

SEQ ID NO: 175 - DNA, 1065 bp, synthetic construct
  source 1..1065: mol_type = other DNA
atgctgttcaacctgcgcatcctgctgaacaacgccgccttccgcaacggccacaacttcatggtgcgcaacttccgctgcggccagcccctgcagaacaaggtgcagctgaagggccgcgacctgctgaccctgaagaacttcaccggcgaggagatcaagtacatgctgtggctgagcgccgacctgaagttccgcatcaagcagaagggcgagtacctgcccctgctgcagggcaagagcctgggcatgatcttcgagaagcgcagcacccgcacccgcctgagcaccgagacaggcttcgccctgctgggcggccacccctgcttcctgaccacccaggacatccacctgggcgtgaacgagagcctgaccgacaccgcccgcgtgctgagcagcatggccgacgccgtgctggcccgcgtgtacaagcagagcgacctggacaccctggccaaggaggccagcatccccatcatcaacggcctgagcgacctgtaccaccccatccagatcctggccgactacctgaccctgcaggagcactacagcagcctgaagggcctgaccctgagctggatcggcgacggcaacaacatcctgcacagcatcatgatgagcgccgccaagttcggcatgcacctgcaggccgccacccccaagggctacgagcccgacgccagcgtgaccaagctggccgagcagtacgccaaggagaacggcaccaagctgctgctgaccaacgaccccctggaggccgcccacggcggcaacgtgctgatcaccgacacctggatcagcatgggccaggaggaggagaagaagaagcgcctgcaggccttccagggctaccaggtgaccatgaagaccgccaaggtggccgccagcgactggaccttcctgcactgcctgccccgcaagcccgaggaggtggacgacgaggtgttctacagcccccgcagcctggtgttccccgaggccgagaaccgcaagtggaccatcatggccgtgatggtgagcctgctgaccgactacagcccccagctgcagaagcccaagttctga

SEQ ID NO: 176 - DNA, 1065 bp, synthetic construct; identical to SEQ ID NO: 175
  source 1..1065: mol_type = other DNA

SEQ ID NO: 177 - DNA, 1065 bp, synthetic construct; identical to SEQ ID NO: 175
  source 1..1065: mol_type = other DNA

SEQ ID NO: 178 - DNA, 1074 bp, synthetic construct
  source 1..1074: mol_type = other DNA
atgctgttcaacctgcgcatcctgctgaacaacgccgccttccgcaacggccacaacttcatggtgcgcaacttccgctgcggccagcccctgcagaacaaggtgcagctgaagggccgcgacctgctgaccctgaagaacttcaccggcgaggagatcaagtacatgctgtggctgagcgccgacctgaagttccgcatcaagcagaagggcgagtacctgcccctgctgcagggcaagagcctgggcatgatcttcgagaagcgcagcacccgcacccgcctgagcaccgagacaggcttcgccctgctgggcggccacccctgcttcctgaccacccaggacatccacctgggcgtgaacgagagcctgaccgacaccgcccgcgtgctgagcagcatggccgacgccgtgctggcccgcgtgtacaagcagagcgacctggacaccctggccaaggaggccagcatccccatcatcaacggcctgagcgacctgtaccaccccatccagatcctggccgactacctgaccctgcaggagcactacagcagcctgaagggcctgaccctgagctggatcggcgacggcaacaacatcctgcacagcatcatgatgagcgccgccaagttcggcatgcacctgcaggccgccacccccaagggctacgagcccgacgccagcgtgaccaagctggccgagcagtacgccaaggagaacggcaccaagctgctgctgaccaacgaccccctggaggccgcccacggcggcaacgtgctgatcaccgacacctggatcagcatgggccaggaggaggagaagaagaagcgcctgcaggccttccagggctaccaggtgaccatgaagaccgccaaggtggccgccagcgactggaccttcctgcactgcctgccccgcaagcccgaggaggtggacgacgaggtgttctacagcccccgcagcctggtgttccccgaggccgagaaccgcaagtggaccatcatggccgtgatggtgagcctgctgaccgactacagcccccagctgcagaagcccaagttctgaataagtgaa

SEQ ID NO: 179 - DNA, 1077 bp, synthetic construct
  source 1..1077: mol_type = other DNA
atgggcgtcttcaacctgcggatcctgctgaacaacgccgccttccggaacggccacaacttcatggtccgcaacttcagatgcggccagcccctgcagaacaaggtgcagctgaagggccgggacctgctgaccctgaagaacttcaccggcgaagagatcaagtacatgctgtggctgagcgccgacctgaagttccggatcaagcagaagggcgagtacctgcccctgctgcaaggcaagagcctgggcatgatcttcgagaagcggagcacccggacccggctgagcaccgagacaggctttgccctgctgggaggccacccctgctttctgaccacccaggacatccacctgggcgtgaacgagagcctgaccgacaccgccagagtgctgagcagcatggccgacgccgtgctggcccgggtgtacaagcagagcgacctggacaccctggccaaagaggccagcatccccatcatcaacggcctgagcgacctgtaccaccccatccagatcctggccgactacctgaccctgcaggaacactacagctccctgaagggcctgaccctgagctggatcggcgacggcaacaacatcctgcacagcatcatgatgagcgccgccaagttcggcatgcatctgcaggccgccacccccaagggctacgagcctgatgccagcgtgaccaagctggccgagcagtacgccaaagagaacggcaccaagctgctgctgaccaacgaccccctggaagccgcccacggcggcaacgtgctgatcaccgacacctggatcagcatgggccaggaagaggaaaagaagaagcggctgcaggccttccagggctaccaggtcacaatgaagaccgccaaggtggccgccagcgactggaccttcctgcactgcctgccccggaagcccgaagaggtggacgacgaggtgttctacagcccccggtccctggtgttccccgaggccgagaaccggaagtggaccattatggccgtgatggtgtccctgctgaccgactactccccccagctgcagaagcccaagttctagataagtgaa

SEQ ID NO: 180 - DNA, 1077 bp, synthetic construct
  source 1..1077: mol_type = other DNA
atgggcgtcttcaacctgcggatcctgctgaacaacgccgccttccggaacggccacaacttcatggtccgcaacttcagatgcggccagcccctgcagaacagggtgcagctgaagggccgggacctgctgaccctgaagaacttcaccggcgaagagatcaggtacatgctgtggctgagcgccgacctgaagttccggatcaagcagaagggcgagtacctgcccctgctgcaaggcaagagcctgggcatgatcttcgagaagcggagcacccggacccggctgagcaccgagacaggctttgccctgctgggaggccacccctgctttctgaccacccaggacatccacctgggcgtgaacgagagcctgaccgacaccgccagagtgctgagcagcatggccgacgccgtgctggcccgggtgtacaagcagagcgacctggacaccctggccaaagaggccagcatccccatcatcaacggcctgagcgacctgtaccaccccatccagatcctggccgactacctgaccctgcaggaacactacagctccctgaagggcctgaccctgagctggatcggcgacggcaacaacatcctgcacagcatcatgatgagcgccgccaagttcggcatgcatctgcaggccgccacccccaagggctacgagcctgatgccagcgtgaccaagctggccgagcagtacgccaaagagaacggcaccaagctgctgctgaccaacgaccccctggaagccgcccacggcggcaacgtgctgatcaccgacacctggatcagcatgggccaggaagaggaaaagaagaagcggctgcaggccttccagggctaccaggtcacaatgaagaccgccaaggtggccgccagcgactggaccttcctgcactgcctgccccggaagcccgaagaggtggacgacgaggtgttctacagcccccggtccctggtgttccccgaggccgagaaccggaagtggaccattatggccgtgatggtgtccctgctgaccgactactccccccagctgcagaagcccaagttctagataagtgaa

SEQ ID NO: 181 - DNA, 1077 bp, synthetic construct
  source 1..1077: mol_type = other DNA
atgctggtcttcaacctgcggatcctgctgaacaacgccgccttccggaacggccacaacttcatggtccgcaacttcagatgcggccagcccctgcagaacagggtgcagctgaagggccgggacctgctgaccctgaagaacttcaccggcgaagagatcaggtacatgctgtggctgagcgccgacctgaagttccggatcaagcagaagggcgagtacctgcccctgctgcaaggcaagagcctgggcatgatcttcgagaagcggagcacccggacccggctgagcaccgagacaggctttgccctgctgggaggccacccctgctttctgaccacccaggacatccacctgggcgtgaacgagagcctgaccgacaccgccagagtgctgagcagcatggccgacgccgtgctggcccgggtgtacaagcagagcgacctggacaccctggccaaagaggccagcatccccatcatcaacggcctgagcgacctgtaccaccccatccagatcctggccgactacctgaccctgcaggaacactacagctccctgaagggcctgaccctgagctggatcggcgacggcaacaacatcctgcacagcatcatgatgagcgccgccaagttcggcatgcatctgcaggccgccacccccaagggctacgagcctgatgccagcgtgaccaagctggccgagcagtacgccaaagagaacggcaccaagctgctgctgaccaacgaccccctggaagccgcccacggcggcaacgtgctgatcaccgacacctggatcagcatgggccaggaagaggaaaagaagaagcggctgcaggccttccagggctaccaggtcacaatgaagaccgccaaggtggccgccagcgactggaccttcctgcactgcctgccccggaagcccgaagaggtggacgacgaggtgttctacagcccccggtccctggtgttccccgaggccgagaaccggaagtggaccattatggccgtgatggtgtccctgctgaccgactactccccccagctgcagaagcccaagttctagataagtgaa

SEQ ID NO: 182 - DNA, 1074 bp, synthetic construct
  source 1..1074: mol_type = other DNA
atgctgttcaacctgaggatcctgctgaacaacgcagctttcaggaacggccacaacttcatggtgaggaacttccggtgcggccagcccctgcagaacaaggtgcagctgaagggcagggacctgctgaccctgaagaacttcaccggagaggagatcaagtacatgctgtggctgagcgcagacctgaagttcaggatcaagcagaagggagagtacctgcccctgctgcaggggaagtccctgggcatgatcttcgagaagaggagtaccaggaccaggctgagcaccgaaaccggcttcgccctgctgggaggacacccctgcttcctgaccacccaggacatccacctgggcgtgaacgagagtctgaccgacaccgccagggtgctgtctagcatggccgacgccgtgctggccagggtgtacaagcagtcagacctggacaccctggctaaggaggccagcatccccatcatcaacggcctgagcgacctgtaccaccccatccagatcctggctgactacctgaccctgcaggagcactacagctctctgaagggcctgaccctgagctggatcggcgacgggaacaacatcctgcacagcatcatgatgagcgccgccaagttcggcatgcacctgcaggccgctacccccaagggttacgagcccgacgccagcgtgaccaagctggcagagcagtacgccaaggagaacggcaccaagctgctgctgaccaacgaccccctggaggccgcccacggaggcaacgtgctgatcaccgacacctggatcagcatgggacaggaggaggagaagaagaagcggctgcaggctttccagggttaccaggtgaccatgaagaccgccaaggtggctgccagcgactggaccttcctgcactgcctgcccaggaagcccgaggaggtggacgacgaggtgttctactctcccaggagcctggtgttccccgaggccgagaacaggaagtggaccatcatggctgtgatggtgtccctgctgaccgactacagcccccagctgcagaagcccaagttctgaataagtgaa

SEQ ID NO: 183 - DNA, 1074 bp, synthetic construct
  source 1..1074: mol_type = other DNA
atgctgttcaacctgaggatcctgctgaacaacgcagctttcaggaacggccacaacttcatggtgaggaacttccggtgcggccagcccctgcagaacaaggtgcagctgaagggcagggacctgctgaccctgaagaacttcaccggagaggagatcaagtacatgctgtggctgagcgcagacctgaagttcaggatcaagcagaagggagagtacctgcccctgctgcaggggaagtccctgggcatgatcttcgagaagaggagtaccaggaccaggctgagcaccgaaaccggcttcgccctgctgggaggacacccctgcttcctgacgacccaggacatccacctcggagtgaacgaatccctcaccgataccgcccgggtgttatcaagcatggcagatgccgtgctggccagggtgtacaaacagtccgatctggacactctggctaaggaggccagcatccccatcatcaacggcctgagcgacctgtaccaccccatccagatcctggctgactacctgaccctgcaggagcactacagctctctgaagggcctgaccctgagctggatcggcgacgggaacaacatcctgcactccatcatgatgtccgccgcgaagttcggaatgcatctgcaagccgccacgccaaaaggatacgaaccggatgcgcccgtgacaaagttggcggaacagtacgctaaggagaacggaaccaagctgctgctgaccaacgaccccctggaggccgcccacggaggcaacgtgctgatcaccgacacctggatcagcatgggacaggaggaggagaagaagaagcggctgcaggctttccagggttaccaggtgaccatgaagaccgccaaggtggctgccagcgactggaccttcctgcactgcctgcccaggaagcccgaggaggtggacgacgaggtgttctactctcccaggagcctggtgttccccgaggccgagaacaggaagtggaccatcatggctgtgatggtgtccctgctgaccgactacagcccccagctgcagaagcccaagttctgaataagtgaa

SEQ ID NO: 184 - DNA, 1074 bp, synthetic construct; identical to SEQ ID NO: 178
  source 1..1074: mol_type = other DNA

SEQ ID NO: 185 - DNA, 1074 bp, synthetic construct; identical to SEQ ID NO: 178
  source 1..1074: mol_type = other DNA

SEQ ID NO: 186 - DNA, 1065 bp, synthetic construct
  source 1..1065: mol_type = other DNA
atgcttttcaacttgagaatcctgctgaacaacgccgcctttcgcaacggtcacaattttatggtcagaaacttcagatgcggacagcccctccaaaacaaggtccagctgaagggccgcgatctcctcaccctgaagaacttcacgggggaggagatcaagtacatgctgtggctctccgctgacctgaagttcaggatcaagcagaagggagaatatctgccgctgctgcaagggaagtccctggggatgattttcgagaagcggagcacccggactcggctctccactgaaactggtttcgcccttctgggcggtcacccctgcttcctgaccactcaagacattcacctcggagtgaacgagtccttgactgacaccgcccgggtgctgtcgagcatggcagacgccgtgctagcccgcgtgtacaagcagtcagacctcgataccctggccaaggaggcttcgatcccgatcatcaacgggttgtccgacctgtaccacccgattcagattctcgccgactacctcaccctgcaagagcattacagctccctgaaggggcttaccctgtcctggattggcgacggaaacaacatcctgcactccattatgatgtcggcggccaagttcggcatgcacctccaagccgcgacccctaagggttacgaaccagacgcgtcagtgactaagctggccgaacagtacgcaaaggaaaatggcacgaagctgctcctgaccaacgatccgttggaagccgcccatggcggaaatgtgctcatcaccgacacctggatctcgatgggacaggaggaagagaagaagaagcggctgcaggcgttccagggctaccaggtcaccatgaaaactgccaaggtggccgccagcgactggaccttcctgcactgccttccgcgcaagcctgaggaggtggacgatgaagtgttctactctccacggtccctggtgttccccgaggcggagaaccgcaaatggaccatcatggctgtgatggtcagcctgctgaccgattacagccctcagttgcaaaagccgaagttttga

SEQ ID NO: 187 - DNA, 1065 bp, synthetic construct
  source 1..1065: mol_type = other DNA
atgctgttcaacctccgcatcctcctcaacaacgccgcattcagaaacgggcacaacttcatggtcagaaacttccgctgcgggcaacccctacaaaacaaggtccagctcaaggggcgggacctcctgaccctgaagaacttcaccggcgaagagatcaagtacatgctgtggctctccgccgacctgaagttccgcatcaagcagaagggagagtacctcccgctgctgcaagggaagtcgctggggatgatcttcgagaagcggtcaaccagaacccggctgtcaaccgaaaccgggttcgcactgctggggggacacccgtgcttcctgaccacccaagacatccacctgggagtgaacgaatcgctgaccgacaccgcccgcgtgctgagctcaatggcggacgccgtgctggcccgcgtgtacaagcagtccgacctggacaccctggccaaggaagcgtccatcccgatcatcaacggactgtccgacctgtaccacccgatccagatcctggcagactacctgaccctgcaagaacactacagctccctgaagggcctgaccctgtcatggatcggggacgggaacaacatcctgcactccataatgatgtcagccgccaagttcggaatgcacctccaagccgcaaccccgaagggctacgaaccggacgcatcagtgaccaaactggccgagcagtacgccaaggaaaacggcaccaagctcctgctgaccaacgacccgctggaggccgcacacggggggaacgtgctgatcaccgacacctggatctccatgggacaggaggaggaaaagaagaagcggctgcaggcgttccaggggtaccaggtcaccatgaaaaccgcgaaggtcgcggcatcagactggaccttcctgcactgcctgccccggaagccggaagaggtggacgacgaggtgttctactcgccgcgctcgctggtgttccccgaggcggagaacaggaagtggaccatcatggcggtgatggtcagcctcctgaccgactactcgccgcagctgcagaagccgaagttctga

SEQ ID NO: 188 - DNA, 1074 bp, synthetic construct
  source 1..1074: mol_type = other DNA
atgcttttcaatctccgcatcctccttaacaacgccgcgtttagaaacggccacaacttcatggtccggaacttcagatgtggccagccgcttcaaaacaaggtccagctgaagggccgggatcttctgaccctgaagaactttactggcgaagagatcaagtacatgctctggctctccgcggacttgaagttccgcattaagcagaagggggaataccttccgctgcttcaaggaaagagcctcggcatgatctttgagaagcgctcaaccaggacccgcctttctactgaaactgggttcgcgctgctcggtggccacccctgcttcctgacgacccaggacatccacctcggagtgaacgaatccctcaccgataccgcccgggtgttatcgagcatggcagatgccgtgctggccagggtgtacaaacagtccgatctggacactctggccaaggaggcgtcaattcctattatcaacggccttagtgacctctaccatccgattcagatcctggccgattacctcaccctgcaagaacactacagctccctgaagggtctgacattgtcctggatcggcgacggcaacaacattctccattccatcatgatgtccgccgcaaaattcggcatgcatcttcaagccgccacgccgaagggttacgagcccgacgcttccgtgactaagctcgccgagcagtacgctaaggagaacggaaccaagcttctgctgactaacgacccactagaagcagcccacgggggcaacgtgcttattactgacacctggatctccatgggccaggaagaagagaaaaagaagcggctgcaggcgttccagggatatcaggtcaccatgaaaaccgccaaggtcgctgcctccgactggaccttcctgcactgcctgcctcgcaagcctgaagaagtggacgacgaggtgttctactcgccacggagcctcgtgttccccgaggccgagaatagaaagtggaccatcatggccgtgatggtgtcactgctcaccgactacagcccgcagcttcagaagcccaagttctgaataagtaga

SEQ ID NO: 189 - DNA, 1074 bp, synthetic construct
  source 1..1074: mol_type = other DNA
atgcttttcaacctgagaatcctcttgaacaatgctgcttttcggaatggccacaactttatggttcggaacttccgttgcggccagcctttacaaaacaaggtccagctgaagggccgggatttgctcacactaaagaactttactggagaagagatcaagtacatgctatggctgtcggccgacctgaagttccgtatcaagcagaagggagaataccttccgctgcttcaaggaaagagcctcggcatgatctttgagaagcgctcaaccaggacccgcctttctactgaaactgggttcgcgctgctcggtggccacccctgcttcctgacgacccaggacatccacctcggagtgaacgaatccctcaccgataccgcccgggtgttatcgagcatggcagatgccgtgctggccagggtgtacaaacagtccgatctcgataccttggcaaaggaggcttccattcccatcatcaacggcctgagcgacctgtaccacccaatccaaatcctggctgactacctgaccctgcaagagcactacagcagcctgaagggtctgaccctgtcatggattggcgatggaaacaatattctgcactccatcatgatgtccgccgcgaagttcggaatgcatctgcaagccgccactccaaaaggatacgaaccggatgcatccgtgaccaagttggcggaacagtacgcgaaggagaacggaaccaagctcctgctgactaacgacccgctcgaggctgcgcatgggggtaacgtgctgattacggacacctggatctccatggggcaggaggaagagaagaagaagagactgcaggcattccaggggtaccaggtcaccatgaaaaccgcaaaagtggcagcttcggactggactttcctgcattgcctgccgaggaagccggaggaagtcgacgacgaagtgttctactcgcctcggtccctggtgttccccgaggccgaaaaccggaagtggaccatcatggccgtgatggtgtccttgctgactgactatagcccgcagctgcagaagcctaagttctgaataagtaga

SEQ ID NO: 190 - DNA, 1074 bp, synthetic construct
  source 1..1074: mol_type = other DNA
atgctgttcaacctgcgcatcctgctgaacaacgccgccttccgcaacggccacaacttcatggtgcgcaacttccgctgcggccagcccctgcagaacaaggtgcagctgaagggccgcgacctgctgaccctgaagaacttcaccggcgaggagatcaagtacatgctgtggctgagcgccgacctgaagttccgcatcaagcagaagggcgagtacctgcccctgctgcagggcaagagcctgggcatgatcttcgagaagcgcagcacccgcacccgcctgagcaccgagacaggcctggccctgctgggcggccacccctgcttcctgaccacccaggacatccacctgggcgtgaacgagagcctgaccgacaccgcccgcgtgctgagcagcatggccgacgccgtgctggcccgcgtgtacaagcagagcgacctggacaccctggccaaggaggccagcatccccatcatcaacggcctgagcgacctgtaccaccccatccagatcctggccgactacctgaccctgcaggagcactacagcagcctgaagggcctgaccctgagctggatcggcgacggcaacaacatcctgcacagcatcatgatgagcgccgccaagttcggcatgcacctgcaggccgccacccccaagggctacgagcccgacgccagcgtgaccaagctggccgagcagtacgccaaggagaacggcaccaagctgctgctgaccaacgaccccctggaggccgcccacggcggcaacgtgctgatcaccgacacctggatcagcatgggccaggaggaggagaagaagaagcgcctgcaggccttccagggctaccaggtgaccatgaagaccgccaaggtggccgccagcgactggaccttcctgcactgcctgccccgcaagcccgaggaggtggacgacgaggtgttctacagcccccgcagcctggtgttccccgaggccgagaaccgcaagtggaccatcatggccgtgatggtgagcctgctgaccgactacagcccccagctgcagaagcccaagttctgaataagtaga

SEQ ID NO: 191 - DNA, 1065 bp, synthetic construct; identical to SEQ ID NO: 136
  source 1..1065: mol_type = other DNA

SEQ ID NO: 192 - DNA, 1065 bp, synthetic construct; identical to SEQ ID NO: 136
  source 1..1065: mol_type = other DNA

SEQ ID NO: 193 - DNA, 1065 bp, synthetic construct; identical to SEQ ID NO: 136
  source 1..1065: mol_type = other DNA

SEQ ID NO: 194 - DNA, 1065 bp, synthetic construct; identical to SEQ ID NO: 136
  source 1..1065: mol_type = other DNA

SEQ ID NO: 195 - DNA, 1065 bp, synthetic construct; identical to SEQ ID NO: 136
  source 1..1065: mol_type = other DNA

SEQ ID NO: 196 - DNA, 1065 bp, synthetic construct
  source 1..1065: mol_type = other DNA
atggtgttcaacctccgcatcctcctcaacaacgccgcattcagaaacgggcacaacttcatggtcagaaacttccgctgcgggcaacccctacaaaacaaggtccagctcaaggggcgggacctcctgaccctgaagaacttcaccggcgaagagatcaagtacatgctgtggctctccgccgacctgaagttccgcatcaagcagaagggagagtacctcccgctgctgcaagggaagtcgctggggatgatcttcgagaagcggtcaaccagaacccggctgtcaaccgaaaccgggttcgcactgctggggggacacccgtgcttcctgaccacccaagacatccacctgggagtgaacgaatcgctgaccgacaccgcccgcgtgctgagctcaatggcggacgccgtgctggcccgcgtgtacaagcagtccgacctggacaccctggccaaggaagcgtccatcccgatcatcaacggactgtccgacctgtaccacccgatccagatcctggcagactacctgaccctgcaagaacactacagctccctgaagggcctgaccctgtcatggatcggggacgggaacaacatcctgcactccataatgatgtcagccgccaagttcggaatgcacctccaagccgcaaccccgaagggctacgaaccggacgcatcagtgaccaaactggccgagcagtacgccaaggaaaacggcaccaagctcctgctgaccaacgacccgctggaggccgcacacggggggaacgtgctgatcaccgacacctggatctccatgggacaggaggaggaaaagaagaagcggctgcaggcgttccaggggtaccaggtcaccatgaaaaccgcgaaggtcgcggcatcagactggaccttcctgcactgcctgccccggaagccggaagaggtggacgacgaggtgttctactcgccgcgctcgctggtgttccccgaggcggagaacaggaagtggaccatcatggcggtgatggtcagcctcctgaccgactactcgccgcagctgcagaagccgaagttctga

SEQ ID NO: 197 - DNA, 1065 bp, synthetic construct
  source 1..1065: mol_type = other DNA
atggtgttcaacctccgcatcctcctcaacaacgccgcattcagaaacgggcacaacttcatggtcagaaacttccgctgcgggcaacccctacaaaaccgggtccagctcaaggggcgggacctcctgaccctgaagaacttcaccggcgaagagatcaagtacatgctgtggctctccgccgacctgaagttccgcatcaagcagaagggagagtacctcccgctgctgcaagggaagtcgctggggatgatcttcgagaagcggtcaaccagaacccggctgtcaaccgaaaccgggttcgcactgctggggggacacccgtgcttcctgaccacccaagacatccacctgggagtgaacgaatcgctgaccgacaccgcccgcgtgctgagctcaatggcggacgccgtgctggcccgcgtgtacaagcagtccgacctggacaccctggccaaggaagcgtccatcccgatcatcaacggactgtccgacctgtaccacccgatccagatcctggcagactacctgaccctgcaagaacactacagctccctgaagggcctgaccctgtcatggatcggggacgggaacaacatcctgcactccataatgatgtcagccgccaagttcggaatgcacctccaagccgcaaccccgaagggctacgaaccggacgcatcagtgaccaaactggccgagcagtacgccaaggaaaacggcaccaagctcctgctgaccaacgacccgctggaggccgcacacggggggaacgtgctgatcaccgacacctggatctccatgggacaggaggaggaaaagaagaagcggctgcaggcgttccaggggtaccaggtcaccatgaaaaccgcgaaggtcgcggcatcagactggaccttcctgcactgcctgccccggaagccggaagaggtggacgacgaggtgttctactcgccgcgctcgctggtgttccccgaggcggagaacaggaagtggaccatcatggcggtgatggtcagcctcctgaccgactactcgccgcagctgcagaagccgaagttctga

SEQ ID NO: 198 - DNA, 1065 bp, synthetic construct
  source 1..1065: mol_type = other DNA
atggtgttcaacctccgcatcctcctcaacaacgccgcattcagaaacgggcacaacttcatggtcagaaacttccgctgcgggcaacccctacaaaaccgggtccagctcaaggggcgggacctcctgaccctgaagaacttcaccggcgaagagatccggtacatgctgtggctctccgccgacctgaagttccgcatcaagcagaagggagagtacctcccgctgctgcaagggaagtcgctggggatgatcttcgagaagcggtcaaccagaacccggctgtcaaccgaaaccgggttcgcactgctggggggacacccgtgcttcctgaccacccaagacatccacctgggagtgaacgaatcgctgaccgacaccgcccgcgtgctgagctcaatggcggacgccgtgctggcccgcgtgtacaagcagtccgacctggacaccctggccaaggaagcgtccatcccgatcatcaacggactgtccgacctgtaccacccgatccagatcctggcagactacctgaccctgcaagaacactacagctccctgaagggcctgaccctgtcatggatcggggacgggaacaacatcctgcactccataatgatgtcagccgccaagttcggaatgcacctccaagccgcaaccccgaagggctacgaaccggacgcatcagtgaccaaactggccgagcagtacgccaaggaaaacggcaccaagctcctgctgaccaacgacccgctggaggccgcacacggggggaacgtgctgatcaccgacacctggatctccatgggacaggaggaggaaaagaagaagcggctgcaggcgttccaggggtaccaggtcaccatgaaaaccgcgaaggtcgcggcatcagactggaccttcctgcactgcctgccccggaagccggaagaggtggacgacgaggtgttctactcgccgcgctcgctggtgttccccgaggcggagaacaggaagtggaccatcatggcggtgatggtcagcctcctgaccgactactcgccgcagctgcagaagccgaagttctga

SEQ ID NO: 199 - DNA, 1065 bp, synthetic construct
  source 1..1065: mol_type = other DNA
atgctggtcaacctccgcatcctcctcaacaacgccgcattcagaaacgggcacaacttcatggtcagaaacttccgctgcgggcaacccctacaaaacaaggtccagctcaaggggcgggacctcctgaccctgaagaacttcaccggcgaagagatcaagtacatgctgtggctctccgccgacctgaagttccgcatcaagcagaagggagagtacctcccgctgctgcaagggaagtcgctggggatgatcttcgagaagcggtcaaccagaacccggctgtcaaccgaaaccgggttcgcactgctggggggacacccgtgcttcctgaccacccaagacatccacctgggagtgaacgaatcgctgaccgacaccgcccgcgtgctgagctcaatggcggacgccgtgctggcccgcgtgtacaagcagtccgacctggacaccctggccaaggaagcgtccatcccgatcatcaacggactgtccgacctgtaccacccgatccagatcctggcagactacctgaccctgcaagaacactacagctccctgaagggcctgaccctgtcatggatcggggacgggaacaacatcctgcactccataatgatgtcagccgccaagttcggaatgcacctccaagccgcaaccccgaagggctacgaaccggacgcatcagtgaccaaactggccgagcagtacgccaaggaaaacggcaccaagctcctgctgaccaacgacccgctggaggccgcacacggggggaacgtgctgatcaccgacacctggatctccatgggacaggaggaggaaaagaagaagcggctgcaggcgttccaggggtaccaggtcaccatgaaaaccgcgaaggtcgcggcatcagactggaccttcctgcactgcctgccccggaagccggaagaggtggacgacgaggtgttctactcgccgcgctcgctggtgttccccgaggcggagaacaggaagtggaccatcatggcggtgatggtcagcctcctgaccgactactcgccgcagctgcagaagccgaagttctga

SEQ ID NO: 200 - DNA, 1065 bp, synthetic construct
  source 1..1065: mol_type = other DNA
atgctggtcaacctccgcatcctcctcaacaacgccgcattcagaaacgggcacaacttcatggtcagaaacttccgctgcgggcaacccctacaaaaccgggtccagctcaaggggcgggacctcctgaccctgaagaacttcaccggcgaagagatcaagtacatgctgtggctctccgccgacctgaagttccgcatcaagcagaagggagagtacctcccgctgctgcaagggaagtcgctggggatgatcttcgagaagcggtcaaccagaacccggctgtcaaccgaaaccgggttcgcactgctggggggacacccgtgcttcctgaccacccaagacatccacctgggagtgaacgaatcgctgaccgacaccgcccgcgtgctgagctcaatggcggacgccgtgctggcccgcgtgtacaagcagtccgacctggacaccctggccaaggaagcgtccatcccgatcatcaacggactgtccgacctgtaccacccgatccagatcctggcagactacctgaccctgcaagaacactacagctccctgaagggcctgaccctgtcatggatcggggacgggaacaacatcctgcactccataatgatgtcagccgccaagttcggaatgcacctccaagccgcaaccccgaagggctacgaaccggacgcatcagtgaccaaactggccgagcagtacgccaaggaaaacggcaccaagctcctgctgaccaacgacccgctggaggccgcacacggggggaacgtgctgatcaccgacacctggatctccatgggacaggaggaggaaaagaagaagcggctgcaggcgttccaggggtaccaggtcaccatgaaaaccgcgaaggtcgcggcatcagactggaccttcctgcactgcctgccccggaagccggaagaggtggacgacgaggtgttctactcgccgcgctcgctggtgttccccgaggcggagaacaggaagtggaccatcatggcggtgatggtcagcctcctgaccgactactcgccgcagctgcagaagccgaagttctga

SEQ ID NO: 201 - DNA, 1065 bp, synthetic construct
  source 1..1065: mol_type = other DNA
atgctggtcaacctccgcatcctcctcaacaacgccgcattcagaaacgggcacaacttcatggtcagaaacttccgctgcgggcaacccctacaaaaccgggtccagctcaaggggcgggacctcctgaccctgaagaacttcaccggcgaagagatccggtacatgctgtggctctccgccgacctgaagttccgcatcaagcagaagggagagtacctcccgctgctgcaagggaagtcgctggggatgatcttcgagaagcggtcaaccagaacccggctgtcaaccgaaaccgggttcgcactgctggggggacacccgtgcttcctgaccacccaagacatccacctgggagtgaacgaatcgctgaccgacaccgcccgcgtgctgagctcaatggcggacgccgtgctggcccgcgtgtacaagcagtccgacctggacaccctggccaaggaagcgtccatcccgatcatcaacggactgtccgacctgtaccacccgatccagatcctggcagactacctgaccctgcaagaacactacagctccctgaagggcctgaccctgtcatggatcggggacgggaacaacatcctgcactccataatgatgtcagccgccaagttcggaatgcacctccaagccgcaaccccgaagggctacgaaccggacgcatcagtgaccaaactggccgagcagtacgccaaggaaaacggcaccaagctcctgctgaccaacgacccgctggaggccgcacacggggggaacgtgctgatcaccgacacctggatctccatgggacaggaggaggaaaagaagaagcggctgcaggcgttccaggggtaccaggtcaccatgaaaaccgcgaaggtcgcggcatcagactggaccttcctgcactgcctgccccggaagccggaagaggtggacgacgaggtgttctactcgccgcgctcgctggtgttccccgaggcggagaacaggaagtggaccatcatggcggtgatggtcagcctcctgaccgactactcgccgcagctgcagaagccgaagttctga

SEQ ID NO: 202 - DNA, 1065 bp, synthetic construct
  source 1..1065: mol_type = other DNA
atgctggtcaacctgcgcatcctgctgaacaacgccgccttccgcaacggccacaacttcatggtgcgcaacttccgctgcggccagcccctgcagaacaaggtgcagctgaagggccgcgacctgctgaccctgaagaacttcaccggcgaggagatcaagtacatgctgtggctgagcgccgacctgaagttccgcatcaagcagaagggcgagtacctgcccctgctgcagggcaagagcctgggcatgatcttcgagaagcgcagcacccgcacccgcctgagcaccgagacaggcttcgccctgctgggcggccacccctgcttcctgaccacccaggacatccacctgggcgtgaacgagagcctgaccgacaccgcccgcgtgctgagcagcatggccgacgccgtgctggcccgcgtgtacaagcagagcgacctggacaccctggccaaggaggccagcatccccatcatcaacggcctgagcgacctgtaccaccccatccagatcctggccgactacctgaccctgcaggagcactacagcagcctgaagggcctgaccctgagctggatcggcgacggcaacaacatcctgcacagcatcatgatgagcgccgccaagttcggcatgcacctgcaggccgccacccccaagggctacgagcccgacgccagcgtgaccaagctggccgagcagtacgccaaggagaacggcaccaagctgctgctgaccaacgaccccctggaggccgcccacggcggcaacgtgctgatcaccgacacctggatcagcatgggccaggaggaggagaagaagaagcgcctgcaggccttccagggctaccaggtgaccatgaagaccgccaaggtggccgccagcgactggaccttcctgcactgcctgccccgcaagcccgaggaggtggacgacgaggtgttctacagcccccgcagcctggtgttccccgaggccgagaaccgcaagtggaccatcatggccgtgatggtgagcctgctgaccgactacagcccccagctgcagaagcccaagttctga

SEQ ID NO: 203 - DNA, 1065 bp, synthetic construct
  source 1..1065: mol_type = other DNA
atgctggtcaacctgcgcatcctgctgaacaacgccgccttccgcaacggccacaacttcatggtgcgcaacttccgctgcggccagcccctgcagaaccgggtgcagctgaagggccgcgacctgctgaccctgaagaacttcaccggcgaggagatcaagtacatgctgtggctgagcgccgacctgaagttccgcatcaagcagaagggcgagtacctgcccctgctgcagggcaagagcctgggcatgatcttcgagaagcgcagcacccgcacccgcctgagcaccgagacaggcttcgccctgctgggcggccacccctgcttcctgaccacccaggacatccacctgggcgtgaacgagagcctgaccgacaccgcccgcgtgctgagcagcatggccgacgccgtgctggcccgcgtgtacaagcagagcgacctggacaccctggccaaggaggccagcatccccatcatcaacggcctgagcgacctgtaccaccccatccagatcctggccgactacctgaccctgcaggagcactacagcagcctgaagggcctgaccctgagctggatcggcgacggcaacaacatcctgcacagcatcatgatgagcgccgccaagttcggcatgcacctgcaggccgccacccccaagggctacgagcccgacgccagcgtgaccaagctggccgagcagtacgccaaggagaacggcaccaagctgctgctgaccaacgaccccctggaggccgcccacggcggcaacgtgctgatcaccgacacctggatcagcatgggccaggaggaggagaagaagaagcgcctgcaggccttccagggctaccaggtgaccatgaagaccgccaaggtggccgccagcgactggaccttcctgcactgcctgccccgcaagcccgaggaggtggacgacgaggtgttctacagcccccgcagcctggtgttccccgaggccgagaaccgcaagtggaccatcatggccgtgatggtgagcctgctgaccgactacagcccccagctgcagaagcccaagttctga

SEQ ID NO: 204 - DNA, 1065 bp, synthetic construct
  source 1..1065: mol_type = other DNA
atgcttgtcaatctccgcatcctccttaacaacgccgcgtttagaaacggccacaacttcatggtccggaacttcagatgtggccagccgcttcaaaacaaggtccagctgaagggccgggatcttctgaccctgaagaactttactggcgaagagatcaagtacatgctctggctctccgcggacttgaagttccgcattaagcagaagggggaataccttccgctgcttcaaggaaagagcctcggcatgatctttgagaagcgctcaaccaggacccgcctttctactgaaactgggttcgcgctgctcggtggccacccctgcttcctgacgacccaggacatccacctcggagtgaacgaatccctcaccgataccgcccgggtgttatcgagcatggcagatgccgtgctggccagggtgtacaaacagtccgatctggacactctggccaaggaggcgtcaattcctattatcaacggccttagtgacctctaccatccgattcagatcctggccgattacctcaccctgcaagaacactacagctccctgaagggtctgacattgtcctggatcggcgacggcaacaacattctccattccatcatgatgtccgccgcaaaattcggcatgcatcttcaagccgccacgccgaagggttacgagcccgacgcttccgtgactaagctcgccgagcagtacgctaaggagaacggaaccaagcttctgctgactaacgacccactagaagcagcccacgggggcaacgtgcttattactgacacctggatctccatgggccaggaagaagagaaaaagaagcggctgcaggcgttccagggatatcaggtcaccatgaaaaccgccaaggtcgctgcctccgactggaccttcctgcactgcctgcctcgcaagcctgaagaagtggacgacgaggtgttctactcgccacggagcctcgtgttccccgaggccgagaatagaaagtggaccatcatggccgtgatggtgtcactgctcaccgactacagcccgcagcttcagaagcccaagttctag

SEQ ID NO: 205 - DNA, 1065 bp, synthetic construct
  source 1..1065: mol_type = other DNA
atgcttgtcaatctccgcatcctccttaacaacgccgcgtttagaaacggccacaacttcatggtccggaacttcagatgtggccagccgcttcaaaaccgggtccagctgaagggccgggatcttctgaccctgaagaactttactggcgaagagatcaagtacatgctctggctctccgcggacttgaagttccgcattaagcagaagggggaataccttccgctgcttcaaggaaagagcctcggcatgatctttgagaagcgctcaaccaggacccgcctttctactgaaactgggttcgcgctgctcggtggccacccctgcttcctgacgacccaggacatccacctcggagtgaacgaatccctcaccgataccgcccgggtgttatcgagcatggcagatgccgtgctggccagggtgtacaaacagtccgatctggacactctggccaaggaggcgtcaattcctattatcaacggccttagtgacctctaccatccgattcagatcctggccgattacctcaccctgcaagaacactacagctccctgaagggtctgacattgtcctggatcggcgacggcaacaacattctccattccatcatgatgtccgccgcaaaattcggcatgcatcttcaagccgccacgccgaagggttacgagcccgacgcttccgtgactaagctcgccgagcagtacgctaaggagaacggaaccaagcttctgctgactaacgacccactagaagcagcccacgggggcaacgtgcttattactgacacctggatctccatgggccaggaagaagagaaaaagaagcggctgcaggcgttccagggatatcaggtcaccatgaaaaccgccaaggtcgctgcctccgactggaccttcctgcactgcctgcctcgcaagcctgaagaagtggacgacgaggtgttctactcgccacggagcctcgtgttccccgaggccgagaatagaaagtggaccatcatggccgtgatggtgtcactgctcaccgactacagcccgcagcttcagaagcccaagttctag

SEQ ID NO: 206 - DNA, 1068 bp, synthetic construct
  source 1..1068: mol_type = other DNA
atgggccttgtcaatctccgcatcctccttaacaacgccgcgtttagaaacggccacaacttcatggtccggaacttcagatgtggccagccgcttcaaaacaaggtccagctgaagggccgggatcttctgaccctgaagaactttactggcgaagagatcaagtacatgctctggctctccgcggacttgaagttccgcattaagcagaagggggaataccttccgctgcttcaaggaaagagcctcggcatgatctttgagaagcgctcaaccaggacccgcctttctactgaaactgggttcgcgctgctcggtggccacccctgcttcctgacgacccaggacatccacctcggagtgaacgaatccctcaccgataccgcccgggtgttatcgagcatggcagatgccgtgctggccagggtgtacaaacagtccgatctggacactctggccaaggaggcgtcaattcctattatcaacggccttagtgacctctaccatccgattcagatcctggccgattacctcaccctgcaagaacactacagctccctgaagggtctgacattgtcctggatcggcgacggcaacaacattctccattccatcatgatgtccgccgcaaaattcggcatgcatcttcaagccgccacgccgaagggttacgagcccgacgcttccgtgactaagctcgccgagcagtacgctaaggagaacggaaccaagcttctgctgactaacgacccactagaagcagcccacgggggcaacgtgcttattactgacacctggatctccatgggccaggaagaagagaaaaagaagcggctgcaggcgttccagggatatcaggtcaccatgaaaaccgccaaggtcgctgcctccgactggaccttcctgcactgcctgcctcgcaagcctgaagaagtggacgacgaggtgttctactcgccacggagcctcgtgttccccgaggccgagaatagaaagtggaccatcatggccgtgatggtgtcactgctcaccgactacagcccgcagcttcagaagcccaagttctag

SEQ ID NO: 207 - DNA, 1068 bp, synthetic construct
  source 1..1068: mol_type = other DNA
atgggccttgtcaatctccgcatcctccttaacaacgccgcgtttagaaacggccacaacttcatggtccggaacttcagatgtggccagccgcttcaaaaccgggtccagctgaagggccgggatcttctgaccctgaagaactttactggcgaagagatcaagtacatgctctggctctccgcggacttgaagttccgcattaagcagaagggggaataccttccgctgcttcaaggaaagagcctcggcatgatctttgagaagcgctcaaccaggacccgcctttctactgaaactgggttcgcgctgctcggtggccacccctgcttcctgacgacccaggacatccacctcggagtgaacgaatccctcaccgataccgcccgggtgttatcgagcatggcagatgccgtgctggccagggtgtacaaacagtccgatctggacactctggccaaggaggcgtcaattcctattatcaacggccttagtgacctctaccatccgattcagatcctggccgattacctcaccctgcaagaacactacagctccctgaagggtctgacattgtcctggatcggcgacggcaacaacattctccattccatcatgatgtccgccgcaaaattcggcatgcatcttcaagccgccacgccgaagggttacgagcccgacgcttccgtgactaagctcgccgagcagtacgctaaggagaacggaaccaagcttctgctgactaacgacccactagaagcagcccacgggggcaacgtgcttattactgacacctggatctccatgggccaggaagaagagaaaaagaagcggctgcaggcgttccagggatatcaggtcaccatgaaaaccgccaaggtcgctgcctccgactggaccttcctgcactgcctgcctcgcaagcctgaagaagtggacgacgaggtgttctactcgccacggagcctcgtgttccccgaggccgagaatagaaagtggaccatcatggccgtgatggtgtcactgctcaccgactacagcccgcagcttcagaagcccaagttctag

SEQ ID NO: 208 - DNA, 1071 bp, synthetic construct
  source 1..1071: mol_type = other DNA
atgggcggacttgtcaatctccgcatcctccttaacaacgccgcgtttagaaacggccacaacttcatggtccggaacttcagatgtggccagccgcttcaaaacaaggtccagctgaagggccgggatcttctgaccctgaagaactttactggcgaagagatcaagtacatgctctggctctccgcggacttgaagttccgcattaagcagaagggggaataccttccgctgcttcaaggaaagagcctcggcatgatctttgagaagcgctcaaccaggacccgcctttctactgaaactgggttcgcgctgctcggtggccacccctgcttcctgacgacccaggacatccacctcggagtgaacgaatccctcaccgataccgcccgggtgttatcgagcatggcagatgccgtgctggccagggtgtacaaacagtccgatctggacactctggccaaggaggcgtcaattcctattatcaacggccttagtgacctctaccatccgattcagatcctggccgattacctcaccctgcaagaacactacagctccctgaagggtctgacattgtcctggatcggcgacggcaacaacattctccattccatcatgatgtccgccgcaaaattcggcatgcatcttcaagccgccacgccgaagggttacgagcccgacgcttccgtgactaagctcgccgagcagtacgctaaggagaacggaaccaagcttctgctgactaacgacccactagaagcagcccacgggggcaacgtgcttattactgacacctggatctccatgggccaggaagaagagaaaaagaagcggctgcaggcgttccagggatatcaggtcaccatgaaaaccgccaaggtcgctgcctccgactggaccttcctgcactgcctgcctcgcaagcctgaagaagtggacgacgaggtgttctactcgccacggagcctcgtgttccccgaggccgagaatagaaagtggaccatcatggccgtgatggtgtcactgctcaccgactacagcccgcagcttcagaagcccaagttctag

SEQ ID NO: 209 - DNA, 1077 bp, synthetic construct
  source 1..1077: mol_type = other DNA
atggcccttttcaatctccgcatcctccttaacaacgccgcgtttagaaacggccacaacttcatggtccggaacttcagatgtggccagccgcttcaaggcaaggtccagctgaagggccgggatcttctgaccctgaagaactttactggcgaagagatcaagtacatgctctggctctccgcggacttgaagttccgcattaagcagaagggggaataccttccgctgcttcaaggaaagagcctcggcatgatctttgagaagcgctcaaccaggacccgcctttctactgaaactgggttcgcgctgctcggtggccacccctgcttcctgacgacccaggacatccacctcggagtgaacgaatccctcaccgataccgcccgggtgttatcgagcatggcagatgccgtgctggccagggtgtacaaacagtccgatctggacactctggccaaggaggcgtcaattcctattatcaacggccttagtgacctctaccatccgattcagatcctggccgattacctcaccctgcaagaacactacagctccctgaagggtctgacattgtcctggatcggcgacggcaacaacattctccattccatcatgatgtccgccgcaaaattcggcatgcatcttcaagccgccacgccgaagggttacgagcccgacgcttccgtgactaagctcgccgagcagtacgctaaggagaacggaaccaagcttctgctgactaacgacccactagaagcagcccacgggggcaacgtgcttattactgacacctggatctccatgggccaggaagaagagaaaaagaagcggctgcaggcgttccagggatatcaggtcaccatgaaaaccgccaaggtcgctgcctccgactggaccttcctgcactgcctgcctcgcaagcctgaagaagtggacgacgaggtgttctactcgccacggagcctcgtgttccccgaggccgagaatagaaagtggaccatcatggccgtgatggtgtcactgctcaccgactacagcccgcagcttcagaagcccaagttctagataagtgaa

SEQ ID NO: 210 - DNA, 1077 bp, synthetic construct
  source 1..1077: mol_type = other DNA
atggcccttttcaatctccgcatcctccttaacaacgccgcgtttagaaacggccacaacttcatggtccggaacttcagatgtggccagccgcttcaaggccgggtccagctgaagggccgggatcttctgaccctgaagaactttactggcgaagagatcaagtacatgctctggctctccgcggacttgaagttccgcattaagcagaagggggaataccttccgctgcttcaaggaaagagcctcggcatgatctttgagaagcgctcaaccaggacccgcctttctactgaaactgggttcgcgctgctcggtggccacccctgcttcctgacgacccaggacatccacctcggagtgaacgaatccctcaccgataccgcccgggtgttatcgagcatggcagatgccgtgctggccagggtgtacaaacagtccgatctggacactctggccaaggaggcgtcaattcctattatcaacggccttagtgacctctaccatccgattcagatcctggccgattacctcaccctgcaagaacactacagctccctgaagggtctgacattgtcctggatcggcgacggcaacaacattctccattccatcatgatgtccgccgcaaaattcggcatgcatcttcaagccgccacgccgaagggttacgagcccgacgcttccgtgactaagctcgccgagcagtacgctaaggagaacggaaccaagcttctgctgactaacgacccactagaagcagcccacgggggcaacgtgcttattactgacacctggatctccatgggccaggaagaagagaaaaagaagcggctgcaggcgttccagggatatcaggtcaccatgaaaaccgccaaggtcgctgcctccgactggaccttcctgcactgcctgcctcgcaagcctgaagaagtggacgacgaggtgttctactcgccacggagcctcgtgttccccgaggccgagaatagaaagtggaccatcatggccgtgatggtgtcactgctcaccgactacagcccgcagcttcagaagcccaagttctagataagtgaa

SEQ ID NO: 211 - DNA, 1077 bp, synthetic construct
  source 1..1077: mol_type = other DNA
atggcccttttcaatctccgcatcctccttaacaacgccgcgtttagaaacggccacaacttcatggtccggaacttcagatgtggccagccgcttcaaggccgggtccagctgaagggccgggatcttctgaccctgaagaactttactggcgaagagatcaggtacatgctctggctctccgcggacttgaagttccgcattaagcagaagggggaataccttccgctgcttcaaggaaagagcctcggcatgatctttgagaagcgctcaaccaggacccgcctttctactgaaactgggttcgcgctgctcggtggccacccctgcttcctgacgacccaggacatccacctcggagtgaacgaatccctcaccgataccgcccgggtgttatcgagcatggcagatgccgtgctggccagggtgtacaaacagtccgatctggacactctggccaaggaggcgtcaattcctattatcaacggccttagtgacctctaccatccgattcagatcctggccgattacctcaccctgcaagaacactacagctccctgaagggtctgacattgtcctggatcggcgacggcaacaacattctccattccatcatgatgtccgccgcaaaattcggcatgcatcttcaagccgccacgccgaagggttacgagcccgacgcttccgtgactaagctcgccgagcagtacgctaaggagaacggaaccaagcttctgctgactaacgacccactagaagcagcccacgggggcaacgtgcttattactgacacctggatctccatgggccaggaagaagagaaaaagaagcggctgcaggcgttccagggatatcaggtcaccatgaaaaccgccaaggtcgctgcctccgactggaccttcctgcactgcctgcctcgcaagcctgaagaagtggacgacgaggtgttctactcgccacggagcctcgtgttccccgaggccgagaatagaaagtggaccatcatggccgtgatggtgtcactgctcaccgactacagcccgcagcttcagaagcccaagttctagataagtgaa

SEQ ID NO: 212 - DNA, 1077 bp, synthetic construct
  source 1..1077: mol_type = other DNA
atggcccttgtcaatctccgcatcctccttaacaacgccgcgtttagaaacggccacaacttcatggtccggaacttcagatgtggccagccgcttcaaggcagggtccagctgaagggccgggatcttctgaccctgaagaactttactggcgaagagatcaagtacatgctctggctctccgcggacttgaagttccgcattaagcagaagggggaataccttccgctgcttcaaggaaagagcctcggcatgatctttgagaagcgctcaaccaggacccgcctttctactgaaactgggttcgcgctgctcggtggccacccctgcttcctgacgacccaggacatccacctcggagtgaacgaatccctcaccgataccgcccgggtgttatcgagcatggcagatgccgtgctggccagggtgtacaaacagtccgatctggacactctggccaaggaggcgtcaattcctattatcaacggccttagtgacctctaccatccgattcagatcctggccgattacctcaccctgcaagaacactacagctccctgaagggtctgacattgtcctggatcggcgacggcaacaacattctccattccatcatgatgtccgccgcaaaattcggcatgcatcttcaagccgccacgccgaagggttacgagcccgacgcttccgtgactaagctcgccgagcagtacgctaaggagaacggaaccaagcttctgctgactaacgacccactagaagcagcccacgggggcaacgtgcttattactgacacctggatctccatgggccaggaagaagagaaaaagaagcggctgcaggcgttccagggatatcaggtcaccatgaaaaccgccaaggtcgctgcctccgactggaccttcctgcactgcctgcctcgcaagcctgaagaagtggacgacgaggtgttctactcgccacggagcctcgtgttccccgaggccgagaatagaaagtggaccatcatggccgtgatggtgtcactgctcaccgactacagcccgcagcttcagaagcccaagttctaagtgaataga

SEQ ID NO: 213 - DNA, 1077 bp, synthetic construct
  source 1..1077: mol_type = other DNA
atggcccttttcaatctccgcatcctccttaacaacgccgcgtttagaaacggccacaacttcatggtccggaacttcagatgtggccagccgcttcaagtcaaggtccagctgaagggccgggatcttctgaccctgaagaactttactggcgaagagatcaagtacatgctctggctctccgcggacttgaagttccgcattaagcagaagggggaataccttccgctgcttcaaggaaagagcctcggcatgatctttgagaagcgctcaaccaggacccgcctttctactgaaactgggttcgcgctgctcggtggccacccctgcttcctgacgacccaggacatccacctcggagtgaacgaatccctcaccgataccgcccgggtgttatcgagcatggcagatgccgtgctggccagggtgtacaaacagtccgatctggacactctggccaaggaggcgtcaattcctattatcaacggccttagtgacctctaccatccgattcagatcctggccgattacctcaccctgcaagaacactacagctccctgaagggtctgacattgtcctggatcggcgacggcaacaacattctccattccatcatgatgtccgccgcaaaattcggcatgcatcttcaagccgccacgccgaagggttacgagcccgacgcttccgtgactaagctcgccgagcagtacgctaaggagaacggaaccaagcttctgctgactaacgacccactagaagcagcccacgggggcaacgtgcttattactgacacctggatctccatgggccaggaagaagagaaaaagaagcggctgcaggcgttccagggatatcaggtcaccatgaaaaccgccaaggtcgctgcctccgactggaccttcctgcactgcctgcctcgcaagcctgaagaagtggacgacgaggtgttctactcgccacggagcctcgtgttccccgaggccgagaatagaaagtggaccatcatggccgtgatggtgtcactgctcaccgactacagcccgcagcttcagaagcccaagttctagataagtgaa

SEQ ID NO: 214 - DNA, 1077 bp, synthetic construct
  source 1..1077: mol_type = other DNA
atggcccttttcaatctccgcatcctccttaacaacgccgcgtttagaaacggccacaacttcatggtccggaacttcagatgtggccagccgcttcaagtcagggtccagctgaagggccgggatcttctgaccctgaagaactttactggcgaagagatcaagtacatgctctggctctccgcggacttgaagttccgcattaagcagaagggggaataccttccgctgcttcaaggaaagagcctcggcatgatctttgagaagcgctcaaccaggacccgcctttctactgaaactgggttcgcgctgctcggtggccacccctgcttcctgacgacccaggacatccacctcggagtgaacgaatccctcaccgataccgcccgggtgttatcgagcatggcagatgccgtgctggccagggtgtacaaacagtccgatctggacactctggccaaggaggcgtcaattcctattatcaacggccttagtgacctctaccatccgattcagatcctggccgattacctcaccctgcaagaacactacagctccctgaagggtctgacattgtcctggatcggcgacggcaacaacattctccattccatcatgatgtccgccgcaaaattcggcatgcatcttcaagccgccacgccgaagggttacgagcccgacgcttccgtgactaagctcgccgagcagtacgctaaggagaacggaaccaagcttctgctgactaacgacccactagaagcagcccacgggggcaacgtgcttattactgacacctggatctccatgggccaggaagaagagaaaaagaagcggctgcaggcgttccagggatatcaggtcaccatgaaaaccgccaaggtcgctgcctccgactggaccttcctgcactgcctgcctcgcaagcctgaagaagtggacgacgaggtgttctactcgccacggagcctcgtgttccccgaggccgagaatagaaagtggaccatcatggccgtgatggtgtcactgctcaccgactacagcccgcagcttcagaagcccaagttctagataagtgaa

SEQ ID NO: 215 - DNA, 1065 bp, synthetic construct; identical to SEQ ID NO: 175
  source 1..1065: mol_type = other DNA

SEQ ID NO: 216 - DNA, 1068 bp, synthetic construct
  source 1..1068: mol_type = other DNA
atgggagtattcaacctgcgcatcctgctgaacaacgccgccttccgcaacggccacaacttcatggtgcgcaacttccgctgcggccagcccctgcagaacaaggtgcagctgaagggccgcgacctgctgaccctgaagaacttcaccggcgaggagatcaagtacatgctgtggctgagcgccgacctgaagttccgcatcaagcagaagggcgagtacctgcccctgctgcagggcaagagcctgggcatgatcttcgagaagcgcagcacccgcacccgcctgagcaccgagacaggcttcgccctgctgggcggccacccctgcttcctgaccacccaggacatccacctgggcgtgaacgagagcctgaccgacaccgcccgcgtgctgagcagcatggccgacgccgtgctggcccgcgtgtacaagcagagcgacctggacaccctggccaaggaggccagcatccccatcatcaacggcctgagcgacctgtaccaccccatccagatcctggccgactacctgaccctgcaggagcactacagcagcctgaagggcctgaccctgagctggatcggcgacggcaacaacatcctgcacagcatcatgatgagcgccgccaagttcggcatgcacctgcaggccgccacccccaagggctacgagcccgacgccagcgtgaccaagctggccgagcagtacgccaaggagaacggcaccaagctgctgctgaccaacgaccccctggaggccgcccacggcggcaacgtgctgatcaccgacacctggatcagcatgggccaggaggaggagaagaagaagcgcctgcaggccttccagggctaccaggtgaccatgaagaccgccaaggtggccgccagcgactggaccttcctgcactgcctgccccgcaagcccgaggaggtggacgacgaggtgttctacagcccccgcagcctggtgttccccgaggccgagaaccgcaagtggaccatcatggccgtgatggtgagcctgctgaccgactacagcccccagctgcagaagcccaagttctga

SEQ ID NO: 217 - DNA, 1068 bp, synthetic construct
  source 1..1068: mol_type = other DNA
atgggagtattcaacctgcgcatcctgctgaacaacgccgccttccgcaacggccacaacttcatggtgcgcaacttccgctgcggccagcccctgcagaaccgggtgcagctgaagggccgcgacctgctgaccctgaagaacttcaccggcgaggagatccggtacatgctgtggctgagcgccgacctgaagttccgcatcaagcagaagggcgagtacctgcccctgctgcagggcaagagcctgggcatgatcttcgagaagcgcagcacccgcacccgcctgagcaccgagacaggcttcgccctgctgggcggccacccctgcttcctgaccacccaggacatccacctgggcgtgaacgagagcctgaccgacaccgcccgcgtgctgagcagcatggccgacgccgtgctggcccgcgtgtacaagcagagcgacctggacaccctggccaaggaggccagcatccccatcatcaacggcctgagcgacctgtaccaccccatccagatcctggccgactacctgaccctgcaggagcactacagcagcctgaagggcctgaccctgagctggatcggcgacggcaacaacatcctgcacagcatcatgatgagcgccgccaagttcggcatgcacctgcaggccgccacccccaagggctacgagcccgacgccagcgtgaccaagctggccgagcagtacgccaaggagaacggcaccaagctgctgctgaccaacgaccccctggaggccgcccacggcggcaacgtgctgatcaccgacacctggatcagcatgggccaggaggaggagaagaagaagcgcctgcaggccttccagggctaccaggtgaccatgaagaccgccaaggtggccgccagcgactggaccttcctgcactgcctgccccgcaagcccgaggaggtggacgacgaggtgttctacagcccccgcagcctggtgttccccgaggccgagaaccgcaagtggaccatcatggccgtgatggtgagcctgctgaccgactacagcccccagctgcagaagcccaagttctga

SEQ ID NO: 218 - DNA, 1068 bp, synthetic construct
  source 1..1068: mol_type = other DNA
atgctggtattcaacctgcgcatcctgctgaacaacgccgccttccgcaacggccacaacttcatggtgcgcaacttccgctgcggccagcccctgcagaaccgggtgcagctgaagggccgcgacctgctgaccctgaagaacttcaccggcgaggagatccggtacatgctgtggctgagcgccgacctgaagttccgcatcaagcagaagggcgagtacctgcccctgctgcagggcaagagcctgggcatgatcttcgagaagcgcagcacccgcacccgcctgagcaccgagacaggcttcgccctgctgggcggccacccctgcttcctgaccacccaggacatccacctgggcgtgaacgagagcctgaccgacaccgcccgcgtgctgagcagcatggccgacgccgtgctggcccgcgtgtacaagcagagcgacctggacaccctggccaaggaggccagcatccccatcatcaacggcctgagcgacctgtaccaccccatccagatcctggccgactacctgaccctgcaggagcactacagcagcctgaagggcctgaccctgagctggatcggcgacggcaacaacatcctgcacagcatcatgatgagcgccgccaagttcggcatgcacctgcaggccgccacccccaagggctacgagcccgacgccagcgtgaccaagctggccgagcagtacgccaaggagaacggcaccaagctgctgctgaccaacgaccccctggaggccgcccacggcggcaacgtgctgatcaccgacacctggatcagcatgggccaggaggaggagaagaagaagcgcctgcaggccttccagggctaccaggtgaccatgaagaccgccaaggtggccgccagcgactggaccttcctgcactgcctgccccgcaagcccgaggaggtggacgacgaggtgttctacagcccccgcagcctggtgttccccgaggccgagaaccgcaagtggaccatcatggccgtgatggtgagcctgctgaccgactacagcccccagctgcagaagcccaagttctga

SEQ ID NO: 219 - DNA, 1068 bp, synthetic construct; identical to SEQ ID NO: 216
  source 1..1068: mol_type = other DNA

SEQ ID NO: 220 - DNA, 1068 bp, synthetic construct; identical to SEQ ID NO: 217
  source 1..1068: mol_type = other DNA

SEQ ID NO: 221 - DNA, 1068 bp, synthetic construct; identical to SEQ ID NO: 218
  source 1..1068: mol_type = other DNA

SEQ ID NO: 222 - DNA, 1073 bp, synthetic construct
  source 1..1073: mol_type = other DNA
atgttgttcaacttgaggatcttgttgaacaacgccgccttcaggaacggacacaacttcatggtaaggaacttcaggtgcggacagcccttgcagaacaaagtacagttgaaaggaagggacttgttgacattgaaaaacttcacaggagaagaaatcaaatacatgttgtggttgtcggccgacttgaaattcaggatcaaacagaaaggagaatacttgcccttgttgcagggaaaatcgttgggaatgatcttcgaaaaaaggtcgacaaggacaaggttgtcgacagaaacaggattcgccttgttgggaggacacccctgcttcttgacaacacaggacatccacttgggagtaaacgaatcgttgacagacacagccagggtattgtcgtcgatggccgacgccgtattggccagggtatacaaacagtcggacttggacacattggccaaagaagcctcgatccccatcatcaacggattgtcggacttgtaccaccccatccagatcttggccgactacttgacattgcaggaacactactcgtcgttgaaaggattgacattgtcgtggatcggagacggaaacaacatcttgcactcgatcatgatgtcggccgccaaattcggaatgcacttgcaggccgccacacccaaaggatacgaacccgacgcctcggtaacaaaattggccgaacagtacgccaaagaaaacggaacaaaattgttgttgacaaacgaccccttggaagccgcccacggaggaaacgtattgatcacagacacatggatctcgatgggacaggaagaagaaaaaaaaaaaaggttgcaggccttccagggataccaggtaacaatgaaaacagccaaagtagccgcctcggactggacattcttgcactgcttgcccaggaaacccgaagaagtagacgacgaagtattctactcgcccaggtcgttggtattccccgaagccgaaaacaggaaatggacaatcatggccgtaatggtatcgttgttgacagactactcgccccagttgcagaaacccaaattctgaatagtgaa

SEQ ID NO: 223 - DNA, 1065 bp, synthetic construct
  source 1..1065: mol_type = other DNA
atgctgttcaacctgcgcatcctgctgaacaacgccgccttccgcaacggccacaacttcatggtgcgcaacttccgctgcggccagcccctgcagggcaaggtgcagctgaagggccgcgacctgctgaccctgaagaacttcaccggcgaggagatcaagtacatgctgtggctgagcgccgacctgaagttccgcatcaagcagaagggcgagtacctgcccctgctgcagggcaagagcctgggcatgatcttcgagaagcgcagcacccgcacccgcctgagcaccgagacaggcttcgccctgctgggcggccacccctgcttcctgaccacccaggacatccacctgggcgtgaacgagagcctgaccgacaccgcccgcgtgctgagcagcatggccgacgccgtgctggcccgcgtgtacaagcagagcgacctggacaccctggccaaggaggccagcatccccatcatcaacggcctgagcgacctgtaccaccccatccagatcctggccgactacctgaccctgcaggagcactacagcagcctgaagggcctgaccctgagctggatcggcgacggcaacaacatcctgcacagcatcatgatgagcgccgccaagttcggcatgcacctgcaggccgccacccccaagggctacgagcccgacgccagcgtgaccaagctggccgagcagtacgccaaggagaacggcaccaagctgctgctgaccaacgaccccctggaggccgcccacggcggcaacgtgctgatcaccgacacctggatcagcatgggccaggaggaggagaagaagaagcgcctgcaggccttccagggctaccaggtgaccatgaagaccgccaaggtggccgccagcgactggaccttcctgcactgcctgccccgcaagcccgaggaggtggacgacgaggtgttctacagcccccgcagcctggtgttccccgaggccgagaaccgcaagtggaccatcatggccgtgatggtgagcctgctgaccgactacagcccccagctgcagaagcccaagttctga

SEQ ID NO: 224 - DNA, 1065 bp, synthetic construct
  source 1..1065: mol_type = other DNA
atgctgttcaacctgcgcatcctgctgaacaacgccgccttccgcaacggccacaacttcatggtgcgcaacttccgctgcggccagcccctgcagggccgggtgcagctgaagggccgcgacctgctgaccctgaagaacttcaccggcgaggagatcaagtacatgctgtggctgagcgccgacctgaagttccgcatcaagcagaagggcgagtacctgcccctgctgcagggcaagagcctgggcatgatcttcgagaagcgcagcacccgcacccgcctgagcaccgagacaggcttcgccctgctgggcggccacccctgcttcctgaccacccaggacatccacctgggcgtgaacgagagcctgaccgacaccgcccgcgtgctgagcagcatggccgacgccgtgctggcccgcgtgtacaagcagagcgacctggacaccctggccaaggaggccagcatccccatcatcaacggcctgagcgacctgtaccaccccatccagatcctggccgactacctgaccctgcaggagcactacagcagcctgaagggcctgaccctgagctggatcggcgacggcaacaacatcctgcacagcatcatgatgagcgccgccaagttcggcatgcacctgcaggccgccacccccaagggctacgagcccgacgccagcgtgaccaagctggccgagcagtacgccaaggagaacggcaccaagctgctgctgaccaacgaccccctggaggccgcccacggcggcaacgtgctgatcaccgacacctggatcagcatgggccaggaggaggagaagaagaagcgcctgcaggccttccagggctaccaggtgaccatgaagaccgccaaggtggccgccagcgactggaccttcctgcactgcctgccccgcaagcccgaggaggtggacgacgaggtgttctacagcccccgcagcctggtgttccccgaggccgagaaccgcaagtggaccatcatggccgtgatggtgagcctgctgaccgactacagcccccagctgcagaagcccaagttctga

SEQ ID NO: 225 - DNA, 1065 bp, synthetic construct
  source 1..1065: mol_type = other DNA
atgctgttcaacctgcgcatcctgctgaacaacgccgccttccgcaacggccacaacttcatggtgcgcaacttccgctgcggccagcccctgcagggccgggtgcagctgaagggccgcgacctgctgaccctgaagaacttcaccggcgaggagatccggtacatgctgtggctgagcgccgacctgaagttccgcatcaagcagaagggcgagtacctgcccctgctgcagggcaagagcctgggcatgatcttcgagaagcgcagcacccgcacccgcctgagcaccgagacaggcttcgccctgctgggcggccacccctgcttcctgaccacccaggacatccacctgggcgtgaacgagagcctgaccgacaccgcccgcgtgctgagcagcatggccgacgccgtgctggcccgcgtgtacaagcagagcgacctggacaccctggccaaggaggccagcatccccatcatcaacggcctgagcgacctgtaccaccccatccagatcctggccgactacctgaccctgcaggagcactacagcagcctgaagggcctgaccctgagctggatcggcgacggcaacaacatcctgcacagcatcatgatgagcgccgccaagttcggcatgcacctgcaggccgccacccccaagggctacgagcccgacgccagcgtgaccaagctggccgagcagtacgccaaggagaacggcaccaagctgctgctgaccaacgaccccctggaggccgcccacggcggcaacgtgctgatcaccgacacctggatcagcatgggccaggaggaggagaagaagaagcgcctgcaggccttccagggctaccaggtgaccatgaagaccgccaaggtggccgccagcgactggaccttcctgcactgcctgccccgcaagcccgaggaggtggacgacgaggtgttctacagcccccgcagcctggtgttccccgaggccgagaaccgcaagtggaccatcatggccgtgatggtgagcctgctgaccgactacagcccccagctgcagaagcccaagttctga

SEQ ID NO: 226 - DNA, 1065 bp, synthetic construct; identical to SEQ ID NO: 223
  source 1..1065: mol_type = other DNA

SEQ ID NO: 227 - DNA, 1065 bp, synthetic construct; identical to SEQ ID NO: 175
  source 1..1065: mol_type = other DNA

SEQ ID NO: 228 - DNA, 1068 bp, synthetic construct; identical to SEQ ID NO: 218
  source 1..1068: mol_type = other DNA

SEQ ID NO: 229 - DNA, 1068 bp, synthetic construct; identical to SEQ ID NO: 218
  source 1..1068: mol_type = other DNA

SEQ ID NO: 230 - RNA, 21 nt, synthetic construct
  source 1..21: mol_type = other RNA
aaccaatcgaaagaaaccaaa

SEQ ID NO: 231 - RNA, 21 nt, synthetic construct
  source 1..21: mol_type = other RNA
ctctaatcaccaggagtaaaa

SEQ ID NO: 232 - RNA, 21 nt, synthetic construct
  source 1..21: mol_type = other RNA
gagagagatcttaacaaaaaa

SEQ ID NO: 233 - RNA, 21 nt, synthetic construct
  source 1..21: mol_type = other RNA
tgtgtaacaacaacaacaaca

SEQ ID NO: 234 - RNA, 21 nt, synthetic construct
  source 1..21: mol_type = other RNA
ccgcagtaggaagagaaagcc

SEQ ID NO: 235 - RNA, 21 nt, synthetic construct
  source 1..21: mol_type = other RNA
aaaaaaaaaagaaatcataaa

SEQ ID NO: 236 - RNA, 21 nt, synthetic construct
  source 1..21: mol_type = other RNA
gagagaagaaagaagaagacg

SEQ ID NO: 237 - RNA, 21 nt, synthetic construct
  source 1..21: mol_type = other RNA
caattaaaaatacttaccaaa

SEQ ID NO: 238 - RNA, 21 nt, synthetic construct
  source 1..21: mol_type = other RNA
gcaaacagagtaagcgaaacg

SEQ ID NO: 239 - RNA, 21 nt, synthetic construct
  source 1..21: mol_type = other RNA
gcgaagaagacgaacgcaaag

SEQ ID NO: 240 - RNA, 21 nt, synthetic construct
  source 1..21: mol_type = other RNA
ttaggactgtattgactggcc

SEQ ID NO: 241 - RNA, 21 nt, synthetic construct
  source 1..21: mol_type = other RNA
atcatcggaattcggaaaaag

SEQ ID NO: 242 - RNA, 21 nt, synthetic construct
  source 1..21: mol_type = other RNA
aaaacaaaagttaaagcagac

SEQ ID NO: 243 - RNA, 21 nt, synthetic construct
  source 1..21: mol_type = other RNA
tttatctcaaataagaaggca

SEQ ID NO: 244 - RNA, 21 nt, synthetic construct
  source 1..21: mol_type = other RNA
ggtggggaggtgagatttctt

SEQ ID NO: 245 - RNA, 21 nt, synthetic construct
  source 1..21: mol_type = other RNA
tgattaggaaactacaaagcc

SEQ ID NO: 246 - RNA, 21 nt, synthetic construct
  source 1..21: mol_type = other RNA
catttttcaatttcataaaac

SEQ ID NO: 247 - RNA, 21 nt, synthetic construct
  source 1..21: mol_type = other RNA
ttacttttaagcccaacaaaa

SEQ ID NO: 248 - RNA, 21 nt, synthetic construct
  source 1..21: mol_type = other RNA
ggcgtgtgtgtgtgttgttga

SEQ ID NO: 249 - RNA, 21 nt, synthetic construct
  source 1..21: mol_type = other RNA
gtggtgaaggggaaggtttag

SEQ ID NO: 250 - RNA, 21 nt, synthetic construct
  source 1..21: mol_type = other RNA
ttgtttttttttggtttggtt

SEQ ID NO: 251 - RNA, 1331 nt, synthetic construct
  source 1..1331: mol_type = other RNA
aggattattacatcaaaacaaaaagccgccaccatgctggtattcaacctgcgcatcctgctgaacaacgccgccttccgcaacggccacaacttcatggtgcgcaacttccgctgcggccagcccctgcagaaccgggtgcagctgaagggccgcgacctgctgaccctgaagaacttcaccggcgaggagatccggtacatgctgtggctgagcgccgacctgaagttccgcatcaagcagaagggcgagtacctgcccctgctgcagggcaagagcctgggcatgatcttcgagaagcgcagcacccgcacccgcctgagcaccgagacaggcttcgccctgctgggcggccacccctgcttcctgaccacccaggacatccacctgggcgtgaacgagagcctgaccgacaccgcccgcgtgctgagcagcatggccgacgccgtgctggcccgcgtgtacaagcagagcgacctggacaccctggccaaggaggccagcatccccatcatcaacggcctgagcgacctgtaccaccccatccagatcctggccgactacctgaccctgcaggagcactacagcagcctgaagggcctgaccctgagctggatcggcgacggcaacaacatcctgcacagcatcatgatgagcgccgccaagttcggcatgcacctgcaggccgccacccccaagggctacgagcccgacgccagcgtgaccaagctggccgagcagtacgccaaggagaacggcaccaagctgctgctgaccaacgaccccctggaggccgcccacggcggcaacgtgctgatcaccgacacctggatcagcatgggccaggaggaggagaagaagaagcgcctgcaggccttccagggctaccaggtgaccatgaagaccgccaaggtggccgccagcgactggaccttcctgcactgcctgccccgcaagcccgaggaggtggacgacgaggtgttctacagcccccgcagcctggtgttccccgaggccgagaaccgcaagtggaccatcatggccgtgatggtgagcctgctgaccgactacagcccccagctgcagaagcccaagttctgaggtctctagtaatgagctggagcctcggtagccgttcctcctgcccgctgggcctcccaacgggccctcctcccctccttgcaccggcccttcctggtctttgaataaagtctgagtgggcagcatctagaaaaaaaaaaaaaaaaaaaaaaaaaaaaaaaaaaaaaaaaaaaaaaaaaaaaaaaaaaaaaaaaaaaaaaaaaaaaaaaaaaaaaaaaaaaaaaaaaaaa

SEQ ID NO: 252 - RNA, 1334 nt, synthetic construct
  source 1..1334: mol_type = other RNA
aggattattacatcaaaacaaaaagccgccaccatgctggtattcaacctgcgcatcctgctgaacaacgccgccttccgcaacggccacaacttcatggtgcgcaacttccgctgcggccagcccctgcagaaccgggtgcagctgaagggccgcgacctgctgaccctgaagaacttcaccggcgaggagatccggtacatgctgtggctgagcgccgacctgaagttccgcatcaagcagaagggcgagtacctgcccctgctgcagggcaagagcctgggcatgatcttcgagaagcgcagcacccgcacccgcctgagcaccgagacaggcttcgccctgctgggcggccacccctgcttcctgaccacccaggacatccacctgggcgtgaacgagagcctgaccgacaccgcccgcgtgctgagcagcatggccgacgccgtgctggcccgcgtgtacaagcagagcgacctggacaccctggccaaggaggccagcatccccatcatcaacggcctgagcgacctgtaccaccccatccagatcctggccgactacctgaccctgcaggagcactacagcagcctgaagggcctgaccctgagctggatcggcgacggcaacaacatcctgcacagcatcatgatgagcgccgccaagttcggcatgcacctgcaggccgccacccccaagggctacgagcccgacgccagcgtgaccaagctggccgagcagtacgccaaggagaacggcaccaagctgctgctgaccaacgaccccctggaggccgcccacggcggcaacgtgctgatcaccgacacctggatcagcatgggccaggaggaggagaagaagaagcgcctgcaggccttccagggctaccaggtgaccatgaagaccgccaaggtggccgccagcgactggaccttcctgcactgcctgccccgcaagcccgaggaggtggacgacgaggtgttctacagcccccgcagcctggtgttccccgaggccgagaaccgcaagtggaccatcatggccgtgatggtgagcctgctgaccgactacagcccccagctgcagaagcccaagttctgaggtctctagtaatgagctggagcctcggtagccgttcctcctgcccgctgggcctcccaacgggccctcctcccctccttgcaccggcccttcctggtctttgaataaagtctgagtgggcagcatctagaaaaaaaaaaaaaaaaaaaaaaaaaaaaaaaaaaaaaaaaaaaaaaaaaaaaaaaaaaaaaaaaaaaaaaaaaaaaaaaaaaaaaaaaaaaaaaaaaaaagct

SEQ ID NO: 253 - RNA, 1328 nt, synthetic construct
  source 1..1328: mol_type = other RNA
aggattattacatcaaaacaaaaagccgccaccatgctgttcaacctgcgcatcctgctgaacaacgccgccttccgcaacggccacaacttcatggtgcgcaacttccgctgcggccagcccctgcagaacaaggtgcagctgaagggccgcgacctgctgaccctgaagaacttcaccggcgaggagatcaagtacatgctgtggctgagcgccgacctgaagttccgcatcaagcagaagggcgagtacctgcccctgctgcagggcaagagcctgggcatgatcttcgagaagcgcagcacccgcacccgcctgagcaccgagacaggcttcgccctgctgggcggccacccctgcttcctgaccacccaggacatccacctgggcgtgaacgagagcctgaccgacaccgcccgcgtgctgagcagcatggccgacgccgtgctggcccgcgtgtacaagcagagcgacctggacaccctggccaaggaggccagcatccccatcatcaacggcctgagcgacctgtaccaccccatccagatcctggccgactacctgaccctgcaggagcactacagcagcctgaagggcctgaccctgagctggatcggcgacggcaacaacatcctgcacagcatcatgatgagcgccgccaagttcggcatgcacctgcaggccgccacccccaagggctacgagcccgacgccagcgtgaccaagctggccgagcagtacgccaaggagaacggcaccaagctgctgctgaccaacgaccccctggaggccgcccacggcggcaacgtgctgatcaccgacacctggatcagcatgggccaggaggaggagaagaagaagcgcctgcaggccttccagggctaccaggtgaccatgaagaccgccaaggtggccgccagcgactggaccttcctgcactgcctgccccgcaagcccgaggaggtggacgacgaggtgttctacagcccccgcagcctggtgttccccgaggccgagaaccgcaagtggaccatcatggccgtgatggtgagcctgctgaccgactacagcccccagctgcagaagcccaagttctgaggtctctagtaatgagctggagcctcggtagccgttcctcctgcccgctgggcctcccaacgggccctcctcccctccttgcaccggcccttcctggtctttgaataaagtctgagtgggcagcatctagaaaaaaaaaaaaaaaaaaaaaaaaaaaaaaaaaaaaaaaaaaaaaaaaaaaaaaaaaaaaaaaaaaaaaaaaaaaaaaaaaaaaaaaaaaaaaaaaaaaa